European Patent Application EP 4 748 855 A1, published May 27, 2026. Title: New molecules for the prevention of false positive agglutination. Applicant: mAb-factory GmbH. Application EP. The sequence listing filed with the application follows.

SEQUENCE LISTING (342 sequences)

SEQ ID NO: 1 - protein, 258 aa, Homo sapiens
VPRWRQQWSGPGTTKRFPETVLARCVKYTEIHPEMRHVDCQSVWDAFKGAFISKHPCNITEEDYQPLMKLGTQTVPCNKILLWSRIKDLAHQFTQVQRDMFTLEDTLLGYLADDLTWCGEFNTSKINYQSCPDWRKDCSNNPVSVFWKTVSRRFAEAACDVVHVMLNGSRSKIFDKNSTFGSVEVHNLQPEKVQTLEAWVIHGGREDSRDLCQDPTIKELESIISKRNIQFSCKNIYRPDKFLQCVKNPEDSSCTSEI

SEQ ID NO: 2 - protein, 258 aa, Homo sapiens
VPRWRQQWSGPGTTKRFPETVLARCVKYTEIHPEMRHVDCQSVWDAFKGAFISKHPCNITEEDYQPLMKLGTQTVPCNKKLLWSRIKDLAHQFTQVQRDMFTLEDTLLGYLADDLTWCGEFNTSKINYQSCPDWRKDCSNNPVSVFWKTVSRRFAEAACDVVHVMLNGSRSKIFDKNSTFGSVEVHNLQPEKVQTLEAWVIHGGREDSRDLCQDPTIKELESIISKRNIQFSCKNIYRPDKFLQCVKNPEDSSCTSEI

SEQ ID NO: 3 - protein, 123 aa, Homo sapiens
QLLFNKTKSVEFTFCNDTVVIPCFVTNMEAQNTTEVYVKWKFKGRDIYTFDGALNKSTVPTDFSSAKIEVSQLLKGDASLKMDKSDAVSHTGNYTCEVTELTREGETIIELKYRVVSWFSPNE

SEQ ID NO: 4 - protein, 4 aa, synthetic construct
AAAS

SEQ ID NO: 5 - protein, 4 aa, synthetic construct
GGGS

SEQ ID NO: 6 - protein, 7 aa, synthetic construct
PPCKCPA

SEQ ID NO: 7 - protein, 10 aa, synthetic construct
PSTCSKPTCP

SEQ ID NO: 8 - protein, 6 aa, synthetic construct
NPCGCT

SEQ ID NO: 9 - protein, 10 aa, synthetic construct
DKTHTCPPCP

SEQ ID NO: 10 - protein, 212 aa, Mus musculus
PEVSSVFIFPPKPKDVLTITLTPKVTCVVVDISKDDPEVQFSWFVDDVEVHTAQTQPREEQFNSTFRSVSELPIMHQDWLNGKEFKCRVNSAAFPAPIEKTISKTKRPKAPQVYTIPPPKEQMAKDKVSLTCMITDFFPEDITVEWQWNGQPAENYKNTQPIMNTNGSYFVYSKLNVQKSNWEAGNTFTCSVLHEGLHNHHTEKSLSHSPGK

SEQ ID NO: 11 - protein, 215 aa, Mus musculus
PNLLGGPSVFIFPPKIKDVLMISLSPIVTCVVVDVSEDDPDVQISWFVNNVEVHTAQTQTHREDYNSTLRVVSALPIQHQDWMSGKEFKCKVNNKDLPAPIERTISKPKSVRAPQVYVLPPPEEEMTKKQVTLTCMVTDFMPEDIYVEWTNNGKTELNYKNTEPVLDSDGSYFMYSKLRVEKKNWVERNSYSCSVVHEGLHNHHTTKSFSRTPGK

SEQ ID NO: 12 - protein, 215 aa, Mus musculus
PDLLGGPSVFIFPPKIKDVLMISLSPMVTCVVVDVSEDDPDVQISWFVNNVEVHTAQTQTHREDYNSTLRVVSALPIQHQDWMSGKEFKCKVNNRALPSPIEKTISKPRPVRAPQVYVLPPPAEEMTKKEFSLTCMITGFLPAEIAVDWTSNGRTEQNYKNTATVLDSDGSYFMYSKLRVQKSTWERGSLFACSVVHEVLHNHLTTKTISRSLGK

SEQ ID NO: 13 - protein, 216 aa, Mus musculus
PDLLGGPSVFIFPPKIKDVLMISLSPMVTCVVVDVSEDDPDVQISWFVNNVEVHTAQTQTHREDYNSTLRVVSALPIQHQDWMSGKEFKCKVNNRALPSPIEKTISKPRGPVRAPQVYVLPPPAEEMTKKEFSLTCMITGFLPAEIAVDWTSNGRTEQNYKNTATVLDSDGSYFMYSKLRVQKSTWERGSLFACSVVHEGLHNHLTTKTISRSLGK

SEQ ID NO: 14 - protein, 215 aa, Lepus americanus
PELLGGPSVFIFPPKPKDTLMISRTPEVTCVVVDVSEDDPEVQFTWYINNEQVRTARPPLREQQFNSTIRVVSTLPIAHEDWLRGKEFKCKVHNKALPAPIEKTISKARQPLEPKVYTMGPPREELSSRSVSLTCMINGFYPSDISVEWEKNGKAEDNYKTTPAVLDSDGSYFLYSKLSVPTSEWQRGDVFTCSVMHEALHNHYTQKSISRSPGK

SEQ ID NO: 15 - protein, 212 aa, Rattus norvegicus
SEVSSVFIFPPKPKDVLTITLTPKVTCVVVDISQDDPEVHFSWFVDDVEVHTAQTRPPEEQFNSTFRSVSELPILHQDWLNGRTFRCKVTSAAFPSPIEKTISKPERTQVPHVYTMSPTKEEMTQNEVSITCMVKGFYPPDIYVEWQMNGQPQENYKNTPPTMDTDGSYFLYSKLNVKKEKWQQGNTFTCSVLHEGLHNHHTEKSLSHSPGK

SEQ ID NO: 16 - protein, 212 aa, Rattus norvegicus
SEVSSVFIFPPKTKDVLTITLTPKVTCVVVDISQNDPEVRFSWFIDDVEVHTAQTHAPEKQSNSTLRSVSELPIVHRDWLNGKTFKCKVNSGAFPAPIEKSISKPETPRGPQVYTMAPPKEEMTQSQVSITCMVKGFYPPDIYTEWKMNGQPQENYKNTPPTMDTDGSYFLYSKLNVKKETWQQGNTFTCSVLHEGLHNHHTEKSLSHSPGK

SEQ ID NO: 17 - protein, 212 aa, Rattus norvegicus; identical to SEQ ID NO: 15

SEQ ID NO: 18 - protein, 215 aa, Rattus norvegicus
DDNLGRPSVFIFPPKPKDILMITLTPKVTCVVVDVSEEEPDVQFSWFVDNVRVFTAQTQPHEEQLNGTFRVVSTLHIQHQDWMSGKEFKCKVNNKDLPSPIEKTISKPRKARTPQVYTIPPPREQMSKNKVSLTCMVTSFYPASISVEWERNGELEQDYKNTLPVLDSDESYFLYSKLSVDTDSWMRGDIYTCSVVHEALHNHHTQKNLSRSPGK

SEQ ID NO: 19 - protein, 483 aa, synthetic construct
MAVPRWRQQWSGPGTTKRFPETVLARCVKYTEIHPEMRHVDCQSVWDAFKGAFISKHPCNITEEDYQPLMKLGTQTVPCNKILLWSRIKDLAHQFTQVQRDMFTLEDTLLGYLADDLTWCGEFNTSKINYQSCPDWRKDCSNNPVSVFWKTVSRRFAEAACDVVHVMLNGSRSKIFDKNSTFGSVEVHNLQPEKVQTLEAWVIHGGREDSRDLCQDPTIKELESIISKRNIQFSCKNIYRPDKFLQCVKNPEDSSCTSEIAAASPPCKCPAPEVSSVFIFPPKPKDVLTITLTPKVTCVVVDISKDDPEVQFSWFVDDVEVHTAQTQPREEQFNSTFRSVSELPIMHQDWLNGKEFKCRVNSAAFPAPIEKTISKTKRPKAPQVYTIPPPKEQMAKDKVSLTCMITDFFPEDITVEWQWNGQPAENYKNTQPIMNTNGSYFVYSKLNVQKSNWEAGNTFTCSVLHEGLHNHHTEKSLSHSPGK

SEQ ID NO: 20 - protein, 483 aa, synthetic construct
MAVPRWRQQWSGPGTTKRFPETVLARCVKYTEIHPEMRHVDCQSVWDAFKGAFISKHPCNITEEDYQPLMKLGTQTVPCNKKLLWSRIKDLAHQFTQVQRDMFTLEDTLLGYLADDLTWCGEFNTSKINYQSCPDWRKDCSNNPVSVFWKTVSRRFAEAACDVVHVMLNGSRSKIFDKNSTFGSVEVHNLQPEKVQTLEAWVIHGGREDSRDLCQDPTIKELESIISKRNIQFSCKNIYRPDKFLQCVKNPEDSSCTSEIAAASPPCKCPAPEVSSVFIFPPKPKDVLTITLTPKVTCVVVDISKDDPEVQFSWFVDDVEVHTAQTQPREEQFNSTFRSVSELPIMHQDWLNGKEFKCRVNSAAFPAPIEKTISKTKRPKAPQVYTIPPPKEQMAKDKVSLTCMITDFFPEDITVEWQWNGQPAENYKNTQPIMNTNGSYFVYSKLNVQKSNWEAGNTFTCSVLHEGLHNHHTEKSLSHSPGK

SEQ ID NO: 21 - protein, 348 aa, synthetic construct
MAQLLFNKTKSVEFTFCNDTVVIPCFVTNMEAQNTTEVYVKWKFKGRDIYTFDGALNKSTVPTDFSSAKIEVSQLLKGDASLKMDKSDAVSHTGNYTCEVTELTREGETIIELKYRVVSWFSPNEAAASPPCKCPAPEVSSVFIFPPKPKDVLTITLTPKVTCVVVDISKDDPEVQFSWFVDDVEVHTAQTQPREEQFNSTFRSVSELPIMHQDWLNGKEFKCRVNSAAFPAPIEKTISKTKRPKAPQVYTIPPPKEQMAKDKVSLTCMITDFFPEDITVEWQWNGQPAENYKNTQPIMNTNGSYFVYSKLNVQKSNWEAGNTFTCSVLHEGLHNHHTEKSLSHSPGK

SEQ ID NO: 22 - protein, 483 aa, synthetic construct
MAVPRWRQQWSGPGTTKRFPETVLARCVKYTEIHPEMRHVDCQSVWDAFKGAFISKHPCNITEEDYQPLMKLGTQTVPCNKILLWSRIKDLAHQFTQVQRDMFTLEDTLLGYLADDLTWCGEFNTSKINYQSCPDWRKDCSNNPVSVFWKTVSRRFAEAACDVVHVMLNGSRSKIFDKNSTFGSVEVHNLQPEKVQTLEAWVIHGGREDSRDLCQDPTIKELESIISKRNIQFSCKNIYRPDKFLQCVKNPEDSSCTSEIGGGSPPCKCPAPEVSSVFIFPPKPKDVLTITLTPKVTCVVVDISKDDPEVQFSWFVDDVEVHTAQTQPREEQFNSTFRSVSELPIMHQDWLNGKEFKCRVNSAAFPAPIEKTISKTKRPKAPQVYTIPPPKEQMAKDKVSLTCMITDFFPEDITVEWQWNGQPAENYKNTQPIMNTNGSYFVYSKLNVQKSNWEAGNTFTCSVLHEGLHNHHTEKSLSHSPGK

SEQ ID NO: 23 - protein, 483 aa, synthetic construct
MAVPRWRQQWSGPGTTKRFPETVLARCVKYTEIHPEMRHVDCQSVWDAFKGAFISKHPCNITEEDYQPLMKLGTQTVPCNKKLLWSRIKDLAHQFTQVQRDMFTLEDTLLGYLADDLTWCGEFNTSKINYQSCPDWRKDCSNNPVSVFWKTVSRRFAEAACDVVHVMLNGSRSKIFDKNSTFGSVEVHNLQPEKVQTLEAWVIHGGREDSRDLCQDPTIKELESIISKRNIQFSCKNIYRPDKFLQCVKNPEDSSCTSEIGGGSPPCKCPAPEVSSVFIFPPKPKDVLTITLTPKVTCVVVDISKDDPEVQFSWFVDDVEVHTAQTQPREEQFNSTFRSVSELPIMHQDWLNGKEFKCRVNSAAFPAPIEKTISKTKRPKAPQVYTIPPPKEQMAKDKVSLTCMITDFFPEDITVEWQWNGQPAENYKNTQPIMNTNGSYFVYSKLNVQKSNWEAGNTFTCSVLHEGLHNHHTEKSLSHSPGK

SEQ ID NO: 24 - protein, 348 aa, synthetic construct
MAQLLFNKTKSVEFTFCNDTVVIPCFVTNMEAQNTTEVYVKWKFKGRDIYTFDGALNKSTVPTDFSSAKIEVSQLLKGDASLKMDKSDAVSHTGNYTCEVTELTREGETIIELKYRVVSWFSPNEGGGSPPCKCPAPEVSSVFIFPPKPKDVLTITLTPKVTCVVVDISKDDPEVQFSWFVDDVEVHTAQTQPREEQFNSTFRSVSELPIMHQDWLNGKEFKCRVNSAAFPAPIEKTISKTKRPKAPQVYTIPPPKEQMAKDKVSLTCMITDFFPEDITVEWQWNGQPAENYKNTQPIMNTNGSYFVYSKLNVQKSNWEAGNTFTCSVLHEGLHNHHTEKSLSHSPGK

SEQ ID NO: 25 - protein, 479 aa, synthetic construct
MAVPRWRQQWSGPGTTKRFPETVLARCVKYTEIHPEMRHVDCQSVWDAFKGAFISKHPCNITEEDYQPLMKLGTQTVPCNKILLWSRIKDLAHQFTQVQRDMFTLEDTLLGYLADDLTWCGEFNTSKINYQSCPDWRKDCSNNPVSVFWKTVSRRFAEAACDVVHVMLNGSRSKIFDKNSTFGSVEVHNLQPEKVQTLEAWVIHGGREDSRDLCQDPTIKELESIISKRNIQFSCKNIYRPDKFLQCVKNPEDSSCTSEIPPCKCPAPEVSSVFIFPPKPKDVLTITLTPKVTCVVVDISKDDPEVQFSWFVDDVEVHTAQTQPREEQFNSTFRSVSELPIMHQDWLNGKEFKCRVNSAAFPAPIEKTISKTKRPKAPQVYTIPPPKEQMAKDKVSLTCMITDFFPEDITVEWQWNGQPAENYKNTQPIMNTNGSYFVYSKLNVQKSNWEAGNTFTCSVLHEGLHNHHTEKSLSHSPGK

SEQ ID NO: 26 - protein, 479 aa, synthetic construct
MAVPRWRQQWSGPGTTKRFPETVLARCVKYTEIHPEMRHVDCQSVWDAFKGAFISKHPCNITEEDYQPLMKLGTQTVPCNKKLLWSRIKDLAHQFTQVQRDMFTLEDTLLGYLADDLTWCGEFNTSKINYQSCPDWRKDCSNNPVSVFWKTVSRRFAEAACDVVHVMLNGSRSKIFDKNSTFGSVEVHNLQPEKVQTLEAWVIHGGREDSRDLCQDPTIKELESIISKRNIQFSCKNIYRPDKFLQCVKNPEDSSCTSEIPPCKCPAPEVSSVFIFPPKPKDVLTITLTPKVTCVVVDISKDDPEVQFSWFVDDVEVHTAQTQPREEQFNSTFRSVSELPIMHQDWLNGKEFKCRVNSAAFPAPIEKTISKTKRPKAPQVYTIPPPKEQMAKDKVSLTCMITDFFPEDITVEWQWNGQPAENYKNTQPIMNTNGSYFVYSKLNVQKSNWEAGNTFTCSVLHEGLHNHHTEKSLSHSPGK

SEQ ID NO: 27 - protein, 344 aa, synthetic construct
MAQLLFNKTKSVEFTFCNDTVVIPCFVTNMEAQNTTEVYVKWKFKGRDIYTFDGALNKSTVPTDFSSAKIEVSQLLKGDASLKMDKSDAVSHTGNYTCEVTELTREGETIIELKYRVVSWFSPNEPPCKCPAPEVSSVFIFPPKPKDVLTITLTPKVTCVVVDISKDDPEVQFSWFVDDVEVHTAQTQPREEQFNSTFRSVSELPIMHQDWLNGKEFKCRVNSAAFPAPIEKTISKTKRPKAPQVYTIPPPKEQMAKDKVSLTCMITDFFPEDITVEWQWNGQPAENYKNTQPIMNTNGSYFVYSKLNVQKSNWEAGNTFTCSVLHEGLHNHHTEKSLSHSPGK

SEQ ID NO: 28 - protein, 486 aa, synthetic construct
MAVPRWRQQWSGPGTTKRFPETVLARCVKYTEIHPEMRHVDCQSVWDAFKGAFISKHPCNITEEDYQPLMKLGTQTVPCNKILLWSRIKDLAHQFTQVQRDMFTLEDTLLGYLADDLTWCGEFNTSKINYQSCPDWRKDCSNNPVSVFWKTVSRRFAEAACDVVHVMLNGSRSKIFDKNSTFGSVEVHNLQPEKVQTLEAWVIHGGREDSRDLCQDPTIKELESIISKRNIQFSCKNIYRPDKFLQCVKNPEDSSCTSEIAAASPSTCSKPTCPPEVSSVFIFPPKPKDVLTITLTPKVTCVVVDISKDDPEVQFSWFVDDVEVHTAQTQPREEQFNSTFRSVSELPIMHQDWLNGKEFKCRVNSAAFPAPIEKTISKTKRPKAPQVYTIPPPKEQMAKDKVSLTCMITDFFPEDITVEWQWNGQPAENYKNTQPIMNTNGSYFVYSKLNVQKSNWEAGNTFTCSVLHEGLHNHHTEKSLSHSPGK

SEQ ID NO: 29 - protein, 486 aa, synthetic construct
MAVPRWRQQWSGPGTTKRFPETVLARCVKYTEIHPEMRHVDCQSVWDAFKGAFISKHPCNITEEDYQPLMKLGTQTVPCNKKLLWSRIKDLAHQFTQVQRDMFTLEDTLLGYLADDLTWCGEFNTSKINYQSCPDWRKDCSNNPVSVFWKTVSRRFAEAACDVVHVMLNGSRSKIFDKNSTFGSVEVHNLQPEKVQTLEAWVIHGGREDSRDLCQDPTIKELESIISKRNIQFSCKNIYRPDKFLQCVKNPEDSSCTSEIAAASPSTCSKPTCPPEVSSVFIFPPKPKDVLTITLTPKVTCVVVDISKDDPEVQFSWFVDDVEVHTAQTQPREEQFNSTFRSVSELPIMHQDWLNGKEFKCRVNSAAFPAPIEKTISKTKRPKAPQVYTIPPPKEQMAKDKVSLTCMITDFFPEDITVEWQWNGQPAENYKNTQPIMNTNGSYFVYSKLNVQKSNWEAGNTFTCSVLHEGLHNHHTEKSLSHSPGK

SEQ ID NO: 30 - protein, 351 aa, synthetic construct
MAQLLFNKTKSVEFTFCNDTVVIPCFVTNMEAQNTTEVYVKWKFKGRDIYTFDGALNKSTVPTDFSSAKIEVSQLLKGDASLKMDKSDAVSHTGNYTCEVTELTREGETIIELKYRVVSWFSPNEAAASPSTCSKPTCPPEVSSVFIFPPKPKDVLTITLTPKVTCVVVDISKDDPEVQFSWFVDDVEVHTAQTQPREEQFNSTFRSVSELPIMHQDWLNGKEFKCRVNSAAFPAPIEKTISKTKRPKAPQVYTIPPPKEQMAKDKVSLTCMITDFFPEDITVEWQWNGQPAENYKNTQPIMNTNGSYFVYSKLNVQKSNWEAGNTFTCSVLHEGLHNHHTEKSLSHSPGK

SEQ ID NO: 31 - protein, 486 aa, synthetic construct
MAVPRWRQQWSGPGTTKRFPETVLARCVKYTEIHPEMRHVDCQSVWDAFKGAFISKHPCNITEEDYQPLMKLGTQTVPCNKILLWSRIKDLAHQFTQVQRDMFTLEDTLLGYLADDLTWCGEFNTSKINYQSCPDWRKDCSNNPVSVFWKTVSRRFAEAACDVVHVMLNGSRSKIFDKNSTFGSVEVHNLQPEKVQTLEAWVIHGGREDSRDLCQDPTIKELESIISKRNIQFSCKNIYRPDKFLQCVKNPEDSSCTSEIGGGSPSTCSKPTCPPEVSSVFIFPPKPKDVLTITLTPKVTCVVVDISKDDPEVQFSWFVDDVEVHTAQTQPREEQFNSTFRSVSELPIMHQDWLNGKEFKCRVNSAAFPAPIEKTISKTKRPKAPQVYTIPPPKEQMAKDKVSLTCMITDFFPEDITVEWQWNGQPAENYKNTQPIMNTNGSYFVYSKLNVQKSNWEAGNTFTCSVLHEGLHNHHTEKSLSHSPGK

SEQ ID NO: 32 - protein, 486 aa, synthetic construct
MAVPRWRQQWSGPGTTKRFPETVLARCVKYTEIHPEMRHVDCQSVWDAFKGAFISKHPCNITEEDYQPLMKLGTQTVPCNKKLLWSRIKDLAHQFTQVQRDMFTLEDTLLGYLADDLTWCGEFNTSKINYQSCPDWRKDCSNNPVSVFWKTVSRRFAEAACDVVHVMLNGSRSKIFDKNSTFGSVEVHNLQPEKVQTLEAWVIHGGREDSRDLCQDPTIKELESIISKRNIQFSCKNIYRPDKFLQCVKNPEDSSCTSEIGGGSPSTCSKPTCPPEVSSVFIFPPKPKDVLTITLTPKVTCVVVDISKDDPEVQFSWFVDDVEVHTAQTQPREEQFNSTFRSVSELPIMHQDWLNGKEFKCRVNSAAFPAPIEKTISKTKRPKAPQVYTIPPPKEQMAKDKVSLTCMITDFFPEDITVEWQWNGQPAENYKNTQPIMNTNGSYFVYSKLNVQKSNWEAGNTFTCSVLHEGLHNHHTEKSLSHSPGK

SEQ ID NO: 33 - protein, 351 aa, synthetic construct
MAQLLFNKTKSVEFTFCNDTVVIPCFVTNMEAQNTTEVYVKWKFKGRDIYTFDGALNKSTVPTDFSSAKIEVSQLLKGDASLKMDKSDAVSHTGNYTCEVTELTREGETIIELKYRVVSWFSPNEGGGSPSTCSKPTCPPEVSSVFIFPPKPKDVLTITLTPKVTCVVVDISKDDPEVQFSWFVDDVEVHTAQTQPREEQFNSTFRSVSELPIMHQDWLNGKEFKCRVNSAAFPAPIEKTISKTKRPKAPQVYTIPPPKEQMAKDKVSLTCMITDFFPEDITVEWQWNGQPAENYKNTQPIMNTNGSYFVYSKLNVQKSNWEAGNTFTCSVLHEGLHNHHTEKSLSHSPGK

SEQ ID NO: 34 - protein, 482 aa, synthetic construct
MAVPRWRQQWSGPGTTKRFPETVLARCVKYTEIHPEMRHVDCQSVWDAFKGAFISKHPCNITEEDYQPLMKLGTQTVPCNKILLWSRIKDLAHQFTQVQRDMFTLEDTLLGYLADDLTWCGEFNTSKINYQSCPDWRKDCSNNPVSVFWKTVSRRFAEAACDVVHVMLNGSRSKIFDKNSTFGSVEVHNLQPEKVQTLEAWVIHGGREDSRDLCQDPTIKELESIISKRNIQFSCKNIYRPDKFLQCVKNPEDSSCTSEIPSTCSKPTCPPEVSSVFIFPPKPKDVLTITLTPKVTCVVVDISKDDPEVQFSWFVDDVEVHTAQTQPREEQFNSTFRSVSELPIMHQDWLNGKEFKCRVNSAAFPAPIEKTISKTKRPKAPQVYTIPPPKEQMAKDKVSLTCMITDFFPEDITVEWQWNGQPAENYKNTQPIMNTNGSYFVYSKLNVQKSNWEAGNTFTCSVLHEGLHNHHTEKSLSHSPGK

SEQ ID NO: 35 - protein, 482 aa, synthetic construct
MAVPRWRQQWSGPGTTKRFPETVLARCVKYTEIHPEMRHVDCQSVWDAFKGAFISKHPCNITEEDYQPLMKLGTQTVPCNKKLLWSRIKDLAHQFTQVQRDMFTLEDTLLGYLADDLTWCGEFNTSKINYQSCPDWRKDCSNNPVSVFWKTVSRRFAEAACDVVHVMLNGSRSKIFDKNSTFGSVEVHNLQPEKVQTLEAWVIHGGREDSRDLCQDPTIKELESIISKRNIQFSCKNIYRPDKFLQCVKNPEDSSCTSEIPSTCSKPTCPPEVSSVFIFPPKPKDVLTITLTPKVTCVVVDISKDDPEVQFSWFVDDVEVHTAQTQPREEQFNSTFRSVSELPIMHQDWLNGKEFKCRVNSAAFPAPIEKTISKTKRPKAPQVYTIPPPKEQMAKDKVSLTCMITDFFPEDITVEWQWNGQPAENYKNTQPIMNTNGSYFVYSKLNVQKSNWEAGNTFTCSVLHEGLHNHHTEKSLSHSPGK

SEQ ID NO: 36 - protein, 347 aa, synthetic construct
MAQLLFNKTKSVEFTFCNDTVVIPCFVTNMEAQNTTEVYVKWKFKGRDIYTFDGALNKSTVPTDFSSAKIEVSQLLKGDASLKMDKSDAVSHTGNYTCEVTELTREGETIIELKYRVVSWFSPNEPSTCSKPTCPPEVSSVFIFPPKPKDVLTITLTPKVTCVVVDISKDDPEVQFSWFVDDVEVHTAQTQPREEQFNSTFRSVSELPIMHQDWLNGKEFKCRVNSAAFPAPIEKTISKTKRPKAPQVYTIPPPKEQMAKDKVSLTCMITDFFPEDITVEWQWNGQPAENYKNTQPIMNTNGSYFVYSKLNVQKSNWEAGNTFTCSVLHEGLHNHHTEKSLSHSPGK

SEQ ID NO: 37 - protein, 482 aa, synthetic construct
MAVPRWRQQWSGPGTTKRFPETVLARCVKYTEIHPEMRHVDCQSVWDAFKGAFISKHPCNITEEDYQPLMKLGTQTVPCNKILLWSRIKDLAHQFTQVQRDMFTLEDTLLGYLADDLTWCGEFNTSKINYQSCPDWRKDCSNNPVSVFWKTVSRRFAEAACDVVHVMLNGSRSKIFDKNSTFGSVEVHNLQPEKVQTLEAWVIHGGREDSRDLCQDPTIKELESIISKRNIQFSCKNIYRPDKFLQCVKNPEDSSCTSEIAAASNPCGCTPEVSSVFIFPPKPKDVLTITLTPKVTCVVVDISKDDPEVQFSWFVDDVEVHTAQTQPREEQFNSTFRSVSELPIMHQDWLNGKEFKCRVNSAAFPAPIEKTISKTKRPKAPQVYTIPPPKEQMAKDKVSLTCMITDFFPEDITVEWQWNGQPAENYKNTQPIMNTNGSYFVYSKLNVQKSNWEAGNTFTCSVLHEGLHNHHTEKSLSHSPGK

SEQ ID NO: 38 - protein, 482 aa, synthetic construct
MAVPRWRQQWSGPGTTKRFPETVLARCVKYTEIHPEMRHVDCQSVWDAFKGAFISKHPCNITEEDYQPLMKLGTQTVPCNKKLLWSRIKDLAHQFTQVQRDMFTLEDTLLGYLADDLTWCGEFNTSKINYQSCPDWRKDCSNNPVSVFWKTVSRRFAEAACDVVHVMLNGSRSKIFDKNSTFGSVEVHNLQPEKVQTLEAWVIHGGREDSRDLCQDPTIKELESIISKRNIQFSCKNIYRPDKFLQCVKNPEDSSCTSEIAAASNPCGCTPEVSSVFIFPPKPKDVLTITLTPKVTCVVVDISKDDPEVQFSWFVDDVEVHTAQTQPREEQFNSTFRSVSELPIMHQDWLNGKEFKCRVNSAAFPAPIEKTISKTKRPKAPQVYTIPPPKEQMAKDKVSLTCMITDFFPEDITVEWQWNGQPAENYKNTQPIMNTNGSYFVYSKLNVQKSNWEAGNTFTCSVLHEGLHNHHTEKSLSHSPGK

SEQ ID NO: 39 - protein, 347 aa, synthetic construct
MAQLLFNKTKSVEFTFCNDTVVIPCFVTNMEAQNTTEVYVKWKFKGRDIYTFDGALNKSTVPTDFSSAKIEVSQLLKGDASLKMDKSDAVSHTGNYTCEVTELTREGETIIELKYRVVSWFSPNEAAASNPCGCTPEVSSVFIFPPKPKDVLTITLTPKVTCVVVDISKDDPEVQFSWFVDDVEVHTAQTQPREEQFNSTFRSVSELPIMHQDWLNGKEFKCRVNSAAFPAPIEKTISKTKRPKAPQVYTIPPPKEQMAKDKVSLTCMITDFFPEDITVEWQWNGQPAENYKNTQPIMNTNGSYFVYSKLNVQKSNWEAGNTFTCSVLHEGLHNHHTEKSLSHSPGK

SEQ ID NO: 40 - protein, 482 aa, synthetic construct
MAVPRWRQQWSGPGTTKRFPETVLARCVKYTEIHPEMRHVDCQSVWDAFKGAFISKHPCNITEEDYQPLMKLGTQTVPCNKILLWSRIKDLAHQFTQVQRDMFTLEDTLLGYLADDLTWCGEFNTSKINYQSCPDWRKDCSNNPVSVFWKTVSRRFAEAACDVVHVMLNGSRSKIFDKNSTFGSVEVHNLQPEKVQTLEAWVIHGGREDSRDLCQDPTIKELESIISKRNIQFSCKNIYRPDKFLQCVKNPEDSSCTSEIGGGSNPCGCTPEVSSVFIFPPKPKDVLTITLTPKVTCVVVDISKDDPEVQFSWFVDDVEVHTAQTQPREEQFNSTFRSVSELPIMHQDWLNGKEFKCRVNSAAFPAPIEKTISKTKRPKAPQVYTIPPPKEQMAKDKVSLTCMITDFFPEDITVEWQWNGQPAENYKNTQPIMNTNGSYFVYSKLNVQKSNWEAGNTFTCSVLHEGLHNHHTEKSLSHSPGK

SEQ ID NO: 41 - protein, 482 aa, synthetic construct
MAVPRWRQQWSGPGTTKRFPETVLARCVKYTEIHPEMRHVDCQSVWDAFKGAFISKHPCNITEEDYQPLMKLGTQTVPCNKKLLWSRIKDLAHQFTQVQRDMFTLEDTLLGYLADDLTWCGEFNTSKINYQSCPDWRKDCSNNPVSVFWKTVSRRFAEAACDVVHVMLNGSRSKIFDKNSTFGSVEVHNLQPEKVQTLEAWVIHGGREDSRDLCQDPTIKELESIISKRNIQFSCKNIYRPDKFLQCVKNPEDSSCTSEIGGGSNPCGCTPEVSSVFIFPPKPKDVLTITLTPKVTCVVVDISKDDPEVQFSWFVDDVEVHTAQTQPREEQFNSTFRSVSELPIMHQDWLNGKEFKCRVNSAAFPAPIEKTISKTKRPKAPQVYTIPPPKEQMAKDKVSLTCMITDFFPEDITVEWQWNGQPAENYKNTQPIMNTNGSYFVYSKLNVQKSNWEAGNTFTCSVLHEGLHNHHTEKSLSHSPGK

SEQ ID NO: 42 - protein, 347 aa, synthetic construct
MAQLLFNKTKSVEFTFCNDTVVIPCFVTNMEAQNTTEVYVKWKFKGRDIYTFDGALNKSTVPTDFSSAKIEVSQLLKGDASLKMDKSDAVSHTGNYTCEVTELTREGETIIELKYRVVSWFSPNEGGGSNPCGCTPEVSSVFIFPPKPKDVLTITLTPKVTCVVVDISKDDPEVQFSWFVDDVEVHTAQTQPREEQFNSTFRSVSELPIMHQDWLNGKEFKCRVNSAAFPAPIEKTISKTKRPKAPQVYTIPPPKEQMAKDKVSLTCMITDFFPEDITVEWQWNGQPAENYKNTQPIMNTNGSYFVYSKLNVQKSNWEAGNTFTCSVLHEGLHNHHTEKSLSHSPGK

SEQ ID NO: 43 - protein, 478 aa, synthetic construct
MAVPRWRQQWSGPGTTKRFPETVLARCVKYTEIHPEMRHVDCQSVWDAFKGAFISKHPCNITEEDYQPLMKLGTQTVPCNKILLWSRIKDLAHQFTQVQRDMFTLEDTLLGYLADDLTWCGEFNTSKINYQSCPDWRKDCSNNPVSVFWKTVSRRFAEAACDVVHVMLNGSRSKIFDKNSTFGSVEVHNLQPEKVQTLEAWVIHGGREDSRDLCQDPTIKELESIISKRNIQFSCKNIYRPDKFLQCVKNPEDSSCTSEINPCGCTPEVSSVFIFPPKPKDVLTITLTPKVTCVVVDISKDDPEVQFSWFVDDVEVHTAQTQPREEQFNSTFRSVSELPIMHQDWLNGKEFKCRVNSAAFPAPIEKTISKTKRPKAPQVYTIPPPKEQMAKDKVSLTCMITDFFPEDITVEWQWNGQPAENYKNTQPIMNTNGSYFVYSKLNVQKSNWEAGNTFTCSVLHEGLHNHHTEKSLSHSPGK

SEQ ID NO: 44 - protein, 478 aa, synthetic construct
MAVPRWRQQWSGPGTTKRFPETVLARCVKYTEIHPEMRHVDCQSVWDAFKGAFISKHPCNITEEDYQPLMKLGTQTVPCNKKLLWSRIKDLAHQFTQVQRDMFTLEDTLLGYLADDLTWCGEFNTSKINYQSCPDWRKDCSNNPVSVFWKTVSRRFAEAACDVVHVMLNGSRSKIFDKNSTFGSVEVHNLQPEKVQTLEAWVIHGGREDSRDLCQDPTIKELESIISKRNIQFSCKNIYRPDKFLQCVKNPEDSSCTSEINPCGCTPEVSSVFIFPPKPKDVLTITLTPKVTCVVVDISKDDPEVQFSWFVDDVEVHTAQTQPREEQFNSTFRSVSELPIMHQDWLNGKEFKCRVNSAAFPAPIEKTISKTKRPKAPQVYTIPPPKEQMAKDKVSLTCMITDFFPEDITVEWQWNGQPAENYKNTQPIMNTNGSYFVYSKLNVQKSNWEAGNTFTCSVLHEGLHNHHTEKSLSHSPGK

SEQ ID NO: 45 - protein, 343 aa, synthetic construct
MAQLLFNKTKSVEFTFCNDTVVIPCFVTNMEAQNTTEVYVKWKFKGRDIYTFDGALNKSTVPTDFSSAKIEVSQLLKGDASLKMDKSDAVSHTGNYTCEVTELTREGETIIELKYRVVSWFSPNENPCGCTPEVSSVFIFPPKPKDVLTITLTPKVTCVVVDISKDDPEVQFSWFVDDVEVHTAQTQPREEQFNSTFRSVSELPIMHQDWLNGKEFKCRVNSAAFPAPIEKTISKTKRPKAPQVYTIPPPKEQMAKDKVSLTCMITDFFPEDITVEWQWNGQPAENYKNTQPIMNTNGSYFVYSKLNVQKSNWEAGNTFTCSVLHEGLHNHHTEKSLSHSPGK

SEQ ID NO: 46 - protein, 486 aa, synthetic construct
MAVPRWRQQWSGPGTTKRFPETVLARCVKYTEIHPEMRHVDCQSVWDAFKGAFISKHPCNITEEDYQPLMKLGTQTVPCNKILLWSRIKDLAHQFTQVQRDMFTLEDTLLGYLADDLTWCGEFNTSKINYQSCPDWRKDCSNNPVSVFWKTVSRRFAEAACDVVHVMLNGSRSKIFDKNSTFGSVEVHNLQPEKVQTLEAWVIHGGREDSRDLCQDPTIKELESIISKRNIQFSCKNIYRPDKFLQCVKNPEDSSCTSEIAAASDKTHTCPPCPPEVSSVFIFPPKPKDVLTITLTPKVTCVVVDISKDDPEVQFSWFVDDVEVHTAQTQPREEQFNSTFRSVSELPIMHQDWLNGKEFKCRVNSAAFPAPIEKTISKTKRPKAPQVYTIPPPKEQMAKDKVSLTCMITDFFPEDITVEWQWNGQPAENYKNTQPIMNTNGSYFVYSKLNVQKSNWEAGNTFTCSVLHEGLHNHHTEKSLSHSPGK

SEQ ID NO: 47 - protein, 486 aa, synthetic construct
MAVPRWRQQWSGPGTTKRFPETVLARCVKYTEIHPEMRHVDCQSVWDAFKGAFISKHPCNITEEDYQPLMKLGTQTVPCNKKLLWSRIKDLAHQFTQVQRDMFTLEDTLLGYLADDLTWCGEFNTSKINYQSCPDWRKDCSNNPVSVFWKTVSRRFAEAACDVVHVMLNGSRSKIFDKNSTFGSVEVHNLQPEKVQTLEAWVIHGGREDSRDLCQDPTIKELESIISKRNIQFSCKNIYRPDKFLQCVKNPEDSSCTSEIAAASDKTHTCPPCPPEVSSVFIFPPKPKDVLTITLTPKVTCVVVDISKDDPEVQFSWFVDDVEVHTAQTQPREEQFNSTFRSVSELPIMHQDWLNGKEFKCRVNSAAFPAPIEKTISKTKRPKAPQVYTIPPPKEQMAKDKVSLTCMITDFFPEDITVEWQWNGQPAENYKNTQPIMNTNGSYFVYSKLNVQKSNWEAGNTFTCSVLHEGLHNHHTEKSLSHSPGK

SEQ ID NO: 48 - protein, 351 aa, synthetic construct
MAQLLFNKTKSVEFTFCNDTVVIPCFVTNMEAQNTTEVYVKWKFKGRDIYTFDGALNKSTVPTDFSSAKIEVSQLLKGDASLKMDKSDAVSHTGNYTCEVTELTREGETIIELKYRVVSWFSPNEAAASDKTHTCPPCPPEVSSVFIFPPKPKDVLTITLTPKVTCVVVDISKDDPEVQFSWFVDDVEVHTAQTQPREEQFNSTFRSVSELPIMHQDWLNGKEFKCRVNSAAFPAPIEKTISKTKRPKAPQVYTIPPPKEQMAKDKVSLTCMITDFFPEDITVEWQWNGQPAENYKNTQPIMNTNGSYFVYSKLNVQKSNWEAGNTFTCSVLHEGLHNHHTEKSLSHSPGK

SEQ ID NO: 49 - protein, 486 aa, synthetic construct
MAVPRWRQQWSGPGTTKRFPETVLARCVKYTEIHPEMRHVDCQSVWDAFKGAFISKHPCNITEEDYQPLMKLGTQTVPCNKILLWSRIKDLAHQFTQVQRDMFTLEDTLLGYLADDLTWCGEFNTSKINYQSCPDWRKDCSNNPVSVFWKTVSRRFAEAACDVVHVMLNGSRSKIFDKNSTFGSVEVHNLQPEKVQTLEAWVIHGGREDSRDLCQDPTIKELESIISKRNIQFSCKNIYRPDKFLQCVKNPEDSSCTSEIGGGSDKTHTCPPCPPEVSSVFIFPPKPKDVLTITLTPKVTCVVVDISKDDPEVQFSWFVDDVEVHTAQTQPREEQFNSTFRSVSELPIMHQDWLNGKEFKCRVNSAAFPAPIEKTISKTKRPKAPQVYTIPPPKEQMAKDKVSLTCMITDFFPEDITVEWQWNGQPAENYKNTQPIMNTNGSYFVYSKLNVQKSNWEAGNTFTCSVLHEGLHNHHTEKSLSHSPGK

SEQ ID NO: 50 - protein, 486 aa, synthetic construct
MAVPRWRQQWSGPGTTKRFPETVLARCVKYTEIHPEMRHVDCQSVWDAFKGAFISKHPCNITEEDYQPLMKLGTQTVPCNKKLLWSRIKDLAHQFTQVQRDMFTLEDTLLGYLADDLTWCGEFNTSKINYQSCPDWRKDCSNNPVSVFWKTVSRRFAEAACDVVHVMLNGSRSKIFDKNSTFGSVEVHNLQPEKVQTLEAWVIHGGREDSRDLCQDPTIKELESIISKRNIQFSCKNIYRPDKFLQCVKNPEDSSCTSEIGGGSDKTHTCPPCPPEVSSVFIFPPKPKDVLTITLTPKVTCVVVDISKDDPEVQFSWFVDDVEVHTAQTQPREEQFNSTFRSVSELPIMHQDWLNGKEFKCRVNSAAFPAPIEKTISKTKRPKAPQVYTIPPPKEQMAKDKVSLTCMITDFFPEDITVEWQWNGQPAENYKNTQPIMNTNGSYFVYSKLNVQKSNWEAGNTFTCSVLHEGLHNHHTEKSLSHSPGK

SEQ ID NO: 51 - protein, 351 aa, synthetic construct
MAQLLFNKTKSVEFTFCNDTVVIPCFVTNMEAQNTTEVYVKWKFKGRDIYTFDGALNKSTVPTDFSSAKIEVSQLLKGDASLKMDKSDAVSHTGNYTCEVTELTREGETIIELKYRVVSWFSPNEGGGSDKTHTCPPCPPEVSSVFIFPPKPKDVLTITLTPKVTCVVVDISKDDPEVQFSWFVDDVEVHTAQTQPREEQFNSTFRSVSELPIMHQDWLNGKEFKCRVNSAAFPAPIEKTISKTKRPKAPQVYTIPPPKEQMAKDKVSLTCMITDFFPEDITVEWQWNGQPAENYKNTQPIMNTNGSYFVYSKLNVQKSNWEAGNTFTCSVLHEGLHNHHTEKSLSHSPGK

SEQ ID NO: 52 - protein, 482 aa, synthetic construct
MAVPRWRQQWSGPGTTKRFPETVLARCVKYTEIHPEMRHVDCQSVWDAFKGAFISKHPCNITEEDYQPLMKLGTQTVPCNKILLWSRIKDLAHQFTQVQRDMFTLEDTLLGYLADDLTWCGEFNTSKINYQSCPDWRKDCSNNPVSVFWKTVSRRFAEAACDVVHVMLNGSRSKIFDKNSTFGSVEVHNLQPEKVQTLEAWVIHGGREDSRDLCQDPTIKELESIISKRNIQFSCKNIYRPDKFLQCVKNPEDSSCTSEIDKTHTCPPCPPEVSSVFIFPPKPKDVLTITLTPKVTCVVVDISKDDPEVQFSWFVDDVEVHTAQTQPREEQFNSTFRSVSELPIMHQDWLNGKEFKCRVNSAAFPAPIEKTISKTKRPKAPQVYTIPPPKEQMAKDKVSLTCMITDFFPEDITVEWQWNGQPAENYKNTQPIMNTNGSYFVYSKLNVQKSNWEAGNTFTCSVLHEGLHNHHTEKSLSHSPGK

SEQ ID NO: 53 - protein, 482 aa, synthetic construct
MAVPRWRQQWSGPGTTKRFPETVLARCVKYTEIHPEMRHVDCQSVWDAFKGAFISKHPCNITEEDYQPLMKLGTQTVPCNKKLLWSRIKDLAHQFTQVQRDMFTLEDTLLGYLADDLTWCGEFNTSKINYQSCPDWRKDCSNNPVSVFWKTVSRRFAEAACDVVHVMLNGSRSKIFDKNSTFGSVEVHNLQPEKVQTLEAWVIHGGREDSRDLCQDPTIKELESIISKRNIQFSCKNIYRPDKFLQCVKNPEDSSCTSEIDKTHTCPPCPPEVSSVFIFPPKPKDVLTITLTPKVTCVVVDISKDDPEVQFSWFVDDVEVHTAQTQPREEQFNSTFRSVSELPIMHQDWLNGKEFKCRVNSAAFPAPIEKTISKTKRPKAPQVYTIPPPKEQMAKDKVSLTCMITDFFPEDITVEWQWNGQPAENYKNTQPIMNTNGSYFVYSKLNVQKSNWEAGNTFTCSVLHEGLHNHHTEKSLSHSPGK

SEQ ID NO: 54 - protein, 347 aa, synthetic construct
MAQLLFNKTKSVEFTFCNDTVVIPCFVTNMEAQNTTEVYVKWKFKGRDIYTFDGALNKSTVPTDFSSAKIEVSQLLKGDASLKMDKSDAVSHTGNYTCEVTELTREGETIIELKYRVVSWFSPNEDKTHTCPPCPPEVSSVFIFPPKPKDVLTITLTPKVTCVVVDISKDDPEVQFSWFVDDVEVHTAQTQPREEQFNSTFRSVSELPIMHQDWLNGKEFKCRVNSAAFPAPIEKTISKTKRPKAPQVYTIPPPKEQMAKDKVSLTCMITDFFPEDITVEWQWNGQPAENYKNTQPIMNTNGSYFVYSKLNVQKSNWEAGNTFTCSVLHEGLHNHHTEKSLSHSPGK

SEQ ID NO: 55 - protein, 486 aa, synthetic construct
MAVPRWRQQWSGPGTTKRFPETVLARCVKYTEIHPEMRHVDCQSVWDAFKGAFISKHPCNITEEDYQPLMKLGTQTVPCNKILLWSRIKDLAHQFTQVQRDMFTLEDTLLGYLADDLTWCGEFNTSKINYQSCPDWRKDCSNNPVSVFWKTVSRRFAEAACDVVHVMLNGSRSKIFDKNSTFGSVEVHNLQPEKVQTLEAWVIHGGREDSRDLCQDPTIKELESIISKRNIQFSCKNIYRPDKFLQCVKNPEDSSCTSEIAAASPPCKCPAPNLLGGPSVFIFPPKIKDVLMISLSPIVTCVVVDVSEDDPDVQISWFVNNVEVHTAQTQTHREDYNSTLRVVSALPIQHQDWMSGKEFKCKVNNKDLPAPIERTISKPKSVRAPQVYVLPPPEEEMTKKQVTLTCMVTDFMPEDIYVEWTNNGKTELNYKNTEPVLDSDGSYFMYSKLRVEKKNWVERNSYSCSVVHEGLHNHHTTKSFSRTPGK

SEQ ID NO: 56 - protein, 486 aa, synthetic construct
MAVPRWRQQWSGPGTTKRFPETVLARCVKYTEIHPEMRHVDCQSVWDAFKGAFISKHPCNITEEDYQPLMKLGTQTVPCNKKLLWSRIKDLAHQFTQVQRDMFTLEDTLLGYLADDLTWCGEFNTSKINYQSCPDWRKDCSNNPVSVFWKTVSRRFAEAACDVVHVMLNGSRSKIFDKNSTFGSVEVHNLQPEKVQTLEAWVIHGGREDSRDLCQDPTIKELESIISKRNIQFSCKNIYRPDKFLQCVKNPEDSSCTSEIAAASPPCKCPAPNLLGGPSVFIFPPKIKDVLMISLSPIVTCVVVDVSEDDPDVQISWFVNNVEVHTAQTQTHREDYNSTLRVVSALPIQHQDWMSGKEFKCKVNNKDLPAPIERTISKPKSVRAPQVYVLPPPEEEMTKKQVTLTCMVTDFMPEDIYVEWTNNGKTELNYKNTEPVLDSDGSYFMYSKLRVEKKNWVERNSYSCSVVHEGLHNHHTTKSFSRTPGK

SEQ ID NO: 57 - protein, 351 aa, synthetic construct
MAQLLFNKTKSVEFTFCNDTVVIPCFVTNMEAQNTTEVYVKWKFKGRDIYTFDGALNKSTVPTDFSSAKIEVSQLLKGDASLKMDKSDAVSHTGNYTCEVTELTREGETIIELKYRVVSWFSPNEAAASPPCKCPAPNLLGGPSVFIFPPKIKDVLMISLSPIVTCVVVDVSEDDPDVQISWFVNNVEVHTAQTQTHREDYNSTLRVVSALPIQHQDWMSGKEFKCKVNNKDLPAPIERTISKPKSVRAPQVYVLPPPEEEMTKKQVTLTCMVTDFMPEDIYVEWTNNGKTELNYKNTEPVLDSDGSYFMYSKLRVEKKNWVERNSYSCSVVHEGLHNHHTTKSFSRTPGK

SEQ ID NO: 58 - protein, 486 aa, synthetic construct
MAVPRWRQQWSGPGTTKRFPETVLARCVKYTEIHPEMRHVDCQSVWDAFKGAFISKHPCNITEEDYQPLMKLGTQTVPCNKILLWSRIKDLAHQFTQVQRDMFTLEDTLLGYLADDLTWCGEFNTSKINYQSCPDWRKDCSNNPVSVFWKTVSRRFAEAACDVVHVMLNGSRSKIFDKNSTFGSVEVHNLQPEKVQTLEAWVIHGGREDSRDLCQDPTIKELESIISKRNIQFSCKNIYRPDKFLQCVKNPEDSSCTSEIGGGSPPCKCPAPNLLGGPSVFIFPPKIKDVLMISLSPIVTCVVVDVSEDDPDVQISWFVNNVEVHTAQTQTHREDYNSTLRVVSALPIQHQDWMSGKEFKCKVNNKDLPAPIERTISKPKSVRAPQVYVLPPPEEEMTKKQVTLTCMVTDFMPEDIYVEWTNNGKTELNYKNTEPVLDSDGSYFMYSKLRVEKKNWVERNSYSCSVVHEGLHNHHTTKSFSRTPGK

SEQ ID NO: 59 - protein, 486 aa, synthetic construct
MAVPRWRQQWSGPGTTKRFPETVLARCVKYTEIHPEMRHVDCQSVWDAFKGAFISKHPCNITEEDYQPLMKLGTQTVPCNKKLLWSRIKDLAHQFTQVQRDMFTLEDTLLGYLADDLTWCGEFNTSKINYQSCPDWRKDCSNNPVSVFWKTVSRRFAEAACDVVHVMLNGSRSKIFDKNSTFGSVEVHNLQPEKVQTLEAWVIHGGREDSRDLCQDPTIKELESIISKRNIQFSCKNIYRPDKFLQCVKNPEDSSCTSEIGGGSPPCKCPAPNLLGGPSVFIFPPKIKDVLMISLSPIVTCVVVDVSEDDPDVQISWFVNNVEVHTAQTQTHREDYNSTLRVVSALPIQHQDWMSGKEFKCKVNNKDLPAPIERTISKPKSVRAPQVYVLPPPEEEMTKKQVTLTCMVTDFMPEDIYVEWTNNGKTELNYKNTEPVLDSDGSYFMYSKLRVEKKNWVERNSYSCSVVHEGLHNHHTTKSFSRTPGK

SEQ ID NO: 60 - protein, 351 aa, synthetic construct
MAQLLFNKTKSVEFTFCNDTVVIPCFVTNMEAQNTTEVYVKWKFKGRDIYTFDGALNKSTVPTDFSSAKIEVSQLLKGDASLKMDKSDAVSHTGNYTCEVTELTREGETIIELKYRVVSWFSPNEGGGSPPCKCPAPNLLGGPSVFIFPPKIKDVLMISLSPIVTCVVVDVSEDDPDVQISWFVNNVEVHTAQTQTHREDYNSTLRVVSALPIQHQDWMSGKEFKCKVNNKDLPAPIERTISKPKSVRAPQVYVLPPPEEEMTKKQVTLTCMVTDFMPEDIYVEWTNNGKTELNYKNTEPVLDSDGSYFMYSKLRVEKKNWVERNSYSCSVVHEGLHNHHTTKSFSRTPGK

SEQ ID NO: 61 - protein, 482 aa, synthetic construct
MAVPRWRQQWSGPGTTKRFPETVLARCVKYTEIHPEMRHVDCQSVWDAFKGAFISKHPCNITEEDYQPLMKLGTQTVPCNKILLWSRIKDLAHQFTQVQRDMFTLEDTLLGYLADDLTWCGEFNTSKINYQSCPDWRKDCSNNPVSVFWKTVSRRFAEAACDVVHVMLNGSRSKIFDKNSTFGSVEVHNLQPEKVQTLEAWVIHGGREDSRDLCQDPTIKELESIISKRNIQFSCKNIYRPDKFLQCVKNPEDSSCTSEIPPCKCPAPNLLGGPSVFIFPPKIKDVLMISLSPIVTCVVVDVSEDDPDVQISWFVNNVEVHTAQTQTHREDYNSTLRVVSALPIQHQDWMSGKEFKCKVNNKDLPAPIERTISKPKSVRAPQVYVLPPPEEEMTKKQVTLTCMVTDFMPEDIYVEWTNNGKTELNYKNTEPVLDSDGSYFMYSKLRVEKKNWVERNSYSCSVVHEGLHNHHTTKSFSRTPGK

SEQ ID NO: 62 - protein, 482 aa, synthetic construct
MAVPRWRQQWSGPGTTKRFPETVLARCVKYTEIHPEMRHVDCQSVWDAFKGAFISKHPCNITEEDYQPLMKLGTQTVPCNKKLLWSRIKDLAHQFTQVQRDMFTLEDTLLGYLADDLTWCGEFNTSKINYQSCPDWRKDCSNNPVSVFWKTVSRRFAEAACDVVHVMLNGSRSKIFDKNSTFGSVEVHNLQPEKVQTLEAWVIHGGREDSRDLCQDPTIKELESIISKRNIQFSCKNIYRPDKFLQCVKNPEDSSCTSEIPPCKCPAPNLLGGPSVFIFPPKIKDVLMISLSPIVTCVVVDVSEDDPDVQISWFVNNVEVHTAQTQTHREDYNSTLRVVSALPIQHQDWMSGKEFKCKVNNKDLPAPIERTISKPKSVRAPQVYVLPPPEEEMTKKQVTLTCMVTDFMPEDIYVEWTNNGKTELNYKNTEPVLDSDGSYFMYSKLRVEKKNWVERNSYSCSVVHEGLHNHHTTKSFSRTPGK

SEQ ID NO: 63 - protein, 347 aa, synthetic construct
MAQLLFNKTKSVEFTFCNDTVVIPCFVTNMEAQNTTEVYVKWKFKGRDIYTFDGALNKSTVPTDFSSAKIEVSQLLKGDASLKMDKSDAVSHTGNYTCEVTELTREGETIIELKYRVVSWFSPNEPPCKCPAPNLLGGPSVFIFPPKIKDVLMISLSPIVTCVVVDVSEDDPDVQISWFVNNVEVHTAQTQTHREDYNSTLRVVSALPIQHQDWMSGKEFKCKVNNKDLPAPIERTISKPKSVRAPQVYVLPPPEEEMTKKQVTLTCMVTDFMPEDIYVEWTNNGKTELNYKNTEPVLDSDGSYFMYSKLRVEKKNWVERNSYSCSVVHEGLHNHHTTKSFSRTPGK

SEQ ID NO: 64 - protein, 489 aa, synthetic construct
MAVPRWRQQWSGPGTTKRFPETVLARCVKYTEIHPEMRHVDCQSVWDAFKGAFISKHPCNITEEDYQPLMKLGTQTVPCNKILLWSRIKDLAHQFTQVQRDMFTLEDTLLGYLADDLTWCGEFNTSKINYQSCPDWRKDCSNNPVSVFWKTVSRRFAEAACDVVHVMLNGSRSKIFDKNSTFGSVEVHNLQPEKVQTLEAWVIHGGREDSRDLCQDPTIKELESIISKRNIQFSCKNIYRPDKFLQCVKNPEDSSCTSEIAAASPSTCSKPTCPPNLLGGPSVFIFPPKIKDVLMISLSPIVTCVVVDVSEDDPDVQISWFVNNVEVHTAQTQTHREDYNSTLRVVSALPIQHQDWMSGKEFKCKVNNKDLPAPIERTISKPKSVRAPQVYVLPPPEEEMTKKQVTLTCMVTDFMPEDIYVEWTNNGKTELNYKNTEPVLDSDGSYFMYSKLRVEKKNWVERNSYSCSVVHEGLHNHHTTKSFSRTPGK

SEQ ID NO: 65 - protein, 489 aa, synthetic construct
MAVPRWRQQWSGPGTTKRFPETVLARCVKYTEIHPEMRHVDCQSVWDAFKGAFISKHPCNITEEDYQPLMKLGTQTVPCNKKLLWSRIKDLAHQFTQVQRDMFTLEDTLLGYLADDLTWCGEFNTSKINYQSCPDWRKDCSNNPVSVFWKTVSRRFAEAACDVVHVMLNGSRSKIFDKNSTFGSVEVHNLQPEKVQTLEAWVIHGGREDSRDLCQDPTIKELESIISKRNIQFSCKNIYRPDKFLQCVKNPEDSSCTSEIAAASPSTCSKPTCPPNLLGGPSVFIFPPKIKDVLMISLSPIVTCVVVDVSEDDPDVQISWFVNNVEVHTAQTQTHREDYNSTLRVVSALPIQHQDWMSGKEFKCKVNNKDLPAPIERTISKPKSVRAPQVYVLPPPEEEMTKKQVTLTCMVTDFMPEDIYVEWTNNGKTELNYKNTEPVLDSDGSYFMYSKLRVEKKNWVERNSYSCSVVHEGLHNHHTTKSFSRTPGK

SEQ ID NO: 66 - protein, 354 aa, synthetic construct
MAQLLFNKTKSVEFTFCNDTVVIPCFVTNMEAQNTTEVYVKWKFKGRDIYTFDGALNKSTVPTDFSSAKIEVSQLLKGDASLKMDKSDAVSHTGNYTCEVTELTREGETIIELKYRVVSWFSPNEAAASPSTCSKPTCPPNLLGGPSVFIFPPKIKDVLMISLSPIVTCVVVDVSEDDPDVQISWFVNNVEVHTAQTQTHREDYNSTLRVVSALPIQHQDWMSGKEFKCKVNNKDLPAPIERTISKPKSVRAPQVYVLPPPEEEMTKKQVTLTCMVTDFMPEDIYVEWTNNGKTELNYKNTEPVLDSDGSYFMYSKLRVEKKNWVERNSYSCSVVHEGLHNHHTTKSFSRTPGK

SEQ ID NO: 67 - protein, 489 aa, synthetic construct
MAVPRWRQQWSGPGTTKRFPETVLARCVKYTEIHPEMRHVDCQSVWDAFKGAFISKHPCNITEEDYQPLMKLGTQTVPCNKILLWSRIKDLAHQFTQVQRDMFTLEDTLLGYLADDLTWCGEFNTSKINYQSCPDWRKDCSNNPVSVFWKTVSRRFAEAACDVVHVMLNGSRSKIFDKNSTFGSVEVHNLQPEKVQTLEAWVIHGGREDSRDLCQDPTIKELESIISKRNIQFSCKNIYRPDKFLQCVKNPEDSSCTSEIGGGSPSTCSKPTCPPNLLGGPSVFIFPPKIKDVLMISLSPIVTCVVVDVSEDDPDVQISWFVNNVEVHTAQTQTHREDYNSTLRVVSALPIQHQDWMSGKEFKCKVNNKDLPAPIERTISKPKSVRAPQVYVLPPPEEEMTKKQVTLTCMVTDFMPEDIYVEWTNNGKTELNYKNTEPVLDSDGSYFMYSKLRVEKKNWVERNSYSCSVVHEGLHNHHTTKSFSRTPGK

SEQ ID NO: 68 - protein, 489 aa, synthetic construct
MAVPRWRQQWSGPGTTKRFPETVLARCVKYTEIHPEMRHVDCQSVWDAFKGAFISKHPCNITEEDYQPLMKLGTQTVPCNKKLLWSRIKDLAHQFTQVQRDMFTLEDTLLGYLADDLTWCGEFNTSKINYQSCPDWRKDCSNNPVSVFWKTVSRRFAEAACDVVHVMLNGSRSKIFDKNSTFGSVEVHNLQPEKVQTLEAWVIHGGREDSRDLCQDPTIKELESIISKRNIQFSCKNIYRPDKFLQCVKNPEDSSCTSEIGGGSPSTCSKPTCPPNLLGGPSVFIFPPKIKDVLMISLSPIVTCVVVDVSEDDPDVQISWFVNNVEVHTAQTQTHREDYNSTLRVVSALPIQHQDWMSGKEFKCKVNNKDLPAPIERTISKPKSVRAPQVYVLPPPEEEMTKKQVTLTCMVTDFMPEDIYVEWTNNGKTELNYKNTEPVLDSDGSYFMYSKLRVEKKNWVERNSYSCSVVHEGLHNHHTTKSFSRTPGK

SEQ ID NO: 69 - protein, 354 aa, synthetic construct
MAQLLFNKTKSVEFTFCNDTVVIPCFVTNMEAQNTTEVYVKWKFKGRDIYTFDGALNKSTVPTDFSSAKIEVSQLLKGDASLKMDKSDAVSHTGNYTCEVTELTREGETIIELKYRVVSWFSPNEGGGSPSTCSKPTCPPNLLGGPSVFIFPPKIKDVLMISLSPIVTCVVVDVSEDDPDVQISWFVNNVEVHTAQTQTHREDYNSTLRVVSALPIQHQDWMSGKEFKCKVNNKDLPAPIERTISKPKSVRAPQVYVLPPPEEEMTKKQVTLTCMVTDFMPEDIYVEWTNNGKTELNYKNTEPVLDSDGSYFMYSKLRVEKKNWVERNSYSCSVVHEGLHNHHTTKSFSRTPGK

SEQ ID NO: 70 - protein, 485 aa, synthetic construct
MAVPRWRQQWSGPGTTKRFPETVLARCVKYTEIHPEMRHVDCQSVWDAFKGAFISKHPCNITEEDYQPLMKLGTQTVPCNKILLWSRIKDLAHQFTQVQRDMFTLEDTLLGYLADDLTWCGEFNTSKINYQSCPDWRKDCSNNPVSVFWKTVSRRFAEAACDVVHVMLNGSRSKIFDKNSTFGSVEVHNLQPEKVQTLEAWVIHGGREDSRDLCQDPTIKELESIISKRNIQFSCKNIYRPDKFLQCVKNPEDSSCTSEIPSTCSKPTCPPNLLGGPSVFIFPPKIKDVLMISLSPIVTCVVVDVSEDDPDVQISWFVNNVEVHTAQTQTHREDYNSTLRVVSALPIQHQDWMSGKEFKCKVNNKDLPAPIERTISKPKSVRAPQVYVLPPPEEEMTKKQVTLTCMVTDFMPEDIYVEWTNNGKTELNYKNTEPVLDSDGSYFMYSKLRVEKKNWVERNSYSCSVVHEGLHNHHTTKSFSRTPGK

SEQ ID NO: 71 - protein, 485 aa, synthetic construct
MAVPRWRQQWSGPGTTKRFPETVLARCVKYTEIHPEMRHVDCQSVWDAFKGAFISKHPCNITEEDYQPLMKLGTQTVPCNKKLLWSRIKDLAHQFTQVQRDMFTLEDTLLGYLADDLTWCGEFNTSKINYQSCPDWRKDCSNNPVSVFWKTVSRRFAEAACDVVHVMLNGSRSKIFDKNSTFGSVEVHNLQPEKVQTLEAWVIHGGREDSRDLCQDPTIKELESIISKRNIQFSCKNIYRPDKFLQCVKNPEDSSCTSEIPSTCSKPTCPPNLLGGPSVFIFPPKIKDVLMISLSPIVTCVVVDVSEDDPDVQISWFVNNVEVHTAQTQTHREDYNSTLRVVSALPIQHQDWMSGKEFKCKVNNKDLPAPIERTISKPKSVRAPQVYVLPPPEEEMTKKQVTLTCMVTDFMPEDIYVEWTNNGKTELNYKNTEPVLDSDGSYFMYSKLRVEKKNWVERNSYSCSVVHEGLHNHHTTKSFSRTPGK

SEQ ID NO: 72 - protein, 350 aa, synthetic construct
MAQLLFNKTKSVEFTFCNDTVVIPCFVTNMEAQNTTEVYVKWKFKGRDIYTFDGALNKSTVPTDFSSAKIEVSQLLKGDASLKMDKSDAVSHTGNYTCEVTELTREGETIIELKYRVVSWFSPNEPSTCSKPTCPPNLLGGPSVFIFPPKIKDVLMISLSPIVTCVVVDVSEDDPDVQISWFVNNVEVHTAQTQTHREDYNSTLRVVSALPIQHQDWMSGKEFKCKVNNKDLPAPIERTISKPKSVRAPQVYVLPPPEEEMTKKQVTLTCMVTDFMPEDIYVEWTNNGKTELNYKNTEPVLDSDGSYFMYSKLRVEKKNWVERNSYSCSVVHEGLHNHHTTKSFSRTPGK

SEQ ID NO: 73 - protein, 485 aa, synthetic construct
MAVPRWRQQWSGPGTTKRFPETVLARCVKYTEIHPEMRHVDCQSVWDAFKGAFISKHPCNITEEDYQPLMKLGTQTVPCNKILLWSRIKDLAHQFTQVQRDMFTLEDTLLGYLADDLTWCGEFNTSKINYQSCPDWRKDCSNNPVSVFWKTVSRRFAEAACDVVHVMLNGSRSKIFDKNSTFGSVEVHNLQPEKVQTLEAWVIHGGREDSRDLCQDPTIKELESIISKRNIQFSCKNIYRPDKFLQCVKNPEDSSCTSEIAAASNPCGCTPNLLGGPSVFIFPPKIKDVLMISLSPIVTCVVVDVSEDDPDVQISWFVNNVEVHTAQTQTHREDYNSTLRVVSALPIQHQDWMSGKEFKCKVNNKDLPAPIERTISKPKSVRAPQVYVLPPPEEEMTKKQVTLTCMVTDFMPEDIYVEWTNNGKTELNYKNTEPVLDSDGSYFMYSKLRVEKKNWVERNSYSCSVVHEGLHNHHTTKSFSRTPGK

SEQ ID NO: 74 - protein, 485 aa, synthetic construct
MAVPRWRQQWSGPGTTKRFPETVLARCVKYTEIHPEMRHVDCQSVWDAFKGAFISKHPCNITEEDYQPLMKLGTQTVPCNKKLLWSRIKDLAHQFTQVQRDMFTLEDTLLGYLADDLTWCGEFNTSKINYQSCPDWRKDCSNNPVSVFWKTVSRRFAEAACDVVHVMLNGSRSKIFDKNSTFGSVEVHNLQPEKVQTLEAWVIHGGREDSRDLCQDPTIKELESIISKRNIQFSCKNIYRPDKFLQCVKNPEDSSCTSEIAAASNPCGCTPNLLGGPSVFIFPPKIKDVLMISLSPIVTCVVVDVSEDDPDVQISWFVNNVEVHTAQTQTHREDYNSTLRVVSALPIQHQDWMSGKEFKCKVNNKDLPAPIERTISKPKSVRAPQVYVLPPPEEEMTKKQVTLTCMVTDFMPEDIYVEWTNNGKTELNYKNTEPVLDSDGSYFMYSKLRVEKKNWVERNSYSCSVVHEGLHNHHTTKSFSRTPGK

SEQ ID NO: 75 - protein, 350 aa, synthetic construct
MAQLLFNKTKSVEFTFCNDTVVIPCFVTNMEAQNTTEVYVKWKFKGRDIYTFDGALNKSTVPTDFSSAKIEVSQLLKGDASLKMDKSDAVSHTGNYTCEVTELTREGETIIELKYRVVSWFSPNEAAASNPCGCTPNLLGGPSVFIFPPKIKDVLMISLSPIVTCVVVDVSEDDPDVQISWFVNNVEVHTAQTQTHREDYNSTLRVVSALPIQHQDWMSGKEFKCKVNNKDLPAPIERTISKPKSVRAPQVYVLPPPEEEMTKKQVTLTCMVTDFMPEDIYVEWTNNGKTELNYKNTEPVLDSDGSYFMYSKLRVEKKNWVERNSYSCSVVHEGLHNHHTTKSFSRTPGK

SEQ ID NO: 76 - protein, 485 aa, synthetic construct
MAVPRWRQQWSGPGTTKRFPETVLARCVKYTEIHPEMRHVDCQSVWDAFKGAFISKHPCNITEEDYQPLMKLGTQTVPCNKILLWSRIKDLAHQFTQVQRDMFTLEDTLLGYLADDLTWCGEFNTSKINYQSCPDWRKDCSNNPVSVFWKTVSRRFAEAACDVVHVMLNGSRSKIFDKNSTFGSVEVHNLQPEKVQTLEAWVIHGGREDSRDLCQDPTIKELESIISKRNIQFSCKNIYRPDKFLQCVKNPEDSSCTSEIGGGSNPCGCTPNLLGGPSVFIFPPKIKDVLMISLSPIVTCVVVDVSEDDPDVQISWFVNNVEVHTAQTQTHREDYNSTLRVVSALPIQHQDWMSGKEFKCKVNNKDLPAPIERTISKPKSVRAPQVYVLPPPEEEMTKKQVTLTCMVTDFMPEDIYVEWTNNGKTELNYKNTEPVLDSDGSYFMYSKLRVEKKNWVERNSYSCSVVHEGLHNHHTTKSFSRTPGK

SEQ ID NO: 77 - protein, 485 aa, synthetic construct
MAVPRWRQQWSGPGTTKRFPETVLARCVKYTEIHPEMRHVDCQSVWDAFKGAFISKHPCNITEEDYQPLMKLGTQTVPCNKKLLWSRIKDLAHQFTQVQRDMFTLEDTLLGYLADDLTWCGEFNTSKINYQSCPDWRKDCSNNPVSVFWKTVSRRFAEAACDVVHVMLNGSRSKIFDKNSTFGSVEVHNLQPEKVQTLEAWVIHGGREDSRDLCQDPTIKELESIISKRNIQFSCKNIYRPDKFLQCVKNPEDSSCTSEIGGGSNPCGCTPNLLGGPSVFIFPPKIKDVLMISLSPIVTCVVVDVSEDDPDVQISWFVNNVEVHTAQTQTHREDYNSTLRVVSALPIQHQDWMSGKEFKCKVNNKDLPAPIERTISKPKSVRAPQVYVLPPPEEEMTKKQVTLTCMVTDFMPEDIYVEWTNNGKTELNYKNTEPVLDSDGSYFMYSKLRVEKKNWVERNSYSCSVVHEGLHNHHTTKSFSRTPGK

SEQ ID NO: 78 - protein, 350 aa, synthetic construct
MAQLLFNKTKSVEFTFCNDTVVIPCFVTNMEAQNTTEVYVKWKFKGRDIYTFDGALNKSTVPTDFSSAKIEVSQLLKGDASLKMDKSDAVSHTGNYTCEVTELTREGETIIELKYRVVSWFSPNEGGGSNPCGCTPNLLGGPSVFIFPPKIKDVLMISLSPIVTCVVVDVSEDDPDVQISWFVNNVEVHTAQTQTHREDYNSTLRVVSALPIQHQDWMSGKEFKCKVNNKDLPAPIERTISKPKSVRAPQVYVLPPPEEEMTKKQVTLTCMVTDFMPEDIYVEWTNNGKTELNYKNTEPVLDSDGSYFMYSKLRVEKKNWVERNSYSCSVVHEGLHNHHTTKSFSRTPGK

SEQ ID NO: 79 - protein, 481 aa, synthetic construct
MAVPRWRQQWSGPGTTKRFPETVLARCVKYTEIHPEMRHVDCQSVWDAFKGAFISKHPCNITEEDYQPLMKLGTQTVPCNKILLWSRIKDLAHQFTQVQRDMFTLEDTLLGYLADDLTWCGEFNTSKINYQSCPDWRKDCSNNPVSVFWKTVSRRFAEAACDVVHVMLNGSRSKIFDKNSTFGSVEVHNLQPEKVQTLEAWVIHGGREDSRDLCQDPTIKELESIISKRNIQFSCKNIYRPDKFLQCVKNPEDSSCTSEINPCGCTPNLLGGPSVFIFPPKIKDVLMISLSPIVTCVVVDVSEDDPDVQISWFVNNVEVHTAQTQTHREDYNSTLRVVSALPIQHQDWMSGKEFKCKVNNKDLPAPIERTISKPKSVRAPQVYVLPPPEEEMTKKQVTLTCMVTDFMPEDIYVEWTNNGKTELNYKNTEPVLDSDGSYFMYSKLRVEKKNWVERNSYSCSVVHEGLHNHHTTKSFSRTPGK

SEQ ID NO: 80 - protein, 481 aa, synthetic construct
MAVPRWRQQWSGPGTTKRFPETVLARCVKYTEIHPEMRHVDCQSVWDAFKGAFISKHPCNITEEDYQPLMKLGTQTVPCNKKLLWSRIKDLAHQFTQVQRDMFTLEDTLLGYLADDLTWCGEFNTSKINYQSCPDWRKDCSNNPVSVFWKTVSRRFAEAACDVVHVMLNGSRSKIFDKNSTFGSVEVHNLQPEKVQTLEAWVIHGGREDSRDLCQDPTIKELESIISKRNIQFSCKNIYRPDKFLQCVKNPEDSSCTSEINPCGCTPNLLGGPSVFIFPPKIKDVLMISLSPIVTCVVVDVSEDDPDVQISWFVNNVEVHTAQTQTHREDYNSTLRVVSALPIQHQDWMSGKEFKCKVNNKDLPAPIERTISKPKSVRAPQVYVLPPPEEEMTKKQVTLTCMVTDFMPEDIYVEWTNNGKTELNYKNTEPVLDSDGSYFMYSKLRVEKKNWVERNSYSCSVVHEGLHNHHTTKSFSRTPGK

SEQ ID NO: 81 - protein, 346 aa, synthetic construct
MAQLLFNKTKSVEFTFCNDTVVIPCFVTNMEAQNTTEVYVKWKFKGRDIYTFDGALNKSTVPTDFSSAKIEVSQLLKGDASLKMDKSDAVSHTGNYTCEVTELTREGETIIELKYRVVSWFSPNENPCGCTPNLLGGPSVFIFPPKIKDVLMISLSPIVTCVVVDVSEDDPDVQISWFVNNVEVHTAQTQTHREDYNSTLRVVSALPIQHQDWMSGKEFKCKVNNKDLPAPIERTISKPKSVRAPQVYVLPPPEEEMTKKQVTLTCMVTDFMPEDIYVEWTNNGKTELNYKNTEPVLDSDGSYFMYSKLRVEKKNWVERNSYSCSVVHEGLHNHHTTKSFSRTPGK

SEQ ID NO: 82 - protein, 489 aa, synthetic construct
MAVPRWRQQWSGPGTTKRFPETVLARCVKYTEIHPEMRHVDCQSVWDAFKGAFISKHPCNITEEDYQPLMKLGTQTVPCNKILLWSRIKDLAHQFTQVQRDMFTLEDTLLGYLADDLTWCGEFNTSKINYQSCPDWRKDCSNNPVSVFWKTVSRRFAEAACDVVHVMLNGSRSKIFDKNSTFGSVEVHNLQPEKVQTLEAWVIHGGREDSRDLCQDPTIKELESIISKRNIQFSCKNIYRPDKFLQCVKNPEDSSCTSEIAAASDKTHTCPPCPPNLLGGPSVFIFPPKIKDVLMISLSPIVTCVVVDVSEDDPDVQISWFVNNVEVHTAQTQTHREDYNSTLRVVSALPIQHQDWMSGKEFKCKVNNKDLPAPIERTISKPKSVRAPQVYVLPPPEEEMTKKQVTLTCMVTDFMPEDIYVEWTNNGKTELNYKNTEPVLDSDGSYFMYSKLRVEKKNWVERNSYSCSVVHEGLHNHHTTKSFSRTPGK

SEQ ID NO: 83 - protein, 489 aa, synthetic construct
MAVPRWRQQWSGPGTTKRFPETVLARCVKYTEIHPEMRHVDCQSVWDAFKGAFISKHPCNITEEDYQPLMKLGTQTVPCNKKLLWSRIKDLAHQFTQVQRDMFTLEDTLLGYLADDLTWCGEFNTSKINYQSCPDWRKDCSNNPVSVFWKTVSRRFAEAACDVVHVMLNGSRSKIFDKNSTFGSVEVHNLQPEKVQTLEAWVIHGGREDSRDLCQDPTIKELESIISKRNIQFSCKNIYRPDKFLQCVKNPEDSSCTSEIAAASDKTHTCPPCPPNLLGGPSVFIFPPKIKDVLMISLSPIVTCVVVDVSEDDPDVQISWFVNNVEVHTAQTQTHREDYNSTLRVVSALPIQHQDWMSGKEFKCKVNNKDLPAPIERTISKPKSVRAPQVYVLPPPEEEMTKKQVTLTCMVTDFMPEDIYVEWTNNGKTELNYKNTEPVLDSDGSYFMYSKLRVEKKNWVERNSYSCSVVHEGLHNHHTTKSFSRTPGK

SEQ ID NO: 84 - protein, 354 aa, synthetic construct
MAQLLFNKTKSVEFTFCNDTVVIPCFVTNMEAQNTTEVYVKWKFKGRDIYTFDGALNKSTVPTDFSSAKIEVSQLLKGDASLKMDKSDAVSHTGNYTCEVTELTREGETIIELKYRVVSWFSPNEAAASDKTHTCPPCPPNLLGGPSVFIFPPKIKDVLMISLSPIVTCVVVDVSEDDPDVQISWFVNNVEVHTAQTQTHREDYNSTLRVVSALPIQHQDWMSGKEFKCKVNNKDLPAPIERTISKPKSVRAPQVYVLPPPEEEMTKKQVTLTCMVTDFMPEDIYVEWTNNGKTELNYKNTEPVLDSDGSYFMYSKLRVEKKNWVERNSYSCSVVHEGLHNHHTTKSFSRTPGK

SEQ ID NO: 85 - protein, 489 aa, synthetic construct
MAVPRWRQQWSGPGTTKRFPETVLARCVKYTEIHPEMRHVDCQSVWDAFKGAFISKHPCNITEEDYQPLMKLGTQTVPCNKILLWSRIKDLAHQFTQVQRDMFTLEDTLLGYLADDLTWCGEFNTSKINYQSCPDWRKDCSNNPVSVFWKTVSRRFAEAACDVVHVMLNGSRSKIFDKNSTFGSVEVHNLQPEKVQTLEAWVIHGGREDSRDLCQDPTIKELESIISKRNIQFSCKNIYRPDKFLQCVKNPEDSSCTSEIGGGSDKTHTCPPCPPNLLGGPSVFIFPPKIKDVLMISLSPIVTCVVVDVSEDDPDVQISWFVNNVEVHTAQTQTHREDYNSTLRVVSALPIQHQDWMSGKEFKCKVNNKDLPAPIERTISKPKSVRAPQVYVLPPPEEEMTKKQVTLTCMVTDFMPEDIYVEWTNNGKTELNYKNTEPVLDSDGSYFMYSKLRVEKKNWVERNSYSCSVVHEGLHNHHTTKSFSRTPGK

SEQ ID NO: 86 - protein, 489 aa, synthetic construct
MAVPRWRQQWSGPGTTKRFPETVLARCVKYTEIHPEMRHVDCQSVWDAFKGAFISKHPCNITEEDYQPLMKLGTQTVPCNKKLLWSRIKDLAHQFTQVQRDMFTLEDTLLGYLADDLTWCGEFNTSKINYQSCPDWRKDCSNNPVSVFWKTVSRRFAEAACDVVHVMLNGSRSKIFDKNSTFGSVEVHNLQPEKVQTLEAWVIHGGREDSRDLCQDPTIKELESIISKRNIQFSCKNIYRPDKFLQCVKNPEDSSCTSEIGGGSDKTHTCPPCPPNLLGGPSVFIFPPKIKDVLMISLSPIVTCVVVDVSEDDPDVQISWFVNNVEVHTAQTQTHREDYNSTLRVVSALPIQHQDWMSGKEFKCKVNNKDLPAPIERTISKPKSVRAPQVYVLPPPEEEMTKKQVTLTCMVTDFMPEDIYVEWTNNGKTELNYKNTEPVLDSDGSYFMYSKLRVEKKNWVERNSYSCSVVHEGLHNHHTTKSFSRTPGK

SEQ ID NO: 87 - protein, 354 aa, synthetic construct
MAQLLFNKTKSVEFTFCNDTVVIPCFVTNMEAQNTTEVYVKWKFKGRDIYTFDGALNKSTVPTDFSSAKIEVSQLLKGDASLKMDKSDAVSHTGNYTCEVTELTREGETIIELKYRVVSWFSPNEGGGSDKTHTCPPCPPNLLGGPSVFIFPPKIKDVLMISLSPIVTCVVVDVSEDDPDVQISWFVNNVEVHTAQTQTHREDYNSTLRVVSALPIQHQDWMSGKEFKCKVNNKDLPAPIERTISKPKSVRAPQVYVLPPPEEEMTKKQVTLTCMVTDFMPEDIYVEWTNNGKTELNYKNTEPVLDSDGSYFMYSKLRVEKKNWVERNSYSCSVVHEGLHNHHTTKSFSRTPGK

SEQ ID NO: 88 - protein, 485 aa, synthetic construct
MAVPRWRQQWSGPGTTKRFPETVLARCVKYTEIHPEMRHVDCQSVWDAFKGAFISKHPCNITEEDYQPLMKLGTQTVPCNKILLWSRIKDLAHQFTQVQRDMFTLEDTLLGYLADDLTWCGEFNTSKINYQSCPDWRKDCSNNPVSVFWKTVSRRFAEAACDVVHVMLNGSRSKIFDKNSTFGSVEVHNLQPEKVQTLEAWVIHGGREDSRDLCQDPTIKELESIISKRNIQFSCKNIYRPDKFLQCVKNPEDSSCTSEIDKTHTCPPCPPNLLGGPSVFIFPPKIKDVLMISLSPIVTCVVVDVSEDDPDVQISWFVNNVEVHTAQTQTHREDYNSTLRVVSALPIQHQDWMSGKEFKCKVNNKDLPAPIERTISKPKSVRAPQVYVLPPPEEEMTKKQVTLTCMVTDFMPEDIYVEWTNNGKTELNYKNTEPVLDSDGSYFMYSKLRVEKKNWVERNSYSCSVVHEGLHNHHTTKSFSRTPGK

SEQ ID NO: 89 - protein, 485 aa, synthetic construct
MAVPRWRQQWSGPGTTKRFPETVLARCVKYTEIHPEMRHVDCQSVWDAFKGAFISKHPCNITEEDYQPLMKLGTQTVPCNKKLLWSRIKDLAHQFTQVQRDMFTLEDTLLGYLADDLTWCGEFNTSKINYQSCPDWRKDCSNNPVSVFWKTVSRRFAEAACDVVHVMLNGSRSKIFDKNSTFGSVEVHNLQPEKVQTLEAWVIHGGREDSRDLCQDPTIKELESIISKRNIQFSCKNIYRPDKFLQCVKNPEDSSCTSEIDKTHTCPPCPPNLLGGPSVFIFPPKIKDVLMISLSPIVTCVVVDVSEDDPDVQISWFVNNVEVHTAQTQTHREDYNSTLRVVSALPIQHQDWMSGKEFKCKVNNKDLPAPIERTISKPKSVRAPQVYVLPPPEEEMTKKQVTLTCMVTDFMPEDIYVEWTNNGKTELNYKNTEPVLDSDGSYFMYSKLRVEKKNWVERNSYSCSVVHEGLHNHHTTKSFSRTPGK

SEQ ID NO: 90 - protein, 350 aa, synthetic construct
MAQLLFNKTKSVEFTFCNDTVVIPCFVTNMEAQNTTEVYVKWKFKGRDIYTFDGALNKSTVPTDFSSAKIEVSQLLKGDASLKMDKSDAVSHTGNYTCEVTELTREGETIIELKYRVVSWFSPNEDKTHTCPPCPPNLLGGPSVFIFPPKIKDVLMISLSPIVTCVVVDVSEDDPDVQISWFVNNVEVHTAQTQTHREDYNSTLRVVSALPIQHQDWMSGKEFKCKVNNKDLPAPIERTISKPKSVRAPQVYVLPPPEEEMTKKQVTLTCMVTDFMPEDIYVEWTNNGKTELNYKNTEPVLDSDGSYFMYSKLRVEKKNWVERNSYSCSVVHEGLHNHHTTKSFSRTPGK

SEQ ID NO: 91 - protein, 486 aa, synthetic construct
MAVPRWRQQWSGPGTTKRFPETVLARCVKYTEIHPEMRHVDCQSVWDAFKGAFISKHPCNITEEDYQPLMKLGTQTVPCNKILLWSRIKDLAHQFTQVQRDMFTLEDTLLGYLADDLTWCGEFNTSKINYQSCPDWRKDCSNNPVSVFWKTVSRRFAEAACDVVHVMLNGSRSKIFDKNSTFGSVEVHNLQPEKVQTLEAWVIHGGREDSRDLCQDPTIKELESIISKRNIQFSCKNIYRPDKFLQCVKNPEDSSCTSEIAAASPPCKCPAPDLLGGPSVFIFPPKIKDVLMISLSPMVTCVVVDVSEDDPDVQISWFVNNVEVHTAQTQTHREDYNSTLRVVSALPIQHQDWMSGKEFKCKVNNRALPSPIEKTISKPRPVRAPQVYVLPPPAEEMTKKEFSLTCMITGFLPAEIAVDWTSNGRTEQNYKNTATVLDSDGSYFMYSKLRVQKSTWERGSLFACSVVHEVLHNHLTTKTISRSLGK

SEQ ID NO: 92 - protein, 486 aa, synthetic construct
MAVPRWRQQWSGPGTTKRFPETVLARCVKYTEIHPEMRHVDCQSVWDAFKGAFISKHPCNITEEDYQPLMKLGTQTVPCNKKLLWSRIKDLAHQFTQVQRDMFTLEDTLLGYLADDLTWCGEFNTSKINYQSCPDWRKDCSNNPVSVFWKTVSRRFAEAACDVVHVMLNGSRSKIFDKNSTFGSVEVHNLQPEKVQTLEAWVIHGGREDSRDLCQDPTIKELESIISKRNIQFSCKNIYRPDKFLQCVKNPEDSSCTSEIAAASPPCKCPAPDLLGGPSVFIFPPKIKDVLMISLSPMVTCVVVDVSEDDPDVQISWFVNNVEVHTAQTQTHREDYNSTLRVVSALPIQHQDWMSGKEFKCKVNNRALPSPIEKTISKPRPVRAPQVYVLPPPAEEMTKKEFSLTCMITGFLPAEIAVDWTSNGRTEQNYKNTATVLDSDGSYFMYSKLRVQKSTWERGSLFACSVVHEVLHNHLTTKTISRSLGK

SEQ ID NO: 93 - protein, 351 aa, synthetic construct
MAQLLFNKTKSVEFTFCNDTVVIPCFVTNMEAQNTTEVYVKWKFKGRDIYTFDGALNKSTVPTDFSSAKIEVSQLLKGDASLKMDKSDAVSHTGNYTCEVTELTREGETIIELKYRVVSWFSPNEAAASPPCKCPAPDLLGGPSVFIFPPKIKDVLMISLSPMVTCVVVDVSEDDPDVQISWFVNNVEVHTAQTQTHREDYNSTLRVVSALPIQHQDWMSGKEFKCKVNNRALPSPIEKTISKPRPVRAPQVYVLPPPAEEMTKKEFSLTCMITGFLPAEIAVDWTSNGRTEQNYKNTATVLDSDGSYFMYSKLRVQKSTWERGSLFACSVVHEVLHNHLTTKTISRSLGK

SEQ ID NO: 94 - protein, 486 aa, synthetic construct
MAVPRWRQQWSGPGTTKRFPETVLARCVKYTEIHPEMRHVDCQSVWDAFKGAFISKHPCNITEEDYQPLMKLGTQTVPCNKILLWSRIKDLAHQFTQVQRDMFTLEDTLLGYLADDLTWCGEFNTSKINYQSCPDWRKDCSNNPVSVFWKTVSRRFAEAACDVVHVMLNGSRSKIFDKNSTFGSVEVHNLQPEKVQTLEAWVIHGGREDSRDLCQDPTIKELESIISKRNIQFSCKNIYRPDKFLQCVKNPEDSSCTSEIGGGSPPCKCPAPDLLGGPSVFIFPPKIKDVLMISLSPMVTCVVVDVSEDDPDVQISWFVNNVEVHTAQTQTHREDYNSTLRVVSALPIQHQDWMSGKEFKCKVNNRALPSPIEKTISKPRPVRAPQVYVLPPPAEEMTKKEFSLTCMITGFLPAEIAVDWTSNGRTEQNYKNTATVLDSDGSYFMYSKLRVQKSTWERGSLFACSVVHEVLHNHLTTKTISRSLGK

SEQ ID NO: 95 - protein, 486 aa, synthetic construct
MAVPRWRQQWSGPGTTKRFPETVLARCVKYTEIHPEMRHVDCQSVWDAFKGAFISKHPCNITEEDYQPLMKLGTQTVPCNKKLLWSRIKDLAHQFTQVQRDMFTLEDTLLGYLADDLTWCGEFNTSKINYQSCPDWRKDCSNNPVSVFWKTVSRRFAEAACDVVHVMLNGSRSKIFDKNSTFGSVEVHNLQPEKVQTLEAWVIHGGREDSRDLCQDPTIKELESIISKRNIQFSCKNIYRPDKFLQCVKNPEDSSCTSEIGGGSPPCKCPAPDLLGGPSVFIFPPKIKDVLMISLSPMVTCVVVDVSEDDPDVQISWFVNNVEVHTAQTQTHREDYNSTLRVVSALPIQHQDWMSGKEFKCKVNNRALPSPIEKTISKPRPVRAPQVYVLPPPAEEMTKKEFSLTCMITGFLPAEIAVDWTSNGRTEQNYKNTATVLDSDGSYFMYSKLRVQKSTWERGSLFACSVVHEVLHNHLTTKTISRSLGK

SEQ ID NO: 96 - protein, 351 aa, synthetic construct
MAQLLFNKTKSVEFTFCNDTVVIPCFVTNMEAQNTTEVYVKWKFKGRDIYTFDGALNKSTVPTDFSSAKIEVSQLLKGDASLKMDKSDAVSHTGNYTCEVTELTREGETIIELKYRVVSWFSPNEGGGSPPCKCPAPDLLGGPSVFIFPPKIKDVLMISLSPMVTCVVVDVSEDDPDVQISWFVNNVEVHTAQTQTHREDYNSTLRVVSALPIQHQDWMSGKEFKCKVNNRALPSPIEKTISKPRPVRAPQVYVLPPPAEEMTKKEFSLTCMITGFLPAEIAVDWTSNGRTEQNYKNTATVLDSDGSYFMYSKLRVQKSTWERGSLFACSVVHEVLHNHLTTKTISRSLGK

SEQ ID NO: 97 - protein, 482 aa, synthetic construct
MAVPRWRQQWSGPGTTKRFPETVLARCVKYTEIHPEMRHVDCQSVWDAFKGAFISKHPCNITEEDYQPLMKLGTQTVPCNKILLWSRIKDLAHQFTQVQRDMFTLEDTLLGYLADDLTWCGEFNTSKINYQSCPDWRKDCSNNPVSVFWKTVSRRFAEAACDVVHVMLNGSRSKIFDKNSTFGSVEVHNLQPEKVQTLEAWVIHGGREDSRDLCQDPTIKELESIISKRNIQFSCKNIYRPDKFLQCVKNPEDSSCTSEIPPCKCPAPDLLGGPSVFIFPPKIKDVLMISLSPMVTCVVVDVSEDDPDVQISWFVNNVEVHTAQTQTHREDYNSTLRVVSALPIQHQDWMSGKEFKCKVNNRALPSPIEKTISKPRPVRAPQVYVLPPPAEEMTKKEFSLTCMITGFLPAEIAVDWTSNGRTEQNYKNTATVLDSDGSYFMYSKLRVQKSTWERGSLFACSVVHEVLHNHLTTKTISRSLGK

SEQ ID NO: 98 - protein, 482 aa, synthetic construct
MAVPRWRQQWSGPGTTKRFPETVLARCVKYTEIHPEMRHVDCQSVWDAFKGAFISKHPCNITEEDYQPLMKLGTQTVPCNKKLLWSRIKDLAHQFTQVQRDMFTLEDTLLGYLADDLTWCGEFNTSKINYQSCPDWRKDCSNNPVSVFWKTVSRRFAEAACDVVHVMLNGSRSKIFDKNSTFGSVEVHNLQPEKVQTLEAWVIHGGREDSRDLCQDPTIKELESIISKRNIQFSCKNIYRPDKFLQCVKNPEDSSCTSEIPPCKCPAPDLLGGPSVFIFPPKIKDVLMISLSPMVTCVVVDVSEDDPDVQISWFVNNVEVHTAQTQTHREDYNSTLRVVSALPIQHQDWMSGKEFKCKVNNRALPSPIEKTISKPRPVRAPQVYVLPPPAEEMTKKEFSLTCMITGFLPAEIAVDWTSNGRTEQNYKNTATVLDSDGSYFMYSKLRVQKSTWERGSLFACSVVHEVLHNHLTTKTISRSLGK

SEQ ID NO: 99 - protein, 347 aa, synthetic construct
MAQLLFNKTKSVEFTFCNDTVVIPCFVTNMEAQNTTEVYVKWKFKGRDIYTFDGALNKSTVPTDFSSAKIEVSQLLKGDASLKMDKSDAVSHTGNYTCEVTELTREGETIIELKYRVVSWFSPNEPPCKCPAPDLLGGPSVFIFPPKIKDVLMISLSPMVTCVVVDVSEDDPDVQISWFVNNVEVHTAQTQTHREDYNSTLRVVSALPIQHQDWMSGKEFKCKVNNRALPSPIEKTISKPRPVRAPQVYVLPPPAEEMTKKEFSLTCMITGFLPAEIAVDWTSNGRTEQNYKNTATVLDSDGSYFMYSKLRVQKSTWERGSLFACSVVHEVLHNHLTTKTISRSLGK

SEQ ID NO: 100 - protein, 489 aa, synthetic construct
MAVPRWRQQWSGPGTTKRFPETVLARCVKYTEIHPEMRHVDCQSVWDAFKGAFISKHPCNITEEDYQPLMKLGTQTVPCNKILLWSRIKDLAHQFTQVQRDMFTLEDTLLGYLADDLTWCGEFNTSKINYQSCPDWRKDCSNNPVSVFWKTVSRRFAEAACDVVHVMLNGSRSKIFDKNSTFGSVEVHNLQPEKVQTLEAWVIHGGREDSRDLCQDPTIKELESIISKRNIQFSCKNIYRPDKFLQCVKNPEDSSCTSEIAAASPSTCSKPTCPPDLLGGPSVFIFPPKIKDVLMISLSPMVTCVVVDVSEDDPDVQISWFVNNVEVHTAQTQTHREDYNSTLRVVSALPIQHQDWMSGKEFKCKVNNRALPSPIEKTISKPRPVRAPQVYVLPPPAEEMTKKEFSLTCMITGFLPAEIAVDWTSNGRTEQNYKNTATVLDSDGSYFMYSKLRVQKSTWERGSLFACSVVHEVLHNHLTTKTISRSLGK

SEQ ID NO: 101 - protein, 489 aa, synthetic construct
MAVPRWRQQWSGPGTTKRFPETVLARCVKYTEIHPEMRHVDCQSVWDAFKGAFISKHPCNITEEDYQPLMKLGTQTVPCNKKLLWSRIKDLAHQFTQVQRDMFTLEDTLLGYLADDLTWCGEFNTSKINYQSCPDWRKDCSNNPVSVFWKTVSRRFAEAACDVVHVMLNGSRSKIFDKNSTFGSVEVHNLQPEKVQTLEAWVIHGGREDSRDLCQDPTIKELESIISKRNIQFSCKNIYRPDKFLQCVKNPEDSSCTSEIAAASPSTCSKPTCPPDLLGGPSVFIFPPKIKDVLMISLSPMVTCVVVDVSEDDPDVQISWFVNNVEVHTAQTQTHREDYNSTLRVVSALPIQHQDWMSGKEFKCKVNNRALPSPIEKTISKPRPVRAPQVYVLPPPAEEMTKKEFSLTCMITGFLPAEIAVDWTSNGRTEQNYKNTATVLDSDGSYFMYSKLRVQKSTWERGSLFACSVVHEVLHNHLTTKTISRSLGK

SEQ ID NO: 102 - protein, 354 aa, synthetic construct
MAQLLFNKTKSVEFTFCNDTVVIPCFVTNMEAQNTTEVYVKWKFKGRDIYTFDGALNKSTVPTDFSSAKIEVSQLLKGDASLKMDKSDAVSHTGNYTCEVTELTREGETIIELKYRVVSWFSPNEAAASPSTCSKPTCPPDLLGGPSVFIFPPKIKDVLMISLSPMVTCVVVDVSEDDPDVQISWFVNNVEVHTAQTQTHREDYNSTLRVVSALPIQHQDWMSGKEFKCKVNNRALPSPIEKTISKPRPVRAPQVYVLPPPAEEMTKKEFSLTCMITGFLPAEIAVDWTSNGRTEQNYKNTATVLDSDGSYFMYSKLRVQKSTWERGSLFACSVVHEVLHNHLTTKTISRSLGK

SEQ ID NO: 103 - protein, 489 aa, synthetic construct
MAVPRWRQQWSGPGTTKRFPETVLARCVKYTEIHPEMRHVDCQSVWDAFKGAFISKHPCNITEEDYQPLMKLGTQTVPCNKILLWSRIKDLAHQFTQVQRDMFTLEDTLLGYLADDLTWCGEFNTSKINYQSCPDWRKDCSNNPVSVFWKTVSRRFAEAACDVVHVMLNGSRSKIFDKNSTFGSVEVHNLQPEKVQTLEAWVIHGGREDSRDLCQDPTIKELESIISKRNIQFSCKNIYRPDKFLQCVKNPEDSSCTSEIGGGSPSTCSKPTCPPDLLGGPSVFIFPPKIKDVLMISLSPMVTCVVVDVSEDDPDVQISWFVNNVEVHTAQTQTHREDYNSTLRVVSALPIQHQDWMSGKEFKCKVNNRALPSPIEKTISKPRPVRAPQVYVLPPPAEEMTKKEFSLTCMITGFLPAEIAVDWTSNGRTEQNYKNTATVLDSDGSYFMYSKLRVQKSTWERGSLFACSVVHEVLHNHLTTKTISRSLGK

SEQ ID NO: 104 - protein, 489 aa, synthetic construct
MAVPRWRQQWSGPGTTKRFPETVLARCVKYTEIHPEMRHVDCQSVWDAFKGAFISKHPCNITEEDYQPLMKLGTQTVPCNKKLLWSRIKDLAHQFTQVQRDMFTLEDTLLGYLADDLTWCGEFNTSKINYQSCPDWRKDCSNNPVSVFWKTVSRRFAEAACDVVHVMLNGSRSKIFDKNSTFGSVEVHNLQPEKVQTLEAWVIHGGREDSRDLCQDPTIKELESIISKRNIQFSCKNIYRPDKFLQCVKNPEDSSCTSEIGGGSPSTCSKPTCPPDLLGGPSVFIFPPKIKDVLMISLSPMVTCVVVDVSEDDPDVQISWFVNNVEVHTAQTQTHREDYNSTLRVVSALPIQHQDWMSGKEFKCKVNNRALPSPIEKTISKPRPVRAPQVYVLPPPAEEMTKKEFSLTCMITGFLPAEIAVDWTSNGRTEQNYKNTATVLDSDGSYFMYSKLRVQKSTWERGSLFACSVVHEVLHNHLTTKTISRSLGK

SEQ ID NO: 105 - protein, 354 aa, synthetic construct
MAQLLFNKTKSVEFTFCNDTVVIPCFVTNMEAQNTTEVYVKWKFKGRDIYTFDGALNKSTVPTDFSSAKIEVSQLLKGDASLKMDKSDAVSHTGNYTCEVTELTREGETIIELKYRVVSWFSPNEGGGSPSTCSKPTCPPDLLGGPSVFIFPPKIKDVLMISLSPMVTCVVVDVSEDDPDVQISWFVNNVEVHTAQTQTHREDYNSTLRVVSALPIQHQDWMSGKEFKCKVNNRALPSPIEKTISKPRPVRAPQVYVLPPPAEEMTKKEFSLTCMITGFLPAEIAVDWTSNGRTEQNYKNTATVLDSDGSYFMYSKLRVQKSTWERGSLFACSVVHEVLHNHLTTKTISRSLGK

SEQ ID NO: 106 - protein, 485 aa, synthetic construct
MAVPRWRQQWSGPGTTKRFPETVLARCVKYTEIHPEMRHVDCQSVWDAFKGAFISKHPCNITEEDYQPLMKLGTQTVPCNKILLWSRIKDLAHQFTQVQRDMFTLEDTLLGYLADDLTWCGEFNTSKINYQSCPDWRKDCSNNPVSVFWKTVSRRFAEAACDVVHVMLNGSRSKIFDKNSTFGSVEVHNLQPEKVQTLEAWVIHGGREDSRDLCQDPTIKELESIISKRNIQFSCKNIYRPDKFLQCVKNPEDSSCTSEIPSTCSKPTCPPDLLGGPSVFIFPPKIKDVLMISLSPMVTCVVVDVSEDDPDVQISWFVNNVEVHTAQTQTHREDYNSTLRVVSALPIQHQDWMSGKEFKCKVNNRALPSPIEKTISKPRPVRAPQVYVLPPPAEEMTKKEFSLTCMITGFLPAEIAVDWTSNGRTEQNYKNTATVLDSDGSYFMYSKLRVQKSTWERGSLFACSVVHEVLHNHLTTKTISRSLGK

SEQ ID NO: 107 - protein, 485 aa, synthetic construct
MAVPRWRQQWSGPGTTKRFPETVLARCVKYTEIHPEMRHVDCQSVWDAFKGAFISKHPCNITEEDYQPLMKLGTQTVPCNKKLLWSRIKDLAHQFTQVQRDMFTLEDTLLGYLADDLTWCGEFNTSKINYQSCPDWRKDCSNNPVSVFWKTVSRRFAEAACDVVHVMLNGSRSKIFDKNSTFGSVEVHNLQPEKVQTLEAWVIHGGREDSRDLCQDPTIKELESIISKRNIQFSCKNIYRPDKFLQCVKNPEDSSCTSEIPSTCSKPTCPPDLLGGPSVFIFPPKIKDVLMISLSPMVTCVVVDVSEDDPDVQISWFVNNVEVHTAQTQTHREDYNSTLRVVSALPIQHQDWMSGKEFKCKVNNRALPSPIEKTISKPRPVRAPQVYVLPPPAEEMTKKEFSLTCMITGFLPAEIAVDWTSNGRTEQNYKNTATVLDSDGSYFMYSKLRVQKSTWERGSLFACSVVHEVLHNHLTTKTISRSLGK

SEQ ID NO: 108 - protein, 350 aa, synthetic construct
MAQLLFNKTKSVEFTFCNDTVVIPCFVTNMEAQNTTEVYVKWKFKGRDIYTFDGALNKSTVPTDFSSAKIEVSQLLKGDASLKMDKSDAVSHTGNYTCEVTELTREGETIIELKYRVVSWFSPNEPSTCSKPTCPPDLLGGPSVFIFPPKIKDVLMISLSPMVTCVVVDVSEDDPDVQISWFVNNVEVHTAQTQTHREDYNSTLRVVSALPIQHQDWMSGKEFKCKVNNRALPSPIEKTISKPRPVRAPQVYVLPPPAEEMTKKEFSLTCMITGFLPAEIAVDWTSNGRTEQNYKNTATVLDSDGSYFMYSKLRVQKSTWERGSLFACSVVHEVLHNHLTTKTISRSLGK

SEQ ID NO: 109 - protein, 485 aa, synthetic construct
MAVPRWRQQWSGPGTTKRFPETVLARCVKYTEIHPEMRHVDCQSVWDAFKGAFISKHPCNITEEDYQPLMKLGTQTVPCNKILLWSRIKDLAHQFTQVQRDMFTLEDTLLGYLADDLTWCGEFNTSKINYQSCPDWRKDCSNNPVSVFWKTVSRRFAEAACDVVHVMLNGSRSKIFDKNSTFGSVEVHNLQPEKVQTLEAWVIHGGREDSRDLCQDPTIKELESIISKRNIQFSCKNIYRPDKFLQCVKNPEDSSCTSEIAAASNPCGCTPDLLGGPSVFIFPPKIKDVLMISLSPMVTCVVVDVSEDDPDVQISWFVNNVEVHTAQTQTHREDYNSTLRVVSALPIQHQDWMSGKEFKCKVNNRALPSPIEKTISKPRPVRAPQVYVLPPPAEEMTKKEFSLTCMITGFLPAEIAVDWTSNGRTEQNYKNTATVLDSDGSYFMYSKLRVQKSTWERGSLFACSVVHEVLHNHLTTKTISRSLGK

SEQ ID NO: 110 - protein, 485 aa, synthetic construct
MAVPRWRQQWSGPGTTKRFPETVLARCVKYTEIHPEMRHVDCQSVWDAFKGAFISKHPCNITEEDYQPLMKLGTQTVPCNKKLLWSRIKDLAHQFTQVQRDMFTLEDTLLGYLADDLTWCGEFNTSKINYQSCPDWRKDCSNNPVSVFWKTVSRRFAEAACDVVHVMLNGSRSKIFDKNSTFGSVEVHNLQPEKVQTLEAWVIHGGREDSRDLCQDPTIKELESIISKRNIQFSCKNIYRPDKFLQCVKNPEDSSCTSEIAAASNPCGCTPDLLGGPSVFIFPPKIKDVLMISLSPMVTCVVVDVSEDDPDVQISWFVNNVEVHTAQTQTHREDYNSTLRVVSALPIQHQDWMSGKEFKCKVNNRALPSPIEKTISKPRPVRAPQVYVLPPPAEEMTKKEFSLTCMITGFLPAEIAVDWTSNGRTEQNYKNTATVLDSDGSYFMYSKLRVQKSTWERGSLFACSVVHEVLHNHLTTKTISRSLGK

SEQ ID NO: 111 - protein, 350 aa, synthetic construct
MAQLLFNKTKSVEFTFCNDTVVIPCFVTNMEAQNTTEVYVKWKFKGRDIYTFDGALNKSTVPTDFSSAKIEVSQLLKGDASLKMDKSDAVSHTGNYTCEVTELTREGETIIELKYRVVSWFSPNEAAASNPCGCTPDLLGGPSVFIFPPKIKDVLMISLSPMVTCVVVDVSEDDPDVQISWFVNNVEVHTAQTQTHREDYNSTLRVVSALPIQHQDWMSGKEFKCKVNNRALPSPIEKTISKPRPVRAPQVYVLPPPAEEMTKKEFSLTCMITGFLPAEIAVDWTSNGRTEQNYKNTATVLDSDGSYFMYSKLRVQKSTWERGSLFACSVVHEVLHNHLTTKTISRSLGK

SEQ ID NO: 112 - protein, 485 aa, synthetic construct
MAVPRWRQQWSGPGTTKRFPETVLARCVKYTEIHPEMRHVDCQSVWDAFKGAFISKHPCNITEEDYQPLMKLGTQTVPCNKILLWSRIKDLAHQFTQVQRDMFTLEDTLLGYLADDLTWCGEFNTSKINYQSCPDWRKDCSNNPVSVFWKTVSRRFAEAACDVVHVMLNGSRSKIFDKNSTFGSVEVHNLQPEKVQTLEAWVIHGGREDSRDLCQDPTIKELESIISKRNIQFSCKNIYRPDKFLQCVKNPEDSSCTSEIGGGSNPCGCTPDLLGGPSVFIFPPKIKDVLMISLSPMVTCVVVDVSEDDPDVQISWFVNNVEVHTAQTQTHREDYNSTLRVVSALPIQHQDWMSGKEFKCKVNNRALPSPIEKTISKPRPVRAPQVYVLPPPAEEMTKKEFSLTCMITGFLPAEIAVDWTSNGRTEQNYKNTATVLDSDGSYFMYSKLRVQKSTWERGSLFACSVVHEVLHNHLTTKTISRSLGK

SEQ ID NO: 113 - protein, 485 aa, synthetic construct
MAVPRWRQQWSGPGTTKRFPETVLARCVKYTEIHPEMRHVDCQSVWDAFKGAFISKHPCNITEEDYQPLMKLGTQTVPCNKKLLWSRIKDLAHQFTQVQRDMFTLEDTLLGYLADDLTWCGEFNTSKINYQSCPDWRKDCSNNPVSVFWKTVSRRFAEAACDVVHVMLNGSRSKIFDKNSTFGSVEVHNLQPEKVQTLEAWVIHGGREDSRDLCQDPTIKELESIISKRNIQFSCKNIYRPDKFLQCVKNPEDSSCTSEIGGGSNPCGCTPDLLGGPSVFIFPPKIKDVLMISLSPMVTCVVVDVSEDDPDVQISWFVNNVEVHTAQTQTHREDYNSTLRVVSALPIQHQDWMSGKEFKCKVNNRALPSPIEKTISKPRPVRAPQVYVLPPPAEEMTKKEFSLTCMITGFLPAEIAVDWTSNGRTEQNYKNTATVLDSDGSYFMYSKLRVQKSTWERGSLFACSVVHEVLHNHLTTKTISRSLGK

SEQ ID NO: 114 - protein, 350 aa, synthetic construct
MAQLLFNKTKSVEFTFCNDTVVIPCFVTNMEAQNTTEVYVKWKFKGRDIYTFDGALNKSTVPTDFSSAKIEVSQLLKGDASLKMDKSDAVSHTGNYTCEVTELTREGETIIELKYRVVSWFSPNEGGGSNPCGCTPDLLGGPSVFIFPPKIKDVLMISLSPMVTCVVVDVSEDDPDVQISWFVNNVEVHTAQTQTHREDYNSTLRVVSALPIQHQDWMSGKEFKCKVNNRALPSPIEKTISKPRPVRAPQVYVLPPPAEEMTKKEFSLTCMITGFLPAEIAVDWTSNGRTEQNYKNTATVLDSDGSYFMYSKLRVQKSTWERGSLFACSVVHEVLHNHLTTKTISRSLGK

SEQ ID NO: 115 - protein, 481 aa, synthetic construct
MAVPRWRQQWSGPGTTKRFPETVLARCVKYTEIHPEMRHVDCQSVWDAFKGAFISKHPCNITEEDYQPLMKLGTQTVPCNKILLWSRIKDLAHQFTQVQRDMFTLEDTLLGYLADDLTWCGEFNTSKINYQSCPDWRKDCSNNPVSVFWKTVSRRFAEAACDVVHVMLNGSRSKIFDKNSTFGSVEVHNLQPEKVQTLEAWVIHGGREDSRDLCQDPTIKELESIISKRNIQFSCKNIYRPDKFLQCVKNPEDSSCTSEINPCGCTPDLLGGPSVFIFPPKIKDVLMISLSPMVTCVVVDVSEDDPDVQISWFVNNVEVHTAQTQTHREDYNSTLRVVSALPIQHQDWMSGKEFKCKVNNRALPSPIEKTISKPRPVRAPQVYVLPPPAEEMTKKEFSLTCMITGFLPAEIAVDWTSNGRTEQNYKNTATVLDSDGSYFMYSKLRVQKSTWERGSLFACSVVHEVLHNHLTTKTISRSLGK

SEQ ID NO: 116 - protein, 481 aa, synthetic construct
MAVPRWRQQWSGPGTTKRFPETVLARCVKYTEIHPEMRHVDCQSVWDAFKGAFISKHPCNITEEDYQPLMKLGTQTVPCNKKLLWSRIKDLAHQFTQVQRDMFTLEDTLLGYLADDLTWCGEFNTSKINYQSCPDWRKDCSNNPVSVFWKTVSRRFAEAACDVVHVMLNGSRSKIFDKNSTFGSVEVHNLQPEKVQTLEAWVIHGGREDSRDLCQDPTIKELESIISKRNIQFSCKNIYRPDKFLQCVKNPEDSSCTSEINPCGCTPDLLGGPSVFIFPPKIKDVLMISLSPMVTCVVVDVSEDDPDVQISWFVNNVEVHTAQTQTHREDYNSTLRVVSALPIQHQDWMSGKEFKCKVNNRALPSPIEKTISKPRPVRAPQVYVLPPPAEEMTKKEFSLTCMITGFLPAEIAVDWTSNGRTEQNYKNTATVLDSDGSYFMYSKLRVQKSTWERGSLFACSVVHEVLHNHLTTKTISRSLGK

SEQ ID NO: 117 - protein, 346 aa, synthetic construct
MAQLLFNKTKSVEFTFCNDTVVIPCFVTNMEAQNTTEVYVKWKFKGRDIYTFDGALNKSTVPTDFSSAKIEVSQLLKGDASLKMDKSDAVSHTGNYTCEVTELTREGETIIELKYRVVSWFSPNENPCGCTPDLLGGPSVFIFPPKIKDVLMISLSPMVTCVVVDVSEDDPDVQISWFVNNVEVHTAQTQTHREDYNSTLRVVSALPIQHQDWMSGKEFKCKVNNRALPSPIEKTISKPRPVRAPQVYVLPPPAEEMTKKEFSLTCMITGFLPAEIAVDWTSNGRTEQNYKNTATVLDSDGSYFMYSKLRVQKSTWERGSLFACSVVHEVLHNHLTTKTISRSLGK

SEQ ID NO: 118 - protein, 489 aa, synthetic construct
MAVPRWRQQWSGPGTTKRFPETVLARCVKYTEIHPEMRHVDCQSVWDAFKGAFISKHPCNITEEDYQPLMKLGTQTVPCNKILLWSRIKDLAHQFTQVQRDMFTLEDTLLGYLADDLTWCGEFNTSKINYQSCPDWRKDCSNNPVSVFWKTVSRRFAEAACDVVHVMLNGSRSKIFDKNSTFGSVEVHNLQPEKVQTLEAWVIHGGREDSRDLCQDPTIKELESIISKRNIQFSCKNIYRPDKFLQCVKNPEDSSCTSEIAAASDKTHTCPPCPPDLLGGPSVFIFPPKIKDVLMISLSPMVTCVVVDVSEDDPDVQISWFVNNVEVHTAQTQTHREDYNSTLRVVSALPIQHQDWMSGKEFKCKVNNRALPSPIEKTISKPRPVRAPQVYVLPPPAEEMTKKEFSLTCMITGFLPAEIAVDWTSNGRTEQNYKNTATVLDSDGSYFMYSKLRVQKSTWERGSLFACSVVHEVLHNHLTTKTISRSLGK

SEQ ID NO: 119 - protein, 489 aa, synthetic construct
MAVPRWRQQWSGPGTTKRFPETVLARCVKYTEIHPEMRHVDCQSVWDAFKGAFISKHPCNITEEDYQPLMKLGTQTVPCNKKLLWSRIKDLAHQFTQVQRDMFTLEDTLLGYLADDLTWCGEFNTSKINYQSCPDWRKDCSNNPVSVFWKTVSRRFAEAACDVVHVMLNGSRSKIFDKNSTFGSVEVHNLQPEKVQTLEAWVIHGGREDSRDLCQDPTIKELESIISKRNIQFSCKNIYRPDKFLQCVKNPEDSSCTSEIAAASDKTHTCPPCPPDLLGGPSVFIFPPKIKDVLMISLSPMVTCVVVDVSEDDPDVQISWFVNNVEVHTAQTQTHREDYNSTLRVVSALPIQHQDWMSGKEFKCKVNNRALPSPIEKTISKPRPVRAPQVYVLPPPAEEMTKKEFSLTCMITGFLPAEIAVDWTSNGRTEQNYKNTATVLDSDGSYFMYSKLRVQKSTWERGSLFACSVVHEVLHNHLTTKTISRSLGK

SEQ ID NO: 120 - protein, 354 aa, synthetic construct
MAQLLFNKTKSVEFTFCNDTVVIPCFVTNMEAQNTTEVYVKWKFKGRDIYTFDGALNKSTVPTDFSSAKIEVSQLLKGDASLKMDKSDAVSHTGNYTCEVTELTREGETIIELKYRVVSWFSPNEAAASDKTHTCPPCPPDLLGGPSVFIFPPKIKDVLMISLSPMVTCVVVDVSEDDPDVQISWFVNNVEVHTAQTQTHREDYNSTLRVVSALPIQHQDWMSGKEFKCKVNNRALPSPIEKTISKPRPVRAPQVYVLPPPAEEMTKKEFSLTCMITGFLPAEIAVDWTSNGRTEQNYKNTATVLDSDGSYFMYSKLRVQKSTWERGSLFACSVVHEVLHNHLTTKTISRSLGK

SEQ ID NO: 121 - protein, 489 aa, synthetic construct
MAVPRWRQQWSGPGTTKRFPETVLARCVKYTEIHPEMRHVDCQSVWDAFKGAFISKHPCNITEEDYQPLMKLGTQTVPCNKILLWSRIKDLAHQFTQVQRDMFTLEDTLLGYLADDLTWCGEFNTSKINYQSCPDWRKDCSNNPVSVFWKTVSRRFAEAACDVVHVMLNGSRSKIFDKNSTFGSVEVHNLQPEKVQTLEAWVIHGGREDSRDLCQDPTIKELESIISKRNIQFSCKNIYRPDKFLQCVKNPEDSSCTSEIGGGSDKTHTCPPCPPDLLGGPSVFIFPPKIKDVLMISLSPMVTCVVVDVSEDDPDVQISWFVNNVEVHTAQTQTHREDYNSTLRVVSALPIQHQDWMSGKEFKCKVNNRALPSPIEKTISKPRPVRAPQVYVLPPPAEEMTKKEFSLTCMITGFLPAEIAVDWTSNGRTEQNYKNTATVLDSDGSYFMYSKLRVQKSTWERGSLFACSVVHEVLHNHLTTKTISRSLGK

SEQ ID NO: 122 - protein, 489 aa, synthetic construct
MAVPRWRQQWSGPGTTKRFPETVLARCVKYTEIHPEMRHVDCQSVWDAFKGAFISKHPCNITEEDYQPLMKLGTQTVPCNKKLLWSRIKDLAHQFTQVQRDMFTLEDTLLGYLADDLTWCGEFNTSKINYQSCPDWRKDCSNNPVSVFWKTVSRRFAEAACDVVHVMLNGSRSKIFDKNSTFGSVEVHNLQPEKVQTLEAWVIHGGREDSRDLCQDPTIKELESIISKRNIQFSCKNIYRPDKFLQCVKNPEDSSCTSEIGGGSDKTHTCPPCPPDLLGGPSVFIFPPKIKDVLMISLSPMVTCVVVDVSEDDPDVQISWFVNNVEVHTAQTQTHREDYNSTLRVVSALPIQHQDWMSGKEFKCKVNNRALPSPIEKTISKPRPVRAPQVYVLPPPAEEMTKKEFSLTCMITGFLPAEIAVDWTSNGRTEQNYKNTATVLDSDGSYFMYSKLRVQKSTWERGSLFACSVVHEVLHNHLTTKTISRSLGK

SEQ ID NO: 123 - protein, 354 aa, synthetic construct
MAQLLFNKTKSVEFTFCNDTVVIPCFVTNMEAQNTTEVYVKWKFKGRDIYTFDGALNKSTVPTDFSSAKIEVSQLLKGDASLKMDKSDAVSHTGNYTCEVTELTREGETIIELKYRVVSWFSPNEGGGSDKTHTCPPCPPDLLGGPSVFIFPPKIKDVLMISLSPMVTCVVVDVSEDDPDVQISWFVNNVEVHTAQTQTHREDYNSTLRVVSALPIQHQDWMSGKEFKCKVNNRALPSPIEKTISKPRPVRAPQVYVLPPPAEEMTKKEFSLTCMITGFLPAEIAVDWTSNGRTEQNYKNTATVLDSDGSYFMYSKLRVQKSTWERGSLFACSVVHEVLHNHLTTKTISRSLGK

SEQ ID NO: 124 - protein, 485 aa, synthetic construct
MAVPRWRQQWSGPGTTKRFPETVLARCVKYTEIHPEMRHVDCQSVWDAFKGAFISKHPCNITEEDYQPLMKLGTQTVPCNKILLWSRIKDLAHQFTQVQRDMFTLEDTLLGYLADDLTWCGEFNTSKINYQSCPDWRKDCSNNPVSVFWKTVSRRFAEAACDVVHVMLNGSRSKIFDKNSTFGSVEVHNLQPEKVQTLEAWVIHGGREDSRDLCQDPTIKELESIISKRNIQFSCKNIYRPDKFLQCVKNPEDSSCTSEIDKTHTCPPCPPDLLGGPSVFIFPPKIKDVLMISLSPMVTCVVVDVSEDDPDVQISWFVNNVEVHTAQTQTHREDYNSTLRVVSALPIQHQDWMSGKEFKCKVNNRALPSPIEKTISKPRPVRAPQVYVLPPPAEEMTKKEFSLTCMITGFLPAEIAVDWTSNGRTEQNYKNTATVLDSDGSYFMYSKLRVQKSTWERGSLFACSVVHEVLHNHLTTKTISRSLGK

SEQ ID NO: 125 - protein, 485 aa, synthetic construct
MAVPRWRQQWSGPGTTKRFPETVLARCVKYTEIHPEMRHVDCQSVWDAFKGAFISKHPCNITEEDYQPLMKLGTQTVPCNKKLLWSRIKDLAHQFTQVQRDMFTLEDTLLGYLADDLTWCGEFNTSKINYQSCPDWRKDCSNNPVSVFWKTVSRRFAEAACDVVHVMLNGSRSKIFDKNSTFGSVEVHNLQPEKVQTLEAWVIHGGREDSRDLCQDPTIKELESIISKRNIQFSCKNIYRPDKFLQCVKNPEDSSCTSEIDKTHTCPPCPPDLLGGPSVFIFPPKIKDVLMISLSPMVTCVVVDVSEDDPDVQISWFVNNVEVHTAQTQTHREDYNSTLRVVSALPIQHQDWMSGKEFKCKVNNRALPSPIEKTISKPRPVRAPQVYVLPPPAEEMTKKEFSLTCMITGFLPAEIAVDWTSNGRTEQNYKNTATVLDSDGSYFMYSKLRVQKSTWERGSLFACSVVHEVLHNHLTTKTISRSLGK

SEQ ID NO: 126 - protein, 350 aa, synthetic construct
MAQLLFNKTKSVEFTFCNDTVVIPCFVTNMEAQNTTEVYVKWKFKGRDIYTFDGALNKSTVPTDFSSAKIEVSQLLKGDASLKMDKSDAVSHTGNYTCEVTELTREGETIIELKYRVVSWFSPNEDKTHTCPPCPPDLLGGPSVFIFPPKIKDVLMISLSPMVTCVVVDVSEDDPDVQISWFVNNVEVHTAQTQTHREDYNSTLRVVSALPIQHQDWMSGKEFKCKVNNRALPSPIEKTISKPRPVRAPQVYVLPPPAEEMTKKEFSLTCMITGFLPAEIAVDWTSNGRTEQNYKNTATVLDSDGSYFMYSKLRVQKSTWERGSLFACSVVHEVLHNHLTTKTISRSLGK

SEQ ID NO: 127 - protein, 487 aa, synthetic construct
MAVPRWRQQWSGPGTTKRFPETVLARCVKYTEIHPEMRHVDCQSVWDAFKGAFISKHPCNITEEDYQPLMKLGTQTVPCNKILLWSRIKDLAHQFTQVQRDMFTLEDTLLGYLADDLTWCGEFNTSKINYQSCPDWRKDCSNNPVSVFWKTVSRRFAEAACDVVHVMLNGSRSKIFDKNSTFGSVEVHNLQPEKVQTLEAWVIHGGREDSRDLCQDPTIKELESIISKRNIQFSCKNIYRPDKFLQCVKNPEDSSCTSEIAAASPPCKCPAPDLLGGPSVFIFPPKIKDVLMISLSPMVTCVVVDVSEDDPDVQISWFVNNVEVHTAQTQTHREDYNSTLRVVSALPIQHQDWMSGKEFKCKVNNRALPSPIEKTISKPRGPVRAPQVYVLPPPAEEMTKKEFSLTCMITGFLPAEIAVDWTSNGRTEQNYKNTATVLDSDGSYFMYSKLRVQKSTWERGSLFACSVVHEGLHNHLTTKTISRSLGK

SEQ ID NO: 128 - protein, 487 aa, synthetic construct
MAVPRWRQQWSGPGTTKRFPETVLARCVKYTEIHPEMRHVDCQSVWDAFKGAFISKHPCNITEEDYQPLMKLGTQTVPCNKKLLWSRIKDLAHQFTQVQRDMFTLEDTLLGYLADDLTWCGEFNTSKINYQSCPDWRKDCSNNPVSVFWKTVSRRFAEAACDVVHVMLNGSRSKIFDKNSTFGSVEVHNLQPEKVQTLEAWVIHGGREDSRDLCQDPTIKELESIISKRNIQFSCKNIYRPDKFLQCVKNPEDSSCTSEIAAASPPCKCPAPDLLGGPSVFIFPPKIKDVLMISLSPMVTCVVVDVSEDDPDVQISWFVNNVEVHTAQTQTHREDYNSTLRVVSALPIQHQDWMSGKEFKCKVNNRALPSPIEKTISKPRGPVRAPQVYVLPPPAEEMTKKEFSLTCMITGFLPAEIAVDWTSNGRTEQNYKNTATVLDSDGSYFMYSKLRVQKSTWERGSLFACSVVHEGLHNHLTTKTISRSLGK

SEQ ID NO: 129 - protein, 352 aa, synthetic construct
MAQLLFNKTKSVEFTFCNDTVVIPCFVTNMEAQNTTEVYVKWKFKGRDIYTFDGALNKSTVPTDFSSAKIEVSQLLKGDASLKMDKSDAVSHTGNYTCEVTELTREGETIIELKYRVVSWFSPNEAAASPPCKCPAPDLLGGPSVFIFPPKIKDVLMISLSPMVTCVVVDVSEDDPDVQISWFVNNVEVHTAQTQTHREDYNSTLRVVSALPIQHQDWMSGKEFKCKVNNRALPSPIEKTISKPRGPVRAPQVYVLPPPAEEMTKKEFSLTCMITGFLPAEIAVDWTSNGRTEQNYKNTATVLDSDGSYFMYSKLRVQKSTWERGSLFACSVVHEGLHNHLTTKTISRSLGK

SEQ ID NO: 130 - protein, 487 aa, synthetic construct
MAVPRWRQQWSGPGTTKRFPETVLARCVKYTEIHPEMRHVDCQSVWDAFKGAFISKHPCNITEEDYQPLMKLGTQTVPCNKILLWSRIKDLAHQFTQVQRDMFTLEDTLLGYLADDLTWCGEFNTSKINYQSCPDWRKDCSNNPVSVFWKTVSRRFAEAACDVVHVMLNGSRSKIFDKNSTFGSVEVHNLQPEKVQTLEAWVIHGGREDSRDLCQDPTIKELESIISKRNIQFSCKNIYRPDKFLQCVKNPEDSSCTSEIGGGSPPCKCPAPDLLGGPSVFIFPPKIKDVLMISLSPMVTCVVVDVSEDDPDVQISWFVNNVEVHTAQTQTHREDYNSTLRVVSALPIQHQDWMSGKEFKCKVNNRALPSPIEKTISKPRGPVRAPQVYVLPPPAEEMTKKEFSLTCMITGFLPAEIAVDWTSNGRTEQNYKNTATVLDSDGSYFMYSKLRVQKSTWERGSLFACSVVHEGLHNHLTTKTISRSLGK

SEQ ID NO: 131 - protein, 487 aa, synthetic construct
MAVPRWRQQWSGPGTTKRFPETVLARCVKYTEIHPEMRHVDCQSVWDAFKGAFISKHPCNITEEDYQPLMKLGTQTVPCNKKLLWSRIKDLAHQFTQVQRDMFTLEDTLLGYLADDLTWCGEFNTSKINYQSCPDWRKDCSNNPVSVFWKTVSRRFAEAACDVVHVMLNGSRSKIFDKNSTFGSVEVHNLQPEKVQTLEAWVIHGGREDSRDLCQDPTIKELESIISKRNIQFSCKNIYRPDKFLQCVKNPEDSSCTSEIGGGSPPCKCPAPDLLGGPSVFIFPPKIKDVLMISLSPMVTCVVVDVSEDDPDVQISWFVNNVEVHTAQTQTHREDYNSTLRVVSALPIQHQDWMSGKEFKCKVNNRALPSPIEKTISKPRGPVRAPQVYVLPPPAEEMTKKEFSLTCMITGFLPAEIAVDWTSNGRTEQNYKNTATVLDSDGSYFMYSKLRVQKSTWERGSLFACSVVHEGLHNHLTTKTISRSLGK

SEQ ID NO: 132 - protein, 352 aa, synthetic construct
MAQLLFNKTKSVEFTFCNDTVVIPCFVTNMEAQNTTEVYVKWKFKGRDIYTFDGALNKSTVPTDFSSAKIEVSQLLKGDASLKMDKSDAVSHTGNYTCEVTELTREGETIIELKYRVVSWFSPNEGGGSPPCKCPAPDLLGGPSVFIFPPKIKDVLMISLSPMVTCVVVDVSEDDPDVQISWFVNNVEVHTAQTQTHREDYNSTLRVVSALPIQHQDWMSGKEFKCKVNNRALPSPIEKTISKPRGPVRAPQVYVLPPPAEEMTKKEFSLTCMITGFLPAEIAVDWTSNGRTEQNYKNTATVLDSDGSYFMYSKLRVQKSTWERGSLFACSVVHEGLHNHLTTKTISRSLGK

SEQ ID NO: 133 - protein, 483 aa, synthetic construct
MAVPRWRQQWSGPGTTKRFPETVLARCVKYTEIHPEMRHVDCQSVWDAFKGAFISKHPCNITEEDYQPLMKLGTQTVPCNKILLWSRIKDLAHQFTQVQRDMFTLEDTLLGYLADDLTWCGEFNTSKINYQSCPDWRKDCSNNPVSVFWKTVSRRFAEAACDVVHVMLNGSRSKIFDKNSTFGSVEVHNLQPEKVQTLEAWVIHGGREDSRDLCQDPTIKELESIISKRNIQFSCKNIYRPDKFLQCVKNPEDSSCTSEIPPCKCPAPDLLGGPSVFIFPPKIKDVLMISLSPMVTCVVVDVSEDDPDVQISWFVNNVEVHTAQTQTHREDYNSTLRVVSALPIQHQDWMSGKEFKCKVNNRALPSPIEKTISKPRGPVRAPQVYVLPPPAEEMTKKEFSLTCMITGFLPAEIAVDWTSNGRTEQNYKNTATVLDSDGSYFMYSKLRVQKSTWERGSLFACSVVHEGLHNHLTTKTISRSLGK

SEQ ID NO: 134 - protein, 483 aa, synthetic construct
MAVPRWRQQWSGPGTTKRFPETVLARCVKYTEIHPEMRHVDCQSVWDAFKGAFISKHPCNITEEDYQPLMKLGTQTVPCNKKLLWSRIKDLAHQFTQVQRDMFTLEDTLLGYLADDLTWCGEFNTSKINYQSCPDWRKDCSNNPVSVFWKTVSRRFAEAACDVVHVMLNGSRSKIFDKNSTFGSVEVHNLQPEKVQTLEAWVIHGGREDSRDLCQDPTIKELESIISKRNIQFSCKNIYRPDKFLQCVKNPEDSSCTSEIPPCKCPAPDLLGGPSVFIFPPKIKDVLMISLSPMVTCVVVDVSEDDPDVQISWFVNNVEVHTAQTQTHREDYNSTLRVVSALPIQHQDWMSGKEFKCKVNNRALPSPIEKTISKPRGPVRAPQVYVLPPPAEEMTKKEFSLTCMITGFLPAEIAVDWTSNGRTEQNYKNTATVLDSDGSYFMYSKLRVQKSTWERGSLFACSVVHEGLHNHLTTKTISRSLGK

SEQ ID NO: 135 - protein, 348 aa, synthetic construct
MAQLLFNKTKSVEFTFCNDTVVIPCFVTNMEAQNTTEVYVKWKFKGRDIYTFDGALNKSTVPTDFSSAKIEVSQLLKGDASLKMDKSDAVSHTGNYTCEVTELTREGETIIELKYRVVSWFSPNEPPCKCPAPDLLGGPSVFIFPPKIKDVLMISLSPMVTCVVVDVSEDDPDVQISWFVNNVEVHTAQTQTHREDYNSTLRVVSALPIQHQDWMSGKEFKCKVNNRALPSPIEKTISKPRGPVRAPQVYVLPPPAEEMTKKEFSLTCMITGFLPAEIAVDWTSNGRTEQNYKNTATVLDSDGSYFMYSKLRVQKSTWERGSLFACSVVHEGLHNHLTTKTISRSLGK

SEQ ID NO: 136 - protein, 490 aa, synthetic construct
MAVPRWRQQWSGPGTTKRFPETVLARCVKYTEIHPEMRHVDCQSVWDAFKGAFISKHPCNITEEDYQPLMKLGTQTVPCNKILLWSRIKDLAHQFTQVQRDMFTLEDTLLGYLADDLTWCGEFNTSKINYQSCPDWRKDCSNNPVSVFWKTVSRRFAEAACDVVHVMLNGSRSKIFDKNSTFGSVEVHNLQPEKVQTLEAWVIHGGREDSRDLCQDPTIKELESIISKRNIQFSCKNIYRPDKFLQCVKNPEDSSCTSEIAAASPSTCSKPTCPPDLLGGPSVFIFPPKIKDVLMISLSPMVTCVVVDVSEDDPDVQISWFVNNVEVHTAQTQTHREDYNSTLRVVSALPIQHQDWMSGKEFKCKVNNRALPSPIEKTISKPRGPVRAPQVYVLPPPAEEMTKKEFSLTCMITGFLPAEIAVDWTSNGRTEQNYKNTATVLDSDGSYFMYSKLRVQKSTWERGSLFACSVVHEGLHNHLTTKTISRSLGK

SEQ ID NO: 137 - protein, 490 aa, synthetic construct
MAVPRWRQQWSGPGTTKRFPETVLARCVKYTEIHPEMRHVDCQSVWDAFKGAFISKHPCNITEEDYQPLMKLGTQTVPCNKKLLWSRIKDLAHQFTQVQRDMFTLEDTLLGYLADDLTWCGEFNTSKINYQSCPDWRKDCSNNPVSVFWKTVSRRFAEAACDVVHVMLNGSRSKIFDKNSTFGSVEVHNLQPEKVQTLEAWVIHGGREDSRDLCQDPTIKELESIISKRNIQFSCKNIYRPDKFLQCVKNPEDSSCTSEIAAASPSTCSKPTCPPDLLGGPSVFIFPPKIKDVLMISLSPMVTCVVVDVSEDDPDVQISWFVNNVEVHTAQTQTHREDYNSTLRVVSALPIQHQDWMSGKEFKCKVNNRALPSPIEKTISKPRGPVRAPQVYVLPPPAEEMTKKEFSLTCMITGFLPAEIAVDWTSNGRTEQNYKNTATVLDSDGSYFMYSKLRVQKSTWERGSLFACSVVHEGLHNHLTTKTISRSLGK

SEQ ID NO: 138 - protein, 355 aa, synthetic construct
MAQLLFNKTKSVEFTFCNDTVVIPCFVTNMEAQNTTEVYVKWKFKGRDIYTFDGALNKSTVPTDFSSAKIEVSQLLKGDASLKMDKSDAVSHTGNYTCEVTELTREGETIIELKYRVVSWFSPNEAAASPSTCSKPTCPPDLLGGPSVFIFPPKIKDVLMISLSPMVTCVVVDVSEDDPDVQISWFVNNVEVHTAQTQTHREDYNSTLRVVSALPIQHQDWMSGKEFKCKVNNRALPSPIEKTISKPRGPVRAPQVYVLPPPAEEMTKKEFSLTCMITGFLPAEIAVDWTSNGRTEQNYKNTATVLDSDGSYFMYSKLRVQKSTWERGSLFACSVVHEGLHNHLTTKTISRSLGK

SEQ ID NO: 139 - protein, 490 aa, synthetic construct
MAVPRWRQQWSGPGTTKRFPETVLARCVKYTEIHPEMRHVDCQSVWDAFKGAFISKHPCNITEEDYQPLMKLGTQTVPCNKILLWSRIKDLAHQFTQVQRDMFTLEDTLLGYLADDLTWCGEFNTSKINYQSCPDWRKDCSNNPVSVFWKTVSRRFAEAACDVVHVMLNGSRSKIFDKNSTFGSVEVHNLQPEKVQTLEAWVIHGGREDSRDLCQDPTIKELESIISKRNIQFSCKNIYRPDKFLQCVKNPEDSSCTSEIGGGSPSTCSKPTCPPDLLGGPSVFIFPPKIKDVLMISLSPMVTCVVVDVSEDDPDVQISWFVNNVEVHTAQTQTHREDYNSTLRVVSALPIQHQDWMSGKEFKCKVNNRALPSPIEKTISKPRGPVRAPQVYVLPPPAEEMTKKEFSLTCMITGFLPAEIAVDWTSNGRTEQNYKNTATVLDSDGSYFMYSKLRVQKSTWERGSLFACSVVHEGLHNHLTTKTISRSLGK

SEQ ID NO: 140 - protein, 490 aa, synthetic construct
MAVPRWRQQWSGPGTTKRFPETVLARCVKYTEIHPEMRHVDCQSVWDAFKGAFISKHPCNITEEDYQPLMKLGTQTVPCNKKLLWSRIKDLAHQFTQVQRDMFTLEDTLLGYLADDLTWCGEFNTSKINYQSCPDWRKDCSNNPVSVFWKTVSRRFAEAACDVVHVMLNGSRSKIFDKNSTFGSVEVHNLQPEKVQTLEAWVIHGGREDSRDLCQDPTIKELESIISKRNIQFSCKNIYRPDKFLQCVKNPEDSSCTSEIGGGSPSTCSKPTCPPDLLGGPSVFIFPPKIKDVLMISLSPMVTCVVVDVSEDDPDVQISWFVNNVEVHTAQTQTHREDYNSTLRVVSALPIQHQDWMSGKEFKCKVNNRALPSPIEKTISKPRGPVRAPQVYVLPPPAEEMTKKEFSLTCMITGFLPAEIAVDWTSNGRTEQNYKNTATVLDSDGSYFMYSKLRVQKSTWERGSLFACSVVHEGLHNHLTTKTISRSLGK

SEQ ID NO: 141 - protein, 355 aa, synthetic construct
MAQLLFNKTKSVEFTFCNDTVVIPCFVTNMEAQNTTEVYVKWKFKGRDIYTFDGALNKSTVPTDFSSAKIEVSQLLKGDASLKMDKSDAVSHTGNYTCEVTELTREGETIIELKYRVVSWFSPNEGGGSPSTCSKPTCPPDLLGGPSVFIFPPKIKDVLMISLSPMVTCVVVDVSEDDPDVQISWFVNNVEVHTAQTQTHREDYNSTLRVVSALPIQHQDWMSGKEFKCKVNNRALPSPIEKTISKPRGPVRAPQVYVLPPPAEEMTKKEFSLTCMITGFLPAEIAVDWTSNGRTEQNYKNTATVLDSDGSYFMYSKLRVQKSTWERGSLFACSVVHEGLHNHLTTKTISRSLGK

SEQ ID NO: 142 - protein, 486 aa, synthetic construct
MAVPRWRQQWSGPGTTKRFPETVLARCVKYTEIHPEMRHVDCQSVWDAFKGAFISKHPCNITEEDYQPLMKLGTQTVPCNKILLWSRIKDLAHQFTQVQRDMFTLEDTLLGYLADDLTWCGEFNTSKINYQSCPDWRKDCSNNPVSVFWKTVSRRFAEAACDVVHVMLNGSRSKIFDKNSTFGSVEVHNLQPEKVQTLEAWVIHGGREDSRDLCQDPTIKELESIISKRNIQFSCKNIYRPDKFLQCVKNPEDSSCTSEIPSTCSKPTCPPDLLGGPSVFIFPPKIKDVLMISLSPMVTCVVVDVSEDDPDVQISWFVNNVEVHTAQTQTHREDYNSTLRVVSALPIQHQDWMSGKEFKCKVNNRALPSPIEKTISKPRGPVRAPQVYVLPPPAEEMTKKEFSLTCMITGFLPAEIAVDWTSNGRTEQNYKNTATVLDSDGSYFMYSKLRVQKSTWERGSLFACSVVHEGLHNHLTTKTISRSLGK

SEQ ID NO: 143 - protein, 486 aa, synthetic construct
MAVPRWRQQWSGPGTTKRFPETVLARCVKYTEIHPEMRHVDCQSVWDAFKGAFISKHPCNITEEDYQPLMKLGTQTVPCNKKLLWSRIKDLAHQFTQVQRDMFTLEDTLLGYLADDLTWCGEFNTSKINYQSCPDWRKDCSNNPVSVFWKTVSRRFAEAACDVVHVMLNGSRSKIFDKNSTFGSVEVHNLQPEKVQTLEAWVIHGGREDSRDLCQDPTIKELESIISKRNIQFSCKNIYRPDKFLQCVKNPEDSSCTSEIPSTCSKPTCPPDLLGGPSVFIFPPKIKDVLMISLSPMVTCVVVDVSEDDPDVQISWFVNNVEVHTAQTQTHREDYNSTLRVVSALPIQHQDWMSGKEFKCKVNNRALPSPIEKTISKPRGPVRAPQVYVLPPPAEEMTKKEFSLTCMITGFLPAEIAVDWTSNGRTEQNYKNTATVLDSDGSYFMYSKLRVQKSTWERGSLFACSVVHEGLHNHLTTKTISRSLGK

SEQ ID NO: 144 - protein, 351 aa, synthetic construct
MAQLLFNKTKSVEFTFCNDTVVIPCFVTNMEAQNTTEVYVKWKFKGRDIYTFDGALNKSTVPTDFSSAKIEVSQLLKGDASLKMDKSDAVSHTGNYTCEVTELTREGETIIELKYRVVSWFSPNEPSTCSKPTCPPDLLGGPSVFIFPPKIKDVLMISLSPMVTCVVVDVSEDDPDVQISWFVNNVEVHTAQTQTHREDYNSTLRVVSALPIQHQDWMSGKEFKCKVNNRALPSPIEKTISKPRGPVRAPQVYVLPPPAEEMTKKEFSLTCMITGFLPAEIAVDWTSNGRTEQNYKNTATVLDSDGSYFMYSKLRVQKSTWERGSLFACSVVHEGLHNHLTTKTISRSLGK

SEQ ID NO: 145 - protein, 486 aa, synthetic construct
MAVPRWRQQWSGPGTTKRFPETVLARCVKYTEIHPEMRHVDCQSVWDAFKGAFISKHPCNITEEDYQPLMKLGTQTVPCNKILLWSRIKDLAHQFTQVQRDMFTLEDTLLGYLADDLTWCGEFNTSKINYQSCPDWRKDCSNNPVSVFWKTVSRRFAEAACDVVHVMLNGSRSKIFDKNSTFGSVEVHNLQPEKVQTLEAWVIHGGREDSRDLCQDPTIKELESIISKRNIQFSCKNIYRPDKFLQCVKNPEDSSCTSEIAAASNPCGCTPDLLGGPSVFIFPPKIKDVLMISLSPMVTCVVVDVSEDDPDVQISWFVNNVEVHTAQTQTHREDYNSTLRVVSALPIQHQDWMSGKEFKCKVNNRALPSPIEKTISKPRGPVRAPQVYVLPPPAEEMTKKEFSLTCMITGFLPAEIAVDWTSNGRTEQNYKNTATVLDSDGSYFMYSKLRVQKSTWERGSLFACSVVHEGLHNHLTTKTISRSLGK

SEQ ID NO: 146 - protein, 486 aa, synthetic construct
MAVPRWRQQWSGPGTTKRFPETVLARCVKYTEIHPEMRHVDCQSVWDAFKGAFISKHPCNITEEDYQPLMKLGTQTVPCNKKLLWSRIKDLAHQFTQVQRDMFTLEDTLLGYLADDLTWCGEFNTSKINYQSCPDWRKDCSNNPVSVFWKTVSRRFAEAACDVVHVMLNGSRSKIFDKNSTFGSVEVHNLQPEKVQTLEAWVIHGGREDSRDLCQDPTIKELESIISKRNIQFSCKNIYRPDKFLQCVKNPEDSSCTSEIAAASNPCGCTPDLLGGPSVFIFPPKIKDVLMISLSPMVTCVVVDVSEDDPDVQISWFVNNVEVHTAQTQTHREDYNSTLRVVSALPIQHQDWMSGKEFKCKVNNRALPSPIEKTISKPRGPVRAPQVYVLPPPAEEMTKKEFSLTCMITGFLPAEIAVDWTSNGRTEQNYKNTATVLDSDGSYFMYSKLRVQKSTWERGSLFACSVVHEGLHNHLTTKTISRSLGK

SEQ ID NO: 147 - protein, 351 aa, synthetic construct
MAQLLFNKTKSVEFTFCNDTVVIPCFVTNMEAQNTTEVYVKWKFKGRDIYTFDGALNKSTVPTDFSSAKIEVSQLLKGDASLKMDKSDAVSHTGNYTCEVTELTREGETIIELKYRVVSWFSPNEAAASNPCGCTPDLLGGPSVFIFPPKIKDVLMISLSPMVTCVVVDVSEDDPDVQISWFVNNVEVHTAQTQTHREDYNSTLRVVSALPIQHQDWMSGKEFKCKVNNRALPSPIEKTISKPRGPVRAPQVYVLPPPAEEMTKKEFSLTCMITGFLPAEIAVDWTSNGRTEQNYKNTATVLDSDGSYFMYSKLRVQKSTWERGSLFACSVVHEGLHNHLTTKTISRSLGK

SEQ ID NO: 148 - protein, 486 aa, synthetic construct
MAVPRWRQQWSGPGTTKRFPETVLARCVKYTEIHPEMRHVDCQSVWDAFKGAFISKHPCNITEEDYQPLMKLGTQTVPCNKILLWSRIKDLAHQFTQVQRDMFTLEDTLLGYLADDLTWCGEFNTSKINYQSCPDWRKDCSNNPVSVFWKTVSRRFAEAACDVVHVMLNGSRSKIFDKNSTFGSVEVHNLQPEKVQTLEAWVIHGGREDSRDLCQDPTIKELESIISKRNIQFSCKNIYRPDKFLQCVKNPEDSSCTSEIGGGSNPCGCTPDLLGGPSVFIFPPKIKDVLMISLSPMVTCVVVDVSEDDPDVQISWFVNNVEVHTAQTQTHREDYNSTLRVVSALPIQHQDWMSGKEFKCKVNNRALPSPIEKTISKPRGPVRAPQVYVLPPPAEEMTKKEFSLTCMITGFLPAEIAVDWTSNGRTEQNYKNTATVLDSDGSYFMYSKLRVQKSTWERGSLFACSVVHEGLHNHLTTKTISRSLGK

SEQ ID NO: 149 - protein, 486 aa, synthetic construct
MAVPRWRQQWSGPGTTKRFPETVLARCVKYTEIHPEMRHVDCQSVWDAFKGAFISKHPCNITEEDYQPLMKLGTQTVPCNKKLLWSRIKDLAHQFTQVQRDMFTLEDTLLGYLADDLTWCGEFNTSKINYQSCPDWRKDCSNNPVSVFWKTVSRRFAEAACDVVHVMLNGSRSKIFDKNSTFGSVEVHNLQPEKVQTLEAWVIHGGREDSRDLCQDPTIKELESIISKRNIQFSCKNIYRPDKFLQCVKNPEDSSCTSEIGGGSNPCGCTPDLLGGPSVFIFPPKIKDVLMISLSPMVTCVVVDVSEDDPDVQISWFVNNVEVHTAQTQTHREDYNSTLRVVSALPIQHQDWMSGKEFKCKVNNRALPSPIEKTISKPRGPVRAPQVYVLPPPAEEMTKKEFSLTCMITGFLPAEIAVDWTSNGRTEQNYKNTATVLDSDGSYFMYSKLRVQKSTWERGSLFACSVVHEGLHNHLTTKTISRSLGK

SEQ ID NO: 150 - protein, 351 aa, synthetic construct
MAQLLFNKTKSVEFTFCNDTVVIPCFVTNMEAQNTTEVYVKWKFKGRDIYTFDGALNKSTVPTDFSSAKIEVSQLLKGDASLKMDKSDAVSHTGNYTCEVTELTREGETIIELKYRVVSWFSPNEGGGSNPCGCTPDLLGGPSVFIFPPKIKDVLMISLSPMVTCVVVDVSEDDPDVQISWFVNNVEVHTAQTQTHREDYNSTLRVVSALPIQHQDWMSGKEFKCKVNNRALPSPIEKTISKPRGPVRAPQVYVLPPPAEEMTKKEFSLTCMITGFLPAEIAVDWTSNGRTEQNYKNTATVLDSDGSYFMYSKLRVQKSTWERGSLFACSVVHEGLHNHLTTKTISRSLGK

SEQ ID NO: 151 - protein, 482 aa, synthetic construct
MAVPRWRQQWSGPGTTKRFPETVLARCVKYTEIHPEMRHVDCQSVWDAFKGAFISKHPCNITEEDYQPLMKLGTQTVPCNKILLWSRIKDLAHQFTQVQRDMFTLEDTLLGYLADDLTWCGEFNTSKINYQSCPDWRKDCSNNPVSVFWKTVSRRFAEAACDVVHVMLNGSRSKIFDKNSTFGSVEVHNLQPEKVQTLEAWVIHGGREDSRDLCQDPTIKELESIISKRNIQFSCKNIYRPDKFLQCVKNPEDSSCTSEINPCGCTPDLLGGPSVFIFPPKIKDVLMISLSPMVTCVVVDVSEDDPDVQISWFVNNVEVHTAQTQTHREDYNSTLRVVSALPIQHQDWMSGKEFKCKVNNRALPSPIEKTISKPRGPVRAPQVYVLPPPAEEMTKKEFSLTCMITGFLPAEIAVDWTSNGRTEQNYKNTATVLDSDGSYFMYSKLRVQKSTWERGSLFACSVVHEGLHNHLTTKTISRSLGK

SEQ ID NO: 152 - protein, 482 aa, synthetic construct
MAVPRWRQQWSGPGTTKRFPETVLARCVKYTEIHPEMRHVDCQSVWDAFKGAFISKHPCNITEEDYQPLMKLGTQTVPCNKKLLWSRIKDLAHQFTQVQRDMFTLEDTLLGYLADDLTWCGEFNTSKINYQSCPDWRKDCSNNPVSVFWKTVSRRFAEAACDVVHVMLNGSRSKIFDKNSTFGSVEVHNLQPEKVQTLEAWVIHGGREDSRDLCQDPTIKELESIISKRNIQFSCKNIYRPDKFLQCVKNPEDSSCTSEINPCGCTPDLLGGPSVFIFPPKIKDVLMISLSPMVTCVVVDVSEDDPDVQISWFVNNVEVHTAQTQTHREDYNSTLRVVSALPIQHQDWMSGKEFKCKVNNRALPSPIEKTISKPRGPVRAPQVYVLPPPAEEMTKKEFSLTCMITGFLPAEIAVDWTSNGRTEQNYKNTATVLDSDGSYFMYSKLRVQKSTWERGSLFACSVVHEGLHNHLTTKTISRSLGK

SEQ ID NO: 153 - protein, 347 aa, synthetic construct
MAQLLFNKTKSVEFTFCNDTVVIPCFVTNMEAQNTTEVYVKWKFKGRDIYTFDGALNKSTVPTDFSSAKIEVSQLLKGDASLKMDKSDAVSHTGNYTCEVTELTREGETIIELKYRVVSWFSPNENPCGCTPDLLGGPSVFIFPPKIKDVLMISLSPMVTCVVVDVSEDDPDVQISWFVNNVEVHTAQTQTHREDYNSTLRVVSALPIQHQDWMSGKEFKCKVNNRALPSPIEKTISKPRGPVRAPQVYVLPPPAEEMTKKEFSLTCMITGFLPAEIAVDWTSNGRTEQNYKNTATVLDSDGSYFMYSKLRVQKSTWERGSLFACSVVHEGLHNHLTTKTISRSLGK

SEQ ID NO: 154 - protein, 490 aa, synthetic construct
MAVPRWRQQWSGPGTTKRFPETVLARCVKYTEIHPEMRHVDCQSVWDAFKGAFISKHPCNITEEDYQPLMKLGTQTVPCNKILLWSRIKDLAHQFTQVQRDMFTLEDTLLGYLADDLTWCGEFNTSKINYQSCPDWRKDCSNNPVSVFWKTVSRRFAEAACDVVHVMLNGSRSKIFDKNSTFGSVEVHNLQPEKVQTLEAWVIHGGREDSRDLCQDPTIKELESIISKRNIQFSCKNIYRPDKFLQCVKNPEDSSCTSEIAAASDKTHTCPPCPPDLLGGPSVFIFPPKIKDVLMISLSPMVTCVVVDVSEDDPDVQISWFVNNVEVHTAQTQTHREDYNSTLRVVSALPIQHQDWMSGKEFKCKVNNRALPSPIEKTISKPRGPVRAPQVYVLPPPAEEMTKKEFSLTCMITGFLPAEIAVDWTSNGRTEQNYKNTATVLDSDGSYFMYSKLRVQKSTWERGSLFACSVVHEGLHNHLTTKTISRSLGK

SEQ ID NO: 155 - protein, 490 aa, synthetic construct
MAVPRWRQQWSGPGTTKRFPETVLARCVKYTEIHPEMRHVDCQSVWDAFKGAFISKHPCNITEEDYQPLMKLGTQTVPCNKKLLWSRIKDLAHQFTQVQRDMFTLEDTLLGYLADDLTWCGEFNTSKINYQSCPDWRKDCSNNPVSVFWKTVSRRFAEAACDVVHVMLNGSRSKIFDKNSTFGSVEVHNLQPEKVQTLEAWVIHGGREDSRDLCQDPTIKELESIISKRNIQFSCKNIYRPDKFLQCVKNPEDSSCTSEIAAASDKTHTCPPCPPDLLGGPSVFIFPPKIKDVLMISLSPMVTCVVVDVSEDDPDVQISWFVNNVEVHTAQTQTHREDYNSTLRVVSALPIQHQDWMSGKEFKCKVNNRALPSPIEKTISKPRGPVRAPQVYVLPPPAEEMTKKEFSLTCMITGFLPAEIAVDWTSNGRTEQNYKNTATVLDSDGSYFMYSKLRVQKSTWERGSLFACSVVHEGLHNHLTTKTISRSLGK

SEQ ID NO: 156 - protein, 355 aa, synthetic construct
MAQLLFNKTKSVEFTFCNDTVVIPCFVTNMEAQNTTEVYVKWKFKGRDIYTFDGALNKSTVPTDFSSAKIEVSQLLKGDASLKMDKSDAVSHTGNYTCEVTELTREGETIIELKYRVVSWFSPNEAAASDKTHTCPPCPPDLLGGPSVFIFPPKIKDVLMISLSPMVTCVVVDVSEDDPDVQISWFVNNVEVHTAQTQTHREDYNSTLRVVSALPIQHQDWMSGKEFKCKVNNRALPSPIEKTISKPRGPVRAPQVYVLPPPAEEMTKKEFSLTCMITGFLPAEIAVDWTSNGRTEQNYKNTATVLDSDGSYFMYSKLRVQKSTWERGSLFACSVVHEGLHNHLTTKTISRSLGK

SEQ ID NO: 157 - protein, 490 aa, synthetic construct
MAVPRWRQQWSGPGTTKRFPETVLARCVKYTEIHPEMRHVDCQSVWDAFKGAFISKHPCNITEEDYQPLMKLGTQTVPCNKILLWSRIKDLAHQFTQVQRDMFTLEDTLLGYLADDLTWCGEFNTSKINYQSCPDWRKDCSNNPVSVFWKTVSRRFAEAACDVVHVMLNGSRSKIFDKNSTFGSVEVHNLQPEKVQTLEAWVIHGGREDSRDLCQDPTIKELESIISKRNIQFSCKNIYRPDKFLQCVKNPEDSSCTSEIGGGSDKTHTCPPCPPDLLGGPSVFIFPPKIKDVLMISLSPMVTCVVVDVSEDDPDVQISWFVNNVEVHTAQTQTHREDYNSTLRVVSALPIQHQDWMSGKEFKCKVNNRALPSPIEKTISKPRGPVRAPQVYVLPPPAEEMTKKEFSLTCMITGFLPAEIAVDWTSNGRTEQNYKNTATVLDSDGSYFMYSKLRVQKSTWERGSLFACSVVHEGLHNHLTTKTISRSLGK

SEQ ID NO: 158 - protein, 490 aa, synthetic construct
MAVPRWRQQWSGPGTTKRFPETVLARCVKYTEIHPEMRHVDCQSVWDAFKGAFISKHPCNITEEDYQPLMKLGTQTVPCNKKLLWSRIKDLAHQFTQVQRDMFTLEDTLLGYLADDLTWCGEFNTSKINYQSCPDWRKDCSNNPVSVFWKTVSRRFAEAACDVVHVMLNGSRSKIFDKNSTFGSVEVHNLQPEKVQTLEAWVIHGGREDSRDLCQDPTIKELESIISKRNIQFSCKNIYRPDKFLQCVKNPEDSSCTSEIGGGSDKTHTCPPCPPDLLGGPSVFIFPPKIKDVLMISLSPMVTCVVVDVSEDDPDVQISWFVNNVEVHTAQTQTHREDYNSTLRVVSALPIQHQDWMSGKEFKCKVNNRALPSPIEKTISKPRGPVRAPQVYVLPPPAEEMTKKEFSLTCMITGFLPAEIAVDWTSNGRTEQNYKNTATVLDSDGSYFMYSKLRVQKSTWERGSLFACSVVHEGLHNHLTTKTISRSLGK

SEQ ID NO: 159 - protein, 355 aa, synthetic construct
MAQLLFNKTKSVEFTFCNDTVVIPCFVTNMEAQNTTEVYVKWKFKGRDIYTFDGALNKSTVPTDFSSAKIEVSQLLKGDASLKMDKSDAVSHTGNYTCEVTELTREGETIIELKYRVVSWFSPNEGGGSDKTHTCPPCPPDLLGGPSVFIFPPKIKDVLMISLSPMVTCVVVDVSEDDPDVQISWFVNNVEVHTAQTQTHREDYNSTLRVVSALPIQHQDWMSGKEFKCKVNNRALPSPIEKTISKPRGPVRAPQVYVLPPPAEEMTKKEFSLTCMITGFLPAEIAVDWTSNGRTEQNYKNTATVLDSDGSYFMYSKLRVQKSTWERGSLFACSVVHEGLHNHLTTKTISRSLGK

SEQ ID NO: 160 - protein, 486 aa, synthetic construct
MAVPRWRQQWSGPGTTKRFPETVLARCVKYTEIHPEMRHVDCQSVWDAFKGAFISKHPCNITEEDYQPLMKLGTQTVPCNKILLWSRIKDLAHQFTQVQRDMFTLEDTLLGYLADDLTWCGEFNTSKINYQSCPDWRKDCSNNPVSVFWKTVSRRFAEAACDVVHVMLNGSRSKIFDKNSTFGSVEVHNLQPEKVQTLEAWVIHGGREDSRDLCQDPTIKELESIISKRNIQFSCKNIYRPDKFLQCVKNPEDSSCTSEIDKTHTCPPCPPDLLGGPSVFIFPPKIKDVLMISLSPMVTCVVVDVSEDDPDVQISWFVNNVEVHTAQTQTHREDYNSTLRVVSALPIQHQDWMSGKEFKCKVNNRALPSPIEKTISKPRGPVRAPQVYVLPPPAEEMTKKEFSLTCMITGFLPAEIAVDWTSNGRTEQNYKNTATVLDSDGSYFMYSKLRVQKSTWERGSLFACSVVHEGLHNHLTTKTISRSLGK

SEQ ID NO: 161 - protein, 486 aa, synthetic construct
MAVPRWRQQWSGPGTTKRFPETVLARCVKYTEIHPEMRHVDCQSVWDAFKGAFISKHPCNITEEDYQPLMKLGTQTVPCNKKLLWSRIKDLAHQFTQVQRDMFTLEDTLLGYLADDLTWCGEFNTSKINYQSCPDWRKDCSNNPVSVFWKTVSRRFAEAACDVVHVMLNGSRSKIFDKNSTFGSVEVHNLQPEKVQTLEAWVIHGGREDSRDLCQDPTIKELESIISKRNIQFSCKNIYRPDKFLQCVKNPEDSSCTSEIDKTHTCPPCPPDLLGGPSVFIFPPKIKDVLMISLSPMVTCVVVDVSEDDPDVQISWFVNNVEVHTAQTQTHREDYNSTLRVVSALPIQHQDWMSGKEFKCKVNNRALPSPIEKTISKPRGPVRAPQVYVLPPPAEEMTKKEFSLTCMITGFLPAEIAVDWTSNGRTEQNYKNTATVLDSDGSYFMYSKLRVQKSTWERGSLFACSVVHEGLHNHLTTKTISRSLGK

SEQ ID NO: 162 - protein, 351 aa, synthetic construct
MAQLLFNKTKSVEFTFCNDTVVIPCFVTNMEAQNTTEVYVKWKFKGRDIYTFDGALNKSTVPTDFSSAKIEVSQLLKGDASLKMDKSDAVSHTGNYTCEVTELTREGETIIELKYRVVSWFSPNEDKTHTCPPCPPDLLGGPSVFIFPPKIKDVLMISLSPMVTCVVVDVSEDDPDVQISWFVNNVEVHTAQTQTHREDYNSTLRVVSALPIQHQDWMSGKEFKCKVNNRALPSPIEKTISKPRGPVRAPQVYVLPPPAEEMTKKEFSLTCMITGFLPAEIAVDWTSNGRTEQNYKNTATVLDSDGSYFMYSKLRVQKSTWERGSLFACSVVHEGLHNHLTTKTISRSLGK

SEQ ID NO: 163 - protein, 486 aa, synthetic construct
MAVPRWRQQWSGPGTTKRFPETVLARCVKYTEIHPEMRHVDCQSVWDAFKGAFISKHPCNITEEDYQPLMKLGTQTVPCNKILLWSRIKDLAHQFTQVQRDMFTLEDTLLGYLADDLTWCGEFNTSKINYQSCPDWRKDCSNNPVSVFWKTVSRRFAEAACDVVHVMLNGSRSKIFDKNSTFGSVEVHNLQPEKVQTLEAWVIHGGREDSRDLCQDPTIKELESIISKRNIQFSCKNIYRPDKFLQCVKNPEDSSCTSEIAAASPPCKCPAPELLGGPSVFIFPPKPKDTLMISRTPEVTCVVVDVSEDDPEVQFTWYINNEQVRTARPPLREQQFNSTIRVVSTLPIAHEDWLRGKEFKCKVHNKALPAPIEKTISKARQPLEPKVYTMGPPREELSSRSVSLTCMINGFYPSDISVEWEKNGKAEDNYKTTPAVLDSDGSYFLYSKLSVPTSEWQRGDVFTCSVMHEALHNHYTQKSISRSPGK

SEQ ID NO: 164 - protein, 486 aa, synthetic construct
MAVPRWRQQWSGPGTTKRFPETVLARCVKYTEIHPEMRHVDCQSVWDAFKGAFISKHPCNITEEDYQPLMKLGTQTVPCNKKLLWSRIKDLAHQFTQVQRDMFTLEDTLLGYLADDLTWCGEFNTSKINYQSCPDWRKDCSNNPVSVFWKTVSRRFAEAACDVVHVMLNGSRSKIFDKNSTFGSVEVHNLQPEKVQTLEAWVIHGGREDSRDLCQDPTIKELESIISKRNIQFSCKNIYRPDKFLQCVKNPEDSSCTSEIAAASPPCKCPAPELLGGPSVFIFPPKPKDTLMISRTPEVTCVVVDVSEDDPEVQFTWYINNEQVRTARPPLREQQFNSTIRVVSTLPIAHEDWLRGKEFKCKVHNKALPAPIEKTISKARQPLEPKVYTMGPPREELSSRSVSLTCMINGFYPSDISVEWEKNGKAEDNYKTTPAVLDSDGSYFLYSKLSVPTSEWQRGDVFTCSVMHEALHNHYTQKSISRSPGK

SEQ ID NO: 165 - protein, 351 aa, synthetic construct
MAQLLFNKTKSVEFTFCNDTVVIPCFVTNMEAQNTTEVYVKWKFKGRDIYTFDGALNKSTVPTDFSSAKIEVSQLLKGDASLKMDKSDAVSHTGNYTCEVTELTREGETIIELKYRVVSWFSPNEAAASPPCKCPAPELLGGPSVFIFPPKPKDTLMISRTPEVTCVVVDVSEDDPEVQFTWYINNEQVRTARPPLREQQFNSTIRVVSTLPIAHEDWLRGKEFKCKVHNKALPAPIEKTISKARQPLEPKVYTMGPPREELSSRSVSLTCMINGFYPSDISVEWEKNGKAEDNYKTTPAVLDSDGSYFLYSKLSVPTSEWQRGDVFTCSVMHEALHNHYTQKSISRSPGK

SEQ ID NO: 166 - protein, 486 aa, synthetic construct
MAVPRWRQQWSGPGTTKRFPETVLARCVKYTEIHPEMRHVDCQSVWDAFKGAFISKHPCNITEEDYQPLMKLGTQTVPCNKILLWSRIKDLAHQFTQVQRDMFTLEDTLLGYLADDLTWCGEFNTSKINYQSCPDWRKDCSNNPVSVFWKTVSRRFAEAACDVVHVMLNGSRSKIFDKNSTFGSVEVHNLQPEKVQTLEAWVIHGGREDSRDLCQDPTIKELESIISKRNIQFSCKNIYRPDKFLQCVKNPEDSSCTSEIGGGSPPCKCPAPELLGGPSVFIFPPKPKDTLMISRTPEVTCVVVDVSEDDPEVQFTWYINNEQVRTARPPLREQQFNSTIRVVSTLPIAHEDWLRGKEFKCKVHNKALPAPIEKTISKARQPLEPKVYTMGPPREELSSRSVSLTCMINGFYPSDISVEWEKNGKAEDNYKTTPAVLDSDGSYFLYSKLSVPTSEWQRGDVFTCSVMHEALHNHYTQKSISRSPGK

SEQ ID NO: 167 - protein, 486 aa, synthetic construct
MAVPRWRQQWSGPGTTKRFPETVLARCVKYTEIHPEMRHVDCQSVWDAFKGAFISKHPCNITEEDYQPLMKLGTQTVPCNKKLLWSRIKDLAHQFTQVQRDMFTLEDTLLGYLADDLTWCGEFNTSKINYQSCPDWRKDCSNNPVSVFWKTVSRRFAEAACDVVHVMLNGSRSKIFDKNSTFGSVEVHNLQPEKVQTLEAWVIHGGREDSRDLCQDPTIKELESIISKRNIQFSCKNIYRPDKFLQCVKNPEDSSCTSEIGGGSPPCKCPAPELLGGPSVFIFPPKPKDTLMISRTPEVTCVVVDVSEDDPEVQFTWYINNEQVRTARPPLREQQFNSTIRVVSTLPIAHEDWLRGKEFKCKVHNKALPAPIEKTISKARQPLEPKVYTMGPPREELSSRSVSLTCMINGFYPSDISVEWEKNGKAEDNYKTTPAVLDSDGSYFLYSKLSVPTSEWQRGDVFTCSVMHEALHNHYTQKSISRSPGK

SEQ ID NO: 168 - protein, 351 aa, synthetic construct
MAQLLFNKTKSVEFTFCNDTVVIPCFVTNMEAQNTTEVYVKWKFKGRDIYTFDGALNKSTVPTDFSSAKIEVSQLLKGDASLKMDKSDAVSHTGNYTCEVTELTREGETIIELKYRVVSWFSPNEGGGSPPCKCPAPELLGGPSVFIFPPKPKDTLMISRTPEVTCVVVDVSEDDPEVQFTWYINNEQVRTARPPLREQQFNSTIRVVSTLPIAHEDWLRGKEFKCKVHNKALPAPIEKTISKARQPLEPKVYTMGPPREELSSRSVSLTCMINGFYPSDISVEWEKNGKAEDNYKTTPAVLDSDGSYFLYSKLSVPTSEWQRGDVFTCSVMHEALHNHYTQKSISRSPGK

SEQ ID NO: 169 - protein, 482 aa, synthetic construct
MAVPRWRQQWSGPGTTKRFPETVLARCVKYTEIHPEMRHVDCQSVWDAFKGAFISKHPCNITEEDYQPLMKLGTQTVPCNKILLWSRIKDLAHQFTQVQRDMFTLEDTLLGYLADDLTWCGEFNTSKINYQSCPDWRKDCSNNPVSVFWKTVSRRFAEAACDVVHVMLNGSRSKIFDKNSTFGSVEVHNLQPEKVQTLEAWVIHGGREDSRDLCQDPTIKELESIISKRNIQFSCKNIYRPDKFLQCVKNPEDSSCTSEIPPCKCPAPELLGGPSVFIFPPKPKDTLMISRTPEVTCVVVDVSEDDPEVQFTWYINNEQVRTARPPLREQQFNSTIRVVSTLPIAHEDWLRGKEFKCKVHNKALPAPIEKTISKARQPLEPKVYTMGPPREELSSRSVSLTCMINGFYPSDISVEWEKNGKAEDNYKTTPAVLDSDGSYFLYSKLSVPTSEWQRGDVFTCSVMHEALHNHYTQKSISRSPGK

SEQ ID NO: 170 - protein, 482 aa, synthetic construct
MAVPRWRQQWSGPGTTKRFPETVLARCVKYTEIHPEMRHVDCQSVWDAFKGAFISKHPCNITEEDYQPLMKLGTQTVPCNKKLLWSRIKDLAHQFTQVQRDMFTLEDTLLGYLADDLTWCGEFNTSKINYQSCPDWRKDCSNNPVSVFWKTVSRRFAEAACDVVHVMLNGSRSKIFDKNSTFGSVEVHNLQPEKVQTLEAWVIHGGREDSRDLCQDPTIKELESIISKRNIQFSCKNIYRPDKFLQCVKNPEDSSCTSEIPPCKCPAPELLGGPSVFIFPPKPKDTLMISRTPEVTCVVVDVSEDDPEVQFTWYINNEQVRTARPPLREQQFNSTIRVVSTLPIAHEDWLRGKEFKCKVHNKALPAPIEKTISKARQPLEPKVYTMGPPREELSSRSVSLTCMINGFYPSDISVEWEKNGKAEDNYKTTPAVLDSDGSYFLYSKLSVPTSEWQRGDVFTCSVMHEALHNHYTQKSISRSPGK

SEQ ID NO: 171 - protein, 347 aa, synthetic construct
MAQLLFNKTKSVEFTFCNDTVVIPCFVTNMEAQNTTEVYVKWKFKGRDIYTFDGALNKSTVPTDFSSAKIEVSQLLKGDASLKMDKSDAVSHTGNYTCEVTELTREGETIIELKYRVVSWFSPNEPPCKCPAPELLGGPSVFIFPPKPKDTLMISRTPEVTCVVVDVSEDDPEVQFTWYINNEQVRTARPPLREQQFNSTIRVVSTLPIAHEDWLRGKEFKCKVHNKALPAPIEKTISKARQPLEPKVYTMGPPREELSSRSVSLTCMINGFYPSDISVEWEKNGKAEDNYKTTPAVLDSDGSYFLYSKLSVPTSEWQRGDVFTCSVMHEALHNHYTQKSISRSPGK

SEQ ID NO: 172 - protein, 489 aa, synthetic construct
MAVPRWRQQWSGPGTTKRFPETVLARCVKYTEIHPEMRHVDCQSVWDAFKGAFISKHPCNITEEDYQPLMKLGTQTVPCNKILLWSRIKDLAHQFTQVQRDMFTLEDTLLGYLADDLTWCGEFNTSKINYQSCPDWRKDCSNNPVSVFWKTVSRRFAEAACDVVHVMLNGSRSKIFDKNSTFGSVEVHNLQPEKVQTLEAWVIHGGREDSRDLCQDPTIKELESIISKRNIQFSCKNIYRPDKFLQCVKNPEDSSCTSEIAAASPSTCSKPTCPPELLGGPSVFIFPPKPKDTLMISRTPEVTCVVVDVSEDDPEVQFTWYINNEQVRTARPPLREQQFNSTIRVVSTLPIAHEDWLRGKEFKCKVHNKALPAPIEKTISKARQPLEPKVYTMGPPREELSSRSVSLTCMINGFYPSDISVEWEKNGKAEDNYKTTPAVLDSDGSYFLYSKLSVPTSEWQRGDVFTCSVMHEALHNHYTQKSISRSPGK

SEQ ID NO: 173 - protein, 489 aa, synthetic construct
MAVPRWRQQWSGPGTTKRFPETVLARCVKYTEIHPEMRHVDCQSVWDAFKGAFISKHPCNITEEDYQPLMKLGTQTVPCNKKLLWSRIKDLAHQFTQVQRDMFTLEDTLLGYLADDLTWCGEFNTSKINYQSCPDWRKDCSNNPVSVFWKTVSRRFAEAACDVVHVMLNGSRSKIFDKNSTFGSVEVHNLQPEKVQTLEAWVIHGGREDSRDLCQDPTIKELESIISKRNIQFSCKNIYRPDKFLQCVKNPEDSSCTSEIAAASPSTCSKPTCPPELLGGPSVFIFPPKPKDTLMISRTPEVTCVVVDVSEDDPEVQFTWYINNEQVRTARPPLREQQFNSTIRVVSTLPIAHEDWLRGKEFKCKVHNKALPAPIEKTISKARQPLEPKVYTMGPPREELSSRSVSLTCMINGFYPSDISVEWEKNGKAEDNYKTTPAVLDSDGSYFLYSKLSVPTSEWQRGDVFTCSVMHEALHNHYTQKSISRSPGK

SEQ ID NO: 174 - protein, 354 aa, synthetic construct
MAQLLFNKTKSVEFTFCNDTVVIPCFVTNMEAQNTTEVYVKWKFKGRDIYTFDGALNKSTVPTDFSSAKIEVSQLLKGDASLKMDKSDAVSHTGNYTCEVTELTREGETIIELKYRVVSWFSPNEAAASPSTCSKPTCPPELLGGPSVFIFPPKPKDTLMISRTPEVTCVVVDVSEDDPEVQFTWYINNEQVRTARPPLREQQFNSTIRVVSTLPIAHEDWLRGKEFKCKVHNKALPAPIEKTISKARQPLEPKVYTMGPPREELSSRSVSLTCMINGFYPSDISVEWEKNGKAEDNYKTTPAVLDSDGSYFLYSKLSVPTSEWQRGDVFTCSVMHEALHNHYTQKSISRSPGK

SEQ ID NO: 175 - protein, 489 aa, synthetic construct
MAVPRWRQQWSGPGTTKRFPETVLARCVKYTEIHPEMRHVDCQSVWDAFKGAFISKHPCNITEEDYQPLMKLGTQTVPCNKILLWSRIKDLAHQFTQVQRDMFTLEDTLLGYLADDLTWCGEFNTSKINYQSCPDWRKDCSNNPVSVFWKTVSRRFAEAACDVVHVMLNGSRSKIFDKNSTFGSVEVHNLQPEKVQTLEAWVIHGGREDSRDLCQDPTIKELESIISKRNIQFSCKNIYRPDKFLQCVKNPEDSSCTSEIGGGSPSTCSKPTCPPELLGGPSVFIFPPKPKDTLMISRTPEVTCVVVDVSEDDPEVQFTWYINNEQVRTARPPLREQQFNSTIRVVSTLPIAHEDWLRGKEFKCKVHNKALPAPIEKTISKARQPLEPKVYTMGPPREELSSRSVSLTCMINGFYPSDISVEWEKNGKAEDNYKTTPAVLDSDGSYFLYSKLSVPTSEWQRGDVFTCSVMHEALHNHYTQKSISRSPGK

SEQ ID NO: 176 - protein, 489 aa, synthetic construct
MAVPRWRQQWSGPGTTKRFPETVLARCVKYTEIHPEMRHVDCQSVWDAFKGAFISKHPCNITEEDYQPLMKLGTQTVPCNKKLLWSRIKDLAHQFTQVQRDMFTLEDTLLGYLADDLTWCGEFNTSKINYQSCPDWRKDCSNNPVSVFWKTVSRRFAEAACDVVHVMLNGSRSKIFDKNSTFGSVEVHNLQPEKVQTLEAWVIHGGREDSRDLCQDPTIKELESIISKRNIQFSCKNIYRPDKFLQCVKNPEDSSCTSEIGGGSPSTCSKPTCPPELLGGPSVFIFPPKPKDTLMISRTPEVTCVVVDVSEDDPEVQFTWYINNEQVRTARPPLREQQFNSTIRVVSTLPIAHEDWLRGKEFKCKVHNKALPAPIEKTISKARQPLEPKVYTMGPPREELSSRSVSLTCMINGFYPSDISVEWEKNGKAEDNYKTTPAVLDSDGSYFLYSKLSVPTSEWQRGDVFTCSVMHEALHNHYTQKSISRSPGK

SEQ ID NO: 177 - protein, 354 aa, synthetic construct
MAQLLFNKTKSVEFTFCNDTVVIPCFVTNMEAQNTTEVYVKWKFKGRDIYTFDGALNKSTVPTDFSSAKIEVSQLLKGDASLKMDKSDAVSHTGNYTCEVTELTREGETIIELKYRVVSWFSPNEGGGSPSTCSKPTCPPELLGGPSVFIFPPKPKDTLMISRTPEVTCVVVDVSEDDPEVQFTWYINNEQVRTARPPLREQQFNSTIRVVSTLPIAHEDWLRGKEFKCKVHNKALPAPIEKTISKARQPLEPKVYTMGPPREELSSRSVSLTCMINGFYPSDISVEWEKNGKAEDNYKTTPAVLDSDGSYFLYSKLSVPTSEWQRGDVFTCSVMHEALHNHYTQKSISRSPGK

SEQ ID NO: 178 - protein, 485 aa, synthetic construct
MAVPRWRQQWSGPGTTKRFPETVLARCVKYTEIHPEMRHVDCQSVWDAFKGAFISKHPCNITEEDYQPLMKLGTQTVPCNKILLWSRIKDLAHQFTQVQRDMFTLEDTLLGYLADDLTWCGEFNTSKINYQSCPDWRKDCSNNPVSVFWKTVSRRFAEAACDVVHVMLNGSRSKIFDKNSTFGSVEVHNLQPEKVQTLEAWVIHGGREDSRDLCQDPTIKELESIISKRNIQFSCKNIYRPDKFLQCVKNPEDSSCTSEIPSTCSKPTCPPELLGGPSVFIFPPKPKDTLMISRTPEVTCVVVDVSEDDPEVQFTWYINNEQVRTARPPLREQQFNSTIRVVSTLPIAHEDWLRGKEFKCKVHNKALPAPIEKTISKARQPLEPKVYTMGPPREELSSRSVSLTCMINGFYPSDISVEWEKNGKAEDNYKTTPAVLDSDGSYFLYSKLSVPTSEWQRGDVFTCSVMHEALHNHYTQKSISRSPGK

SEQ ID NO: 179 - protein, 485 aa, synthetic construct
MAVPRWRQQWSGPGTTKRFPETVLARCVKYTEIHPEMRHVDCQSVWDAFKGAFISKHPCNITEEDYQPLMKLGTQTVPCNKKLLWSRIKDLAHQFTQVQRDMFTLEDTLLGYLADDLTWCGEFNTSKINYQSCPDWRKDCSNNPVSVFWKTVSRRFAEAACDVVHVMLNGSRSKIFDKNSTFGSVEVHNLQPEKVQTLEAWVIHGGREDSRDLCQDPTIKELESIISKRNIQFSCKNIYRPDKFLQCVKNPEDSSCTSEIPSTCSKPTCPPELLGGPSVFIFPPKPKDTLMISRTPEVTCVVVDVSEDDPEVQFTWYINNEQVRTARPPLREQQFNSTIRVVSTLPIAHEDWLRGKEFKCKVHNKALPAPIEKTISKARQPLEPKVYTMGPPREELSSRSVSLTCMINGFYPSDISVEWEKNGKAEDNYKTTPAVLDSDGSYFLYSKLSVPTSEWQRGDVFTCSVMHEALHNHYTQKSISRSPGK

SEQ ID NO: 180 - protein, 350 aa, synthetic construct
MAQLLFNKTKSVEFTFCNDTVVIPCFVTNMEAQNTTEVYVKWKFKGRDIYTFDGALNKSTVPTDFSSAKIEVSQLLKGDASLKMDKSDAVSHTGNYTCEVTELTREGETIIELKYRVVSWFSPNEPSTCSKPTCPPELLGGPSVFIFPPKPKDTLMISRTPEVTCVVVDVSEDDPEVQFTWYINNEQVRTARPPLREQQFNSTIRVVSTLPIAHEDWLRGKEFKCKVHNKALPAPIEKTISKARQPLEPKVYTMGPPREELSSRSVSLTCMINGFYPSDISVEWEKNGKAEDNYKTTPAVLDSDGSYFLYSKLSVPTSEWQRGDVFTCSVMHEALHNHYTQKSISRSPGK

SEQ ID NO: 181 - protein, 485 aa, synthetic construct
MAVPRWRQQWSGPGTTKRFPETVLARCVKYTEIHPEMRHVDCQSVWDAFKGAFISKHPCNITEEDYQPLMKLGTQTVPCNKILLWSRIKDLAHQFTQVQRDMFTLEDTLLGYLADDLTWCGEFNTSKINYQSCPDWRKDCSNNPVSVFWKTVSRRFAEAACDVVHVMLNGSRSKIFDKNSTFGSVEVHNLQPEKVQTLEAWVIHGGREDSRDLCQDPTIKELESIISKRNIQFSCKNIYRPDKFLQCVKNPEDSSCTSEIAAASNPCGCTPELLGGPSVFIFPPKPKDTLMISRTPEVTCVVVDVSEDDPEVQFTWYINNEQVRTARPPLREQQFNSTIRVVSTLPIAHEDWLRGKEFKCKVHNKALPAPIEKTISKARQPLEPKVYTMGPPREELSSRSVSLTCMINGFYPSDISVEWEKNGKAEDNYKTTPAVLDSDGSYFLYSKLSVPTSEWQRGDVFTCSVMHEALHNHYTQKSISRSPGK

SEQ ID NO: 182 - protein, 485 aa, synthetic construct
MAVPRWRQQWSGPGTTKRFPETVLARCVKYTEIHPEMRHVDCQSVWDAFKGAFISKHPCNITEEDYQPLMKLGTQTVPCNKKLLWSRIKDLAHQFTQVQRDMFTLEDTLLGYLADDLTWCGEFNTSKINYQSCPDWRKDCSNNPVSVFWKTVSRRFAEAACDVVHVMLNGSRSKIFDKNSTFGSVEVHNLQPEKVQTLEAWVIHGGREDSRDLCQDPTIKELESIISKRNIQFSCKNIYRPDKFLQCVKNPEDSSCTSEIAAASNPCGCTPELLGGPSVFIFPPKPKDTLMISRTPEVTCVVVDVSEDDPEVQFTWYINNEQVRTARPPLREQQFNSTIRVVSTLPIAHEDWLRGKEFKCKVHNKALPAPIEKTISKARQPLEPKVYTMGPPREELSSRSVSLTCMINGFYPSDISVEWEKNGKAEDNYKTTPAVLDSDGSYFLYSKLSVPTSEWQRGDVFTCSVMHEALHNHYTQKSISRSPGK

SEQ ID NO: 183 - protein, 350 aa, synthetic construct
MAQLLFNKTKSVEFTFCNDTVVIPCFVTNMEAQNTTEVYVKWKFKGRDIYTFDGALNKSTVPTDFSSAKIEVSQLLKGDASLKMDKSDAVSHTGNYTCEVTELTREGETIIELKYRVVSWFSPNEAAASNPCGCTPELLGGPSVFIFPPKPKDTLMISRTPEVTCVVVDVSEDDPEVQFTWYINNEQVRTARPPLREQQFNSTIRVVSTLPIAHEDWLRGKEFKCKVHNKALPAPIEKTISKARQPLEPKVYTMGPPREELSSRSVSLTCMINGFYPSDISVEWEKNGKAEDNYKTTPAVLDSDGSYFLYSKLSVPTSEWQRGDVFTCSVMHEALHNHYTQKSISRSPGK

SEQ ID NO: 184 - protein, 485 aa, synthetic construct
MAVPRWRQQWSGPGTTKRFPETVLARCVKYTEIHPEMRHVDCQSVWDAFKGAFISKHPCNITEEDYQPLMKLGTQTVPCNKILLWSRIKDLAHQFTQVQRDMFTLEDTLLGYLADDLTWCGEFNTSKINYQSCPDWRKDCSNNPVSVFWKTVSRRFAEAACDVVHVMLNGSRSKIFDKNSTFGSVEVHNLQPEKVQTLEAWVIHGGREDSRDLCQDPTIKELESIISKRNIQFSCKNIYRPDKFLQCVKNPEDSSCTSEIGGGSNPCGCTPELLGGPSVFIFPPKPKDTLMISRTPEVTCVVVDVSEDDPEVQFTWYINNEQVRTARPPLREQQFNSTIRVVSTLPIAHEDWLRGKEFKCKVHNKALPAPIEKTISKARQPLEPKVYTMGPPREELSSRSVSLTCMINGFYPSDISVEWEKNGKAEDNYKTTPAVLDSDGSYFLYSKLSVPTSEWQRGDVFTCSVMHEALHNHYTQKSISRSPGK

SEQ ID NO: 185 - protein, 485 aa, synthetic construct
MAVPRWRQQWSGPGTTKRFPETVLARCVKYTEIHPEMRHVDCQSVWDAFKGAFISKHPCNITEEDYQPLMKLGTQTVPCNKKLLWSRIKDLAHQFTQVQRDMFTLEDTLLGYLADDLTWCGEFNTSKINYQSCPDWRKDCSNNPVSVFWKTVSRRFAEAACDVVHVMLNGSRSKIFDKNSTFGSVEVHNLQPEKVQTLEAWVIHGGREDSRDLCQDPTIKELESIISKRNIQFSCKNIYRPDKFLQCVKNPEDSSCTSEIGGGSNPCGCTPELLGGPSVFIFPPKPKDTLMISRTPEVTCVVVDVSEDDPEVQFTWYINNEQVRTARPPLREQQFNSTIRVVSTLPIAHEDWLRGKEFKCKVHNKALPAPIEKTISKARQPLEPKVYTMGPPREELSSRSVSLTCMINGFYPSDISVEWEKNGKAEDNYKTTPAVLDSDGSYFLYSKLSVPTSEWQRGDVFTCSVMHEALHNHYTQKSISRSPGK

SEQ ID NO: 186 - protein, 350 aa, synthetic construct
MAQLLFNKTKSVEFTFCNDTVVIPCFVTNMEAQNTTEVYVKWKFKGRDIYTFDGALNKSTVPTDFSSAKIEVSQLLKGDASLKMDKSDAVSHTGNYTCEVTELTREGETIIELKYRVVSWFSPNEGGGSNPCGCTPELLGGPSVFIFPPKPKDTLMISRTPEVTCVVVDVSEDDPEVQFTWYINNEQVRTARPPLREQQFNSTIRVVSTLPIAHEDWLRGKEFKCKVHNKALPAPIEKTISKARQPLEPKVYTMGPPREELSSRSVSLTCMINGFYPSDISVEWEKNGKAEDNYKTTPAVLDSDGSYFLYSKLSVPTSEWQRGDVFTCSVMHEALHNHYTQKSISRSPGK

SEQ ID NO: 187 - protein, 481 aa, synthetic construct
MAVPRWRQQWSGPGTTKRFPETVLARCVKYTEIHPEMRHVDCQSVWDAFKGAFISKHPCNITEEDYQPLMKLGTQTVPCNKILLWSRIKDLAHQFTQVQRDMFTLEDTLLGYLADDLTWCGEFNTSKINYQSCPDWRKDCSNNPVSVFWKTVSRRFAEAACDVVHVMLNGSRSKIFDKNSTFGSVEVHNLQPEKVQTLEAWVIHGGREDSRDLCQDPTIKELESIISKRNIQFSCKNIYRPDKFLQCVKNPEDSSCTSEINPCGCTPELLGGPSVFIFPPKPKDTLMISRTPEVTCVVVDVSEDDPEVQFTWYINNEQVRTARPPLREQQFNSTIRVVSTLPIAHEDWLRGKEFKCKVHNKALPAPIEKTISKARQPLEPKVYTMGPPREELSSRSVSLTCMINGFYPSDISVEWEKNGKAEDNYKTTPAVLDSDGSYFLYSKLSVPTSEWQRGDVFTCSVMHEALHNHYTQKSISRSPGK

SEQ ID NO: 188 - protein, 481 aa, synthetic construct
MAVPRWRQQWSGPGTTKRFPETVLARCVKYTEIHPEMRHVDCQSVWDAFKGAFISKHPCNITEEDYQPLMKLGTQTVPCNKKLLWSRIKDLAHQFTQVQRDMFTLEDTLLGYLADDLTWCGEFNTSKINYQSCPDWRKDCSNNPVSVFWKTVSRRFAEAACDVVHVMLNGSRSKIFDKNSTFGSVEVHNLQPEKVQTLEAWVIHGGREDSRDLCQDPTIKELESIISKRNIQFSCKNIYRPDKFLQCVKNPEDSSCTSEINPCGCTPELLGGPSVFIFPPKPKDTLMISRTPEVTCVVVDVSEDDPEVQFTWYINNEQVRTARPPLREQQFNSTIRVVSTLPIAHEDWLRGKEFKCKVHNKALPAPIEKTISKARQPLEPKVYTMGPPREELSSRSVSLTCMINGFYPSDISVEWEKNGKAEDNYKTTPAVLDSDGSYFLYSKLSVPTSEWQRGDVFTCSVMHEALHNHYTQKSISRSPGK

SEQ ID NO: 189 - protein, 346 aa, synthetic construct
MAQLLFNKTKSVEFTFCNDTVVIPCFVTNMEAQNTTEVYVKWKFKGRDIYTFDGALNKSTVPTDFSSAKIEVSQLLKGDASLKMDKSDAVSHTGNYTCEVTELTREGETIIELKYRVVSWFSPNENPCGCTPELLGGPSVFIFPPKPKDTLMISRTPEVTCVVVDVSEDDPEVQFTWYINNEQVRTARPPLREQQFNSTIRVVSTLPIAHEDWLRGKEFKCKVHNKALPAPIEKTISKARQPLEPKVYTMGPPREELSSRSVSLTCMINGFYPSDISVEWEKNGKAEDNYKTTPAVLDSDGSYFLYSKLSVPTSEWQRGDVFTCSVMHEALHNHYTQKSISRSPGK

SEQ ID NO: 190 - protein, 489 aa, synthetic construct
MAVPRWRQQWSGPGTTKRFPETVLARCVKYTEIHPEMRHVDCQSVWDAFKGAFISKHPCNITEEDYQPLMKLGTQTVPCNKILLWSRIKDLAHQFTQVQRDMFTLEDTLLGYLADDLTWCGEFNTSKINYQSCPDWRKDCSNNPVSVFWKTVSRRFAEAACDVVHVMLNGSRSKIFDKNSTFGSVEVHNLQPEKVQTLEAWVIHGGREDSRDLCQDPTIKELESIISKRNIQFSCKNIYRPDKFLQCVKNPEDSSCTSEIAAASDKTHTCPPCPPELLGGPSVFIFPPKPKDTLMISRTPEVTCVVVDVSEDDPEVQFTWYINNEQVRTARPPLREQQFNSTIRVVSTLPIAHEDWLRGKEFKCKVHNKALPAPIEKTISKARQPLEPKVYTMGPPREELSSRSVSLTCMINGFYPSDISVEWEKNGKAEDNYKTTPAVLDSDGSYFLYSKLSVPTSEWQRGDVFTCSVMHEALHNHYTQKSISRSPGK

SEQ ID NO: 191 - protein, 489 aa, synthetic construct
MAVPRWRQQWSGPGTTKRFPETVLARCVKYTEIHPEMRHVDCQSVWDAFKGAFISKHPCNITEEDYQPLMKLGTQTVPCNKKLLWSRIKDLAHQFTQVQRDMFTLEDTLLGYLADDLTWCGEFNTSKINYQSCPDWRKDCSNNPVSVFWKTVSRRFAEAACDVVHVMLNGSRSKIFDKNSTFGSVEVHNLQPEKVQTLEAWVIHGGREDSRDLCQDPTIKELESIISKRNIQFSCKNIYRPDKFLQCVKNPEDSSCTSEIAAASDKTHTCPPCPPELLGGPSVFIFPPKPKDTLMISRTPEVTCVVVDVSEDDPEVQFTWYINNEQVRTARPPLREQQFNSTIRVVSTLPIAHEDWLRGKEFKCKVHNKALPAPIEKTISKARQPLEPKVYTMGPPREELSSRSVSLTCMINGFYPSDISVEWEKNGKAEDNYKTTPAVLDSDGSYFLYSKLSVPTSEWQRGDVFTCSVMHEALHNHYTQKSISRSPGK

SEQ ID NO: 192 - protein, 354 aa, synthetic construct
MAQLLFNKTKSVEFTFCNDTVVIPCFVTNMEAQNTTEVYVKWKFKGRDIYTFDGALNKSTVPTDFSSAKIEVSQLLKGDASLKMDKSDAVSHTGNYTCEVTELTREGETIIELKYRVVSWFSPNEAAASDKTHTCPPCPPELLGGPSVFIFPPKPKDTLMISRTPEVTCVVVDVSEDDPEVQFTWYINNEQVRTARPPLREQQFNSTIRVVSTLPIAHEDWLRGKEFKCKVHNKALPAPIEKTISKARQPLEPKVYTMGPPREELSSRSVSLTCMINGFYPSDISVEWEKNGKAEDNYKTTPAVLDSDGSYFLYSKLSVPTSEWQRGDVFTCSVMHEALHNHYTQKSISRSPGK

SEQ ID NO: 193 - protein, 489 aa, synthetic construct
MAVPRWRQQWSGPGTTKRFPETVLARCVKYTEIHPEMRHVDCQSVWDAFKGAFISKHPCNITEEDYQPLMKLGTQTVPCNKILLWSRIKDLAHQFTQVQRDMFTLEDTLLGYLADDLTWCGEFNTSKINYQSCPDWRKDCSNNPVSVFWKTVSRRFAEAACDVVHVMLNGSRSKIFDKNSTFGSVEVHNLQPEKVQTLEAWVIHGGREDSRDLCQDPTIKELESIISKRNIQFSCKNIYRPDKFLQCVKNPEDSSCTSEIGGGSDKTHTCPPCPPELLGGPSVFIFPPKPKDTLMISRTPEVTCVVVDVSEDDPEVQFTWYINNEQVRTARPPLREQQFNSTIRVVSTLPIAHEDWLRGKEFKCKVHNKALPAPIEKTISKARQPLEPKVYTMGPPREELSSRSVSLTCMINGFYPSDISVEWEKNGKAEDNYKTTPAVLDSDGSYFLYSKLSVPTSEWQRGDVFTCSVMHEALHNHYTQKSISRSPGK

SEQ ID NO: 194 - protein, 489 aa, synthetic construct
MAVPRWRQQWSGPGTTKRFPETVLARCVKYTEIHPEMRHVDCQSVWDAFKGAFISKHPCNITEEDYQPLMKLGTQTVPCNKKLLWSRIKDLAHQFTQVQRDMFTLEDTLLGYLADDLTWCGEFNTSKINYQSCPDWRKDCSNNPVSVFWKTVSRRFAEAACDVVHVMLNGSRSKIFDKNSTFGSVEVHNLQPEKVQTLEAWVIHGGREDSRDLCQDPTIKELESIISKRNIQFSCKNIYRPDKFLQCVKNPEDSSCTSEIGGGSDKTHTCPPCPPELLGGPSVFIFPPKPKDTLMISRTPEVTCVVVDVSEDDPEVQFTWYINNEQVRTARPPLREQQFNSTIRVVSTLPIAHEDWLRGKEFKCKVHNKALPAPIEKTISKARQPLEPKVYTMGPPREELSSRSVSLTCMINGFYPSDISVEWEKNGKAEDNYKTTPAVLDSDGSYFLYSKLSVPTSEWQRGDVFTCSVMHEALHNHYTQKSISRSPGK

SEQ ID NO: 195 - protein, 354 aa, synthetic construct
MAQLLFNKTKSVEFTFCNDTVVIPCFVTNMEAQNTTEVYVKWKFKGRDIYTFDGALNKSTVPTDFSSAKIEVSQLLKGDASLKMDKSDAVSHTGNYTCEVTELTREGETIIELKYRVVSWFSPNEGGGSDKTHTCPPCPPELLGGPSVFIFPPKPKDTLMISRTPEVTCVVVDVSEDDPEVQFTWYINNEQVRTARPPLREQQFNSTIRVVSTLPIAHEDWLRGKEFKCKVHNKALPAPIEKTISKARQPLEPKVYTMGPPREELSSRSVSLTCMINGFYPSDISVEWEKNGKAEDNYKTTPAVLDSDGSYFLYSKLSVPTSEWQRGDVFTCSVMHEALHNHYTQKSISRSPGK

SEQ ID NO: 196 - protein, 485 aa, synthetic construct
MAVPRWRQQWSGPGTTKRFPETVLARCVKYTEIHPEMRHVDCQSVWDAFKGAFISKHPCNITEEDYQPLMKLGTQTVPCNKILLWSRIKDLAHQFTQVQRDMFTLEDTLLGYLADDLTWCGEFNTSKINYQSCPDWRKDCSNNPVSVFWKTVSRRFAEAACDVVHVMLNGSRSKIFDKNSTFGSVEVHNLQPEKVQTLEAWVIHGGREDSRDLCQDPTIKELESIISKRNIQFSCKNIYRPDKFLQCVKNPEDSSCTSEIDKTHTCPPCPPELLGGPSVFIFPPKPKDTLMISRTPEVTCVVVDVSEDDPEVQFTWYINNEQVRTARPPLREQQFNSTIRVVSTLPIAHEDWLRGKEFKCKVHNKALPAPIEKTISKARQPLEPKVYTMGPPREELSSRSVSLTCMINGFYPSDISVEWEKNGKAEDNYKTTPAVLDSDGSYFLYSKLSVPTSEWQRGDVFTCSVMHEALHNHYTQKSISRSPGK

SEQ ID NO: 197 - protein, 485 aa, synthetic construct
MAVPRWRQQWSGPGTTKRFPETVLARCVKYTEIHPEMRHVDCQSVWDAFKGAFISKHPCNITEEDYQPLMKLGTQTVPCNKKLLWSRIKDLAHQFTQVQRDMFTLEDTLLGYLADDLTWCGEFNTSKINYQSCPDWRKDCSNNPVSVFWKTVSRRFAEAACDVVHVMLNGSRSKIFDKNSTFGSVEVHNLQPEKVQTLEAWVIHGGREDSRDLCQDPTIKELESIISKRNIQFSCKNIYRPDKFLQCVKNPEDSSCTSEIDKTHTCPPCPPELLGGPSVFIFPPKPKDTLMISRTPEVTCVVVDVSEDDPEVQFTWYINNEQVRTARPPLREQQFNSTIRVVSTLPIAHEDWLRGKEFKCKVHNKALPAPIEKTISKARQPLEPKVYTMGPPREELSSRSVSLTCMINGFYPSDISVEWEKNGKAEDNYKTTPAVLDSDGSYFLYSKLSVPTSEWQRGDVFTCSVMHEALHNHYTQKSISRSPGK

SEQ ID NO: 198 - protein, 350 aa, synthetic construct
MAQLLFNKTKSVEFTFCNDTVVIPCFVTNMEAQNTTEVYVKWKFKGRDIYTFDGALNKSTVPTDFSSAKIEVSQLLKGDASLKMDKSDAVSHTGNYTCEVTELTREGETIIELKYRVVSWFSPNEDKTHTCPPCPPELLGGPSVFIFPPKPKDTLMISRTPEVTCVVVDVSEDDPEVQFTWYINNEQVRTARPPLREQQFNSTIRVVSTLPIAHEDWLRGKEFKCKVHNKALPAPIEKTISKARQPLEPKVYTMGPPREELSSRSVSLTCMINGFYPSDISVEWEKNGKAEDNYKTTPAVLDSDGSYFLYSKLSVPTSEWQRGDVFTCSVMHEALHNHYTQKSISRSPGK

SEQ ID NO: 199 - protein, 483 aa, synthetic construct
MAVPRWRQQWSGPGTTKRFPETVLARCVKYTEIHPEMRHVDCQSVWDAFKGAFISKHPCNITEEDYQPLMKLGTQTVPCNKILLWSRIKDLAHQFTQVQRDMFTLEDTLLGYLADDLTWCGEFNTSKINYQSCPDWRKDCSNNPVSVFWKTVSRRFAEAACDVVHVMLNGSRSKIFDKNSTFGSVEVHNLQPEKVQTLEAWVIHGGREDSRDLCQDPTIKELESIISKRNIQFSCKNIYRPDKFLQCVKNPEDSSCTSEIAAASPPCKCPASEVSSVFIFPPKPKDVLTITLTPKVTCVVVDISQDDPEVHFSWFVDDVEVHTAQTRPPEEQFNSTFRSVSELPILHQDWLNGRTFRCKVTSAAFPSPIEKTISKPERTQVPHVYTMSPTKEEMTQNEVSITCMVKGFYPPDIYVEWQMNGQPQENYKNTPPTMDTDGSYFLYSKLNVKKEKWQQGNTFTCSVLHEGLHNHHTEKSLSHSPGK

SEQ ID NO: 200 - protein, 483 aa, synthetic construct
MAVPRWRQQWSGPGTTKRFPETVLARCVKYTEIHPEMRHVDCQSVWDAFKGAFISKHPCNITEEDYQPLMKLGTQTVPCNKKLLWSRIKDLAHQFTQVQRDMFTLEDTLLGYLADDLTWCGEFNTSKINYQSCPDWRKDCSNNPVSVFWKTVSRRFAEAACDVVHVMLNGSRSKIFDKNSTFGSVEVHNLQPEKVQTLEAWVIHGGREDSRDLCQDPTIKELESIISKRNIQFSCKNIYRPDKFLQCVKNPEDSSCTSEIAAASPPCKCPASEVSSVFIFPPKPKDVLTITLTPKVTCVVVDISQDDPEVHFSWFVDDVEVHTAQTRPPEEQFNSTFRSVSELPILHQDWLNGRTFRCKVTSAAFPSPIEKTISKPERTQVPHVYTMSPTKEEMTQNEVSITCMVKGFYPPDIYVEWQMNGQPQENYKNTPPTMDTDGSYFLYSKLNVKKEKWQQGNTFTCSVLHEGLHNHHTEKSLSHSPGK

SEQ ID NO: 201 - protein, 348 aa, synthetic construct
MAQLLFNKTKSVEFTFCNDTVVIPCFVTNMEAQNTTEVYVKWKFKGRDIYTFDGALNKSTVPTDFSSAKIEVSQLLKGDASLKMDKSDAVSHTGNYTCEVTELTREGETIIELKYRVVSWFSPNEAAASPPCKCPASEVSSVFIFPPKPKDVLTITLTPKVTCVVVDISQDDPEVHFSWFVDDVEVHTAQTRPPEEQFNSTFRSVSELPILHQDWLNGRTFRCKVTSAAFPSPIEKTISKPERTQVPHVYTMSPTKEEMTQNEVSITCMVKGFYPPDIYVEWQMNGQPQENYKNTPPTMDTDGSYFLYSKLNVKKEKWQQGNTFTCSVLHEGLHNHHTEKSLSHSPGK

SEQ ID NO: 202 - protein, 483 aa, synthetic construct
MAVPRWRQQWSGPGTTKRFPETVLARCVKYTEIHPEMRHVDCQSVWDAFKGAFISKHPCNITEEDYQPLMKLGTQTVPCNKILLWSRIKDLAHQFTQVQRDMFTLEDTLLGYLADDLTWCGEFNTSKINYQSCPDWRKDCSNNPVSVFWKTVSRRFAEAACDVVHVMLNGSRSKIFDKNSTFGSVEVHNLQPEKVQTLEAWVIHGGREDSRDLCQDPTIKELESIISKRNIQFSCKNIYRPDKFLQCVKNPEDSSCTSEIGGGSPPCKCPASEVSSVFIFPPKPKDVLTITLTPKVTCVVVDISQDDPEVHFSWFVDDVEVHTAQTRPPEEQFNSTFRSVSELPILHQDWLNGRTFRCKVTSAAFPSPIEKTISKPERTQVPHVYTMSPTKEEMTQNEVSITCMVKGFYPPDIYVEWQMNGQPQENYKNTPPTMDTDGSYFLYSKLNVKKEKWQQGNTFTCSVLHEGLHNHHTEKSLSHSPGK

SEQ ID NO: 203 - protein, 483 aa, synthetic construct
MAVPRWRQQWSGPGTTKRFPETVLARCVKYTEIHPEMRHVDCQSVWDAFKGAFISKHPCNITEEDYQPLMKLGTQTVPCNKKLLWSRIKDLAHQFTQVQRDMFTLEDTLLGYLADDLTWCGEFNTSKINYQSCPDWRKDCSNNPVSVFWKTVSRRFAEAACDVVHVMLNGSRSKIFDKNSTFGSVEVHNLQPEKVQTLEAWVIHGGREDSRDLCQDPTIKELESIISKRNIQFSCKNIYRPDKFLQCVKNPEDSSCTSEIGGGSPPCKCPASEVSSVFIFPPKPKDVLTITLTPKVTCVVVDISQDDPEVHFSWFVDDVEVHTAQTRPPEEQFNSTFRSVSELPILHQDWLNGRTFRCKVTSAAFPSPIEKTISKPERTQVPHVYTMSPTKEEMTQNEVSITCMVKGFYPPDIYVEWQMNGQPQENYKNTPPTMDTDGSYFLYSKLNVKKEKWQQGNTFTCSVLHEGLHNHHTEKSLSHSPGK

SEQ ID NO: 204 - protein, 348 aa, synthetic construct
MAQLLFNKTKSVEFTFCNDTVVIPCFVTNMEAQNTTEVYVKWKFKGRDIYTFDGALNKSTVPTDFSSAKIEVSQLLKGDASLKMDKSDAVSHTGNYTCEVTELTREGETIIELKYRVVSWFSPNEGGGSPPCKCPASEVSSVFIFPPKPKDVLTITLTPKVTCVVVDISQDDPEVHFSWFVDDVEVHTAQTRPPEEQFNSTFRSVSELPILHQDWLNGRTFRCKVTSAAFPSPIEKTISKPERTQVPHVYTMSPTKEEMTQNEVSITCMVKGFYPPDIYVEWQMNGQPQENYKNTPPTMDTDGSYFLYSKLNVKKEKWQQGNTFTCSVLHEGLHNHHTEKSLSHSPGK

SEQ ID NO: 205 - protein, 479 aa, synthetic construct
MAVPRWRQQWSGPGTTKRFPETVLARCVKYTEIHPEMRHVDCQSVWDAFKGAFISKHPCNITEEDYQPLMKLGTQTVPCNKILLWSRIKDLAHQFTQVQRDMFTLEDTLLGYLADDLTWCGEFNTSKINYQSCPDWRKDCSNNPVSVFWKTVSRRFAEAACDVVHVMLNGSRSKIFDKNSTFGSVEVHNLQPEKVQTLEAWVIHGGREDSRDLCQDPTIKELESIISKRNIQFSCKNIYRPDKFLQCVKNPEDSSCTSEIPPCKCPASEVSSVFIFPPKPKDVLTITLTPKVTCVVVDISQDDPEVHFSWFVDDVEVHTAQTRPPEEQFNSTFRSVSELPILHQDWLNGRTFRCKVTSAAFPSPIEKTISKPERTQVPHVYTMSPTKEEMTQNEVSITCMVKGFYPPDIYVEWQMNGQPQENYKNTPPTMDTDGSYFLYSKLNVKKEKWQQGNTFTCSVLHEGLHNHHTEKSLSHSPGK

SEQ ID NO: 206 - protein, 479 aa, synthetic construct
MAVPRWRQQWSGPGTTKRFPETVLARCVKYTEIHPEMRHVDCQSVWDAFKGAFISKHPCNITEEDYQPLMKLGTQTVPCNKKLLWSRIKDLAHQFTQVQRDMFTLEDTLLGYLADDLTWCGEFNTSKINYQSCPDWRKDCSNNPVSVFWKTVSRRFAEAACDVVHVMLNGSRSKIFDKNSTFGSVEVHNLQPEKVQTLEAWVIHGGREDSRDLCQDPTIKELESIISKRNIQFSCKNIYRPDKFLQCVKNPEDSSCTSEIPPCKCPASEVSSVFIFPPKPKDVLTITLTPKVTCVVVDISQDDPEVHFSWFVDDVEVHTAQTRPPEEQFNSTFRSVSELPILHQDWLNGRTFRCKVTSAAFPSPIEKTISKPERTQVPHVYTMSPTKEEMTQNEVSITCMVKGFYPPDIYVEWQMNGQPQENYKNTPPTMDTDGSYFLYSKLNVKKEKWQQGNTFTCSVLHEGLHNHHTEKSLSHSPGK

SEQ ID NO: 207 - protein, 344 aa, synthetic construct
MAQLLFNKTKSVEFTFCNDTVVIPCFVTNMEAQNTTEVYVKWKFKGRDIYTFDGALNKSTVPTDFSSAKIEVSQLLKGDASLKMDKSDAVSHTGNYTCEVTELTREGETIIELKYRVVSWFSPNEPPCKCPASEVSSVFIFPPKPKDVLTITLTPKVTCVVVDISQDDPEVHFSWFVDDVEVHTAQTRPPEEQFNSTFRSVSELPILHQDWLNGRTFRCKVTSAAFPSPIEKTISKPERTQVPHVYTMSPTKEEMTQNEVSITCMVKGFYPPDIYVEWQMNGQPQENYKNTPPTMDTDGSYFLYSKLNVKKEKWQQGNTFTCSVLHEGLHNHHTEKSLSHSPGK

SEQ ID NO: 208 - protein, 486 aa, synthetic construct
MAVPRWRQQWSGPGTTKRFPETVLARCVKYTEIHPEMRHVDCQSVWDAFKGAFISKHPCNITEEDYQPLMKLGTQTVPCNKILLWSRIKDLAHQFTQVQRDMFTLEDTLLGYLADDLTWCGEFNTSKINYQSCPDWRKDCSNNPVSVFWKTVSRRFAEAACDVVHVMLNGSRSKIFDKNSTFGSVEVHNLQPEKVQTLEAWVIHGGREDSRDLCQDPTIKELESIISKRNIQFSCKNIYRPDKFLQCVKNPEDSSCTSEIAAASPSTCSKPTCPSEVSSVFIFPPKPKDVLTITLTPKVTCVVVDISQDDPEVHFSWFVDDVEVHTAQTRPPEEQFNSTFRSVSELPILHQDWLNGRTFRCKVTSAAFPSPIEKTISKPERTQVPHVYTMSPTKEEMTQNEVSITCMVKGFYPPDIYVEWQMNGQPQENYKNTPPTMDTDGSYFLYSKLNVKKEKWQQGNTFTCSVLHEGLHNHHTEKSLSHSPGK

SEQ ID NO: 209 - protein, 486 aa, synthetic construct
MAVPRWRQQWSGPGTTKRFPETVLARCVKYTEIHPEMRHVDCQSVWDAFKGAFISKHPCNITEEDYQPLMKLGTQTVPCNKKLLWSRIKDLAHQFTQVQRDMFTLEDTLLGYLADDLTWCGEFNTSKINYQSCPDWRKDCSNNPVSVFWKTVSRRFAEAACDVVHVMLNGSRSKIFDKNSTFGSVEVHNLQPEKVQTLEAWVIHGGREDSRDLCQDPTIKELESIISKRNIQFSCKNIYRPDKFLQCVKNPEDSSCTSEIAAASPSTCSKPTCPSEVSSVFIFPPKPKDVLTITLTPKVTCVVVDISQDDPEVHFSWFVDDVEVHTAQTRPPEEQFNSTFRSVSELPILHQDWLNGRTFRCKVTSAAFPSPIEKTISKPERTQVPHVYTMSPTKEEMTQNEVSITCMVKGFYPPDIYVEWQMNGQPQENYKNTPPTMDTDGSYFLYSKLNVKKEKWQQGNTFTCSVLHEGLHNHHTEKSLSHSPGK

SEQ ID NO: 210 - protein, 351 aa, synthetic construct
MAQLLFNKTKSVEFTFCNDTVVIPCFVTNMEAQNTTEVYVKWKFKGRDIYTFDGALNKSTVPTDFSSAKIEVSQLLKGDASLKMDKSDAVSHTGNYTCEVTELTREGETIIELKYRVVSWFSPNEAAASPSTCSKPTCPSEVSSVFIFPPKPKDVLTITLTPKVTCVVVDISQDDPEVHFSWFVDDVEVHTAQTRPPEEQFNSTFRSVSELPILHQDWLNGRTFRCKVTSAAFPSPIEKTISKPERTQVPHVYTMSPTKEEMTQNEVSITCMVKGFYPPDIYVEWQMNGQPQENYKNTPPTMDTDGSYFLYSKLNVKKEKWQQGNTFTCSVLHEGLHNHHTEKSLSHSPGK

SEQ ID NO: 211 - protein, 486 aa, synthetic construct
MAVPRWRQQWSGPGTTKRFPETVLARCVKYTEIHPEMRHVDCQSVWDAFKGAFISKHPCNITEEDYQPLMKLGTQTVPCNKILLWSRIKDLAHQFTQVQRDMFTLEDTLLGYLADDLTWCGEFNTSKINYQSCPDWRKDCSNNPVSVFWKTVSRRFAEAACDVVHVMLNGSRSKIFDKNSTFGSVEVHNLQPEKVQTLEAWVIHGGREDSRDLCQDPTIKELESIISKRNIQFSCKNIYRPDKFLQCVKNPEDSSCTSEIGGGSPSTCSKPTCPSEVSSVFIFPPKPKDVLTITLTPKVTCVVVDISQDDPEVHFSWFVDDVEVHTAQTRPPEEQFNSTFRSVSELPILHQDWLNGRTFRCKVTSAAFPSPIEKTISKPERTQVPHVYTMSPTKEEMTQNEVSITCMVKGFYPPDIYVEWQMNGQPQENYKNTPPTMDTDGSYFLYSKLNVKKEKWQQGNTFTCSVLHEGLHNHHTEKSLSHSPGK

SEQ ID NO: 212 - protein, 486 aa, synthetic construct
MAVPRWRQQWSGPGTTKRFPETVLARCVKYTEIHPEMRHVDCQSVWDAFKGAFISKHPCNITEEDYQPLMKLGTQTVPCNKKLLWSRIKDLAHQFTQVQRDMFTLEDTLLGYLADDLTWCGEFNTSKINYQSCPDWRKDCSNNPVSVFWKTVSRRFAEAACDVVHVMLNGSRSKIFDKNSTFGSVEVHNLQPEKVQTLEAWVIHGGREDSRDLCQDPTIKELESIISKRNIQFSCKNIYRPDKFLQCVKNPEDSSCTSEIGGGSPSTCSKPTCPSEVSSVFIFPPKPKDVLTITLTPKVTCVVVDISQDDPEVHFSWFVDDVEVHTAQTRPPEEQFNSTFRSVSELPILHQDWLNGRTFRCKVTSAAFPSPIEKTISKPERTQVPHVYTMSPTKEEMTQNEVSITCMVKGFYPPDIYVEWQMNGQPQENYKNTPPTMDTDGSYFLYSKLNVKKEKWQQGNTFTCSVLHEGLHNHHTEKSLSHSPGK

SEQ ID NO: 213 - protein, 351 aa, synthetic construct
MAQLLFNKTKSVEFTFCNDTVVIPCFVTNMEAQNTTEVYVKWKFKGRDIYTFDGALNKSTVPTDFSSAKIEVSQLLKGDASLKMDKSDAVSHTGNYTCEVTELTREGETIIELKYRVVSWFSPNEGGGSPSTCSKPTCPSEVSSVFIFPPKPKDVLTITLTPKVTCVVVDISQDDPEVHFSWFVDDVEVHTAQTRPPEEQFNSTFRSVSELPILHQDWLNGRTFRCKVTSAAFPSPIEKTISKPERTQVPHVYTMSPTKEEMTQNEVSITCMVKGFYPPDIYVEWQMNGQPQENYKNTPPTMDTDGSYFLYSKLNVKKEKWQQGNTFTCSVLHEGLHNHHTEKSLSHSPGK

SEQ ID NO: 214 - protein, 482 aa, synthetic construct
MAVPRWRQQWSGPGTTKRFPETVLARCVKYTEIHPEMRHVDCQSVWDAFKGAFISKHPCNITEEDYQPLMKLGTQTVPCNKILLWSRIKDLAHQFTQVQRDMFTLEDTLLGYLADDLTWCGEFNTSKINYQSCPDWRKDCSNNPVSVFWKTVSRRFAEAACDVVHVMLNGSRSKIFDKNSTFGSVEVHNLQPEKVQTLEAWVIHGGREDSRDLCQDPTIKELESIISKRNIQFSCKNIYRPDKFLQCVKNPEDSSCTSEIPSTCSKPTCPSEVSSVFIFPPKPKDVLTITLTPKVTCVVVDISQDDPEVHFSWFVDDVEVHTAQTRPPEEQFNSTFRSVSELPILHQDWLNGRTFRCKVTSAAFPSPIEKTISKPERTQVPHVYTMSPTKEEMTQNEVSITCMVKGFYPPDIYVEWQMNGQPQENYKNTPPTMDTDGSYFLYSKLNVKKEKWQQGNTFTCSVLHEGLHNHHTEKSLSHSPGK

SEQ ID NO: 215 - protein, 482 aa, synthetic construct
MAVPRWRQQWSGPGTTKRFPETVLARCVKYTEIHPEMRHVDCQSVWDAFKGAFISKHPCNITEEDYQPLMKLGTQTVPCNKKLLWSRIKDLAHQFTQVQRDMFTLEDTLLGYLADDLTWCGEFNTSKINYQSCPDWRKDCSNNPVSVFWKTVSRRFAEAACDVVHVMLNGSRSKIFDKNSTFGSVEVHNLQPEKVQTLEAWVIHGGREDSRDLCQDPTIKELESIISKRNIQFSCKNIYRPDKFLQCVKNPEDSSCTSEIPSTCSKPTCPSEVSSVFIFPPKPKDVLTITLTPKVTCVVVDISQDDPEVHFSWFVDDVEVHTAQTRPPEEQFNSTFRSVSELPILHQDWLNGRTFRCKVTSAAFPSPIEKTISKPERTQVPHVYTMSPTKEEMTQNEVSITCMVKGFYPPDIYVEWQMNGQPQENYKNTPPTMDTDGSYFLYSKLNVKKEKWQQGNTFTCSVLHEGLHNHHTEKSLSHSPGK

SEQ ID NO: 216 - protein, 347 aa, synthetic construct
MAQLLFNKTKSVEFTFCNDTVVIPCFVTNMEAQNTTEVYVKWKFKGRDIYTFDGALNKSTVPTDFSSAKIEVSQLLKGDASLKMDKSDAVSHTGNYTCEVTELTREGETIIELKYRVVSWFSPNEPSTCSKPTCPSEVSSVFIFPPKPKDVLTITLTPKVTCVVVDISQDDPEVHFSWFVDDVEVHTAQTRPPEEQFNSTFRSVSELPILHQDWLNGRTFRCKVTSAAFPSPIEKTISKPERTQVPHVYTMSPTKEEMTQNEVSITCMVKGFYPPDIYVEWQMNGQPQENYKNTPPTMDTDGSYFLYSKLNVKKEKWQQGNTFTCSVLHEGLHNHHTEKSLSHSPGK

SEQ ID NO: 217 - protein, 482 aa, synthetic construct
MAVPRWRQQWSGPGTTKRFPETVLARCVKYTEIHPEMRHVDCQSVWDAFKGAFISKHPCNITEEDYQPLMKLGTQTVPCNKILLWSRIKDLAHQFTQVQRDMFTLEDTLLGYLADDLTWCGEFNTSKINYQSCPDWRKDCSNNPVSVFWKTVSRRFAEAACDVVHVMLNGSRSKIFDKNSTFGSVEVHNLQPEKVQTLEAWVIHGGREDSRDLCQDPTIKELESIISKRNIQFSCKNIYRPDKFLQCVKNPEDSSCTSEIAAASNPCGCTSEVSSVFIFPPKPKDVLTITLTPKVTCVVVDISQDDPEVHFSWFVDDVEVHTAQTRPPEEQFNSTFRSVSELPILHQDWLNGRTFRCKVTSAAFPSPIEKTISKPERTQVPHVYTMSPTKEEMTQNEVSITCMVKGFYPPDIYVEWQMNGQPQENYKNTPPTMDTDGSYFLYSKLNVKKEKWQQGNTFTCSVLHEGLHNHHTEKSLSHSPGK

SEQ ID NO: 218 - protein, 482 aa, synthetic construct
MAVPRWRQQWSGPGTTKRFPETVLARCVKYTEIHPEMRHVDCQSVWDAFKGAFISKHPCNITEEDYQPLMKLGTQTVPCNKKLLWSRIKDLAHQFTQVQRDMFTLEDTLLGYLADDLTWCGEFNTSKINYQSCPDWRKDCSNNPVSVFWKTVSRRFAEAACDVVHVMLNGSRSKIFDKNSTFGSVEVHNLQPEKVQTLEAWVIHGGREDSRDLCQDPTIKELESIISKRNIQFSCKNIYRPDKFLQCVKNPEDSSCTSEIAAASNPCGCTSEVSSVFIFPPKPKDVLTITLTPKVTCVVVDISQDDPEVHFSWFVDDVEVHTAQTRPPEEQFNSTFRSVSELPILHQDWLNGRTFRCKVTSAAFPSPIEKTISKPERTQVPHVYTMSPTKEEMTQNEVSITCMVKGFYPPDIYVEWQMNGQPQENYKNTPPTMDTDGSYFLYSKLNVKKEKWQQGNTFTCSVLHEGLHNHHTEKSLSHSPGK

SEQ ID NO: 219 - protein, 347 aa, synthetic construct
MAQLLFNKTKSVEFTFCNDTVVIPCFVTNMEAQNTTEVYVKWKFKGRDIYTFDGALNKSTVPTDFSSAKIEVSQLLKGDASLKMDKSDAVSHTGNYTCEVTELTREGETIIELKYRVVSWFSPNEAAASNPCGCTSEVSSVFIFPPKPKDVLTITLTPKVTCVVVDISQDDPEVHFSWFVDDVEVHTAQTRPPEEQFNSTFRSVSELPILHQDWLNGRTFRCKVTSAAFPSPIEKTISKPERTQVPHVYTMSPTKEEMTQNEVSITCMVKGFYPPDIYVEWQMNGQPQENYKNTPPTMDTDGSYFLYSKLNVKKEKWQQGNTFTCSVLHEGLHNHHTEKSLSHSPGK

SEQ ID NO: 220 - protein, 482 aa, synthetic construct
MAVPRWRQQWSGPGTTKRFPETVLARCVKYTEIHPEMRHVDCQSVWDAFKGAFISKHPCNITEEDYQPLMKLGTQTVPCNKILLWSRIKDLAHQFTQVQRDMFTLEDTLLGYLADDLTWCGEFNTSKINYQSCPDWRKDCSNNPVSVFWKTVSRRFAEAACDVVHVMLNGSRSKIFDKNSTFGSVEVHNLQPEKVQTLEAWVIHGGREDSRDLCQDPTIKELESIISKRNIQFSCKNIYRPDKFLQCVKNPEDSSCTSEIGGGSNPCGCTSEVSSVFIFPPKPKDVLTITLTPKVTCVVVDISQDDPEVHFSWFVDDVEVHTAQTRPPEEQFNSTFRSVSELPILHQDWLNGRTFRCKVTSAAFPSPIEKTISKPERTQVPHVYTMSPTKEEMTQNEVSITCMVKGFYPPDIYVEWQMNGQPQENYKNTPPTMDTDGSYFLYSKLNVKKEKWQQGNTFTCSVLHEGLHNHHTEKSLSHSPGK

SEQ ID NO: 221 - protein, 482 aa, synthetic construct
MAVPRWRQQWSGPGTTKRFPETVLARCVKYTEIHPEMRHVDCQSVWDAFKGAFISKHPCNITEEDYQPLMKLGTQTVPCNKKLLWSRIKDLAHQFTQVQRDMFTLEDTLLGYLADDLTWCGEFNTSKINYQSCPDWRKDCSNNPVSVFWKTVSRRFAEAACDVVHVMLNGSRSKIFDKNSTFGSVEVHNLQPEKVQTLEAWVIHGGREDSRDLCQDPTIKELESIISKRNIQFSCKNIYRPDKFLQCVKNPEDSSCTSEIGGGSNPCGCTSEVSSVFIFPPKPKDVLTITLTPKVTCVVVDISQDDPEVHFSWFVDDVEVHTAQTRPPEEQFNSTFRSVSELPILHQDWLNGRTFRCKVTSAAFPSPIEKTISKPERTQVPHVYTMSPTKEEMTQNEVSITCMVKGFYPPDIYVEWQMNGQPQENYKNTPPTMDTDGSYFLYSKLNVKKEKWQQGNTFTCSVLHEGLHNHHTEKSLSHSPGK

SEQ ID NO: 222 - protein, 347 aa, synthetic construct
MAQLLFNKTKSVEFTFCNDTVVIPCFVTNMEAQNTTEVYVKWKFKGRDIYTFDGALNKSTVPTDFSSAKIEVSQLLKGDASLKMDKSDAVSHTGNYTCEVTELTREGETIIELKYRVVSWFSPNEGGGSNPCGCTSEVSSVFIFPPKPKDVLTITLTPKVTCVVVDISQDDPEVHFSWFVDDVEVHTAQTRPPEEQFNSTFRSVSELPILHQDWLNGRTFRCKVTSAAFPSPIEKTISKPERTQVPHVYTMSPTKEEMTQNEVSITCMVKGFYPPDIYVEWQMNGQPQENYKNTPPTMDTDGSYFLYSKLNVKKEKWQQGNTFTCSVLHEGLHNHHTEKSLSHSPGK

SEQ ID NO: 223 - protein, 486 aa, synthetic construct
MAVPRWRQQWSGPGTTKRFPETVLARCVKYTEIHPEMRHVDCQSVWDAFKGAFISKHPCNITEEDYQPLMKLGTQTVPCNKILLWSRIKDLAHQFTQVQRDMFTLEDTLLGYLADDLTWCGEFNTSKINYQSCPDWRKDCSNNPVSVFWKTVSRRFAEAACDVVHVMLNGSRSKIFDKNSTFGSVEVHNLQPEKVQTLEAWVIHGGREDSRDLCQDPTIKELESIISKRNIQFSCKNIYRPDKFLQCVKNPEDSSCTSEIAAASDKTHTCPPCPSEVSSVFIFPPKPKDVLTITLTPKVTCVVVDISQDDPEVHFSWFVDDVEVHTAQTRPPEEQFNSTFRSVSELPILHQDWLNGRTFRCKVTSAAFPSPIEKTISKPERTQVPHVYTMSPTKEEMTQNEVSITCMVKGFYPPDIYVEWQMNGQPQENYKNTPPTMDTDGSYFLYSKLNVKKEKWQQGNTFTCSVLHEGLHNHHTEKSLSHSPGK

SEQ ID NO: 224 - protein, 486 aa, synthetic construct
MAVPRWRQQWSGPGTTKRFPETVLARCVKYTEIHPEMRHVDCQSVWDAFKGAFISKHPCNITEEDYQPLMKLGTQTVPCNKKLLWSRIKDLAHQFTQVQRDMFTLEDTLLGYLADDLTWCGEFNTSKINYQSCPDWRKDCSNNPVSVFWKTVSRRFAEAACDVVHVMLNGSRSKIFDKNSTFGSVEVHNLQPEKVQTLEAWVIHGGREDSRDLCQDPTIKELESIISKRNIQFSCKNIYRPDKFLQCVKNPEDSSCTSEIAAASDKTHTCPPCPSEVSSVFIFPPKPKDVLTITLTPKVTCVVVDISQDDPEVHFSWFVDDVEVHTAQTRPPEEQFNSTFRSVSELPILHQDWLNGRTFRCKVTSAAFPSPIEKTISKPERTQVPHVYTMSPTKEEMTQNEVSITCMVKGFYPPDIYVEWQMNGQPQENYKNTPPTMDTDGSYFLYSKLNVKKEKWQQGNTFTCSVLHEGLHNHHTEKSLSHSPGK

SEQ ID NO: 225 - protein, 351 aa, synthetic construct
MAQLLFNKTKSVEFTFCNDTVVIPCFVTNMEAQNTTEVYVKWKFKGRDIYTFDGALNKSTVPTDFSSAKIEVSQLLKGDASLKMDKSDAVSHTGNYTCEVTELTREGETIIELKYRVVSWFSPNEAAASDKTHTCPPCPSEVSSVFIFPPKPKDVLTITLTPKVTCVVVDISQDDPEVHFSWFVDDVEVHTAQTRPPEEQFNSTFRSVSELPILHQDWLNGRTFRCKVTSAAFPSPIEKTISKPERTQVPHVYTMSPTKEEMTQNEVSITCMVKGFYPPDIYVEWQMNGQPQENYKNTPPTMDTDGSYFLYSKLNVKKEKWQQGNTFTCSVLHEGLHNHHTEKSLSHSPGK

SEQ ID NO: 226 - protein, 486 aa, synthetic construct
MAVPRWRQQWSGPGTTKRFPETVLARCVKYTEIHPEMRHVDCQSVWDAFKGAFISKHPCNITEEDYQPLMKLGTQTVPCNKILLWSRIKDLAHQFTQVQRDMFTLEDTLLGYLADDLTWCGEFNTSKINYQSCPDWRKDCSNNPVSVFWKTVSRRFAEAACDVVHVMLNGSRSKIFDKNSTFGSVEVHNLQPEKVQTLEAWVIHGGREDSRDLCQDPTIKELESIISKRNIQFSCKNIYRPDKFLQCVKNPEDSSCTSEIGGGSDKTHTCPPCPSEVSSVFIFPPKPKDVLTITLTPKVTCVVVDISQDDPEVHFSWFVDDVEVHTAQTRPPEEQFNSTFRSVSELPILHQDWLNGRTFRCKVTSAAFPSPIEKTISKPERTQVPHVYTMSPTKEEMTQNEVSITCMVKGFYPPDIYVEWQMNGQPQENYKNTPPTMDTDGSYFLYSKLNVKKEKWQQGNTFTCSVLHEGLHNHHTEKSLSHSPGK

SEQ ID NO: 227 - protein, 486 aa, synthetic construct
MAVPRWRQQWSGPGTTKRFPETVLARCVKYTEIHPEMRHVDCQSVWDAFKGAFISKHPCNITEEDYQPLMKLGTQTVPCNKKLLWSRIKDLAHQFTQVQRDMFTLEDTLLGYLADDLTWCGEFNTSKINYQSCPDWRKDCSNNPVSVFWKTVSRRFAEAACDVVHVMLNGSRSKIFDKNSTFGSVEVHNLQPEKVQTLEAWVIHGGREDSRDLCQDPTIKELESIISKRNIQFSCKNIYRPDKFLQCVKNPEDSSCTSEIGGGSDKTHTCPPCPSEVSSVFIFPPKPKDVLTITLTPKVTCVVVDISQDDPEVHFSWFVDDVEVHTAQTRPPEEQFNSTFRSVSELPILHQDWLNGRTFRCKVTSAAFPSPIEKTISKPERTQVPHVYTMSPTKEEMTQNEVSITCMVKGFYPPDIYVEWQMNGQPQENYKNTPPTMDTDGSYFLYSKLNVKKEKWQQGNTFTCSVLHEGLHNHHTEKSLSHSPGK

SEQ ID NO: 228 - protein, 351 aa, synthetic construct
MAQLLFNKTKSVEFTFCNDTVVIPCFVTNMEAQNTTEVYVKWKFKGRDIYTFDGALNKSTVPTDFSSAKIEVSQLLKGDASLKMDKSDAVSHTGNYTCEVTELTREGETIIELKYRVVSWFSPNEGGGSDKTHTCPPCPSEVSSVFIFPPKPKDVLTITLTPKVTCVVVDISQDDPEVHFSWFVDDVEVHTAQTRPPEEQFNSTFRSVSELPILHQDWLNGRTFRCKVTSAAFPSPIEKTISKPERTQVPHVYTMSPTKEEMTQNEVSITCMVKGFYPPDIYVEWQMNGQPQENYKNTPPTMDTDGSYFLYSKLNVKKEKWQQGNTFTCSVLHEGLHNHHTEKSLSHSPGK

SEQ ID NO: 229 - protein, 482 aa, synthetic construct
MAVPRWRQQWSGPGTTKRFPETVLARCVKYTEIHPEMRHVDCQSVWDAFKGAFISKHPCNITEEDYQPLMKLGTQTVPCNKILLWSRIKDLAHQFTQVQRDMFTLEDTLLGYLADDLTWCGEFNTSKINYQSCPDWRKDCSNNPVSVFWKTVSRRFAEAACDVVHVMLNGSRSKIFDKNSTFGSVEVHNLQPEKVQTLEAWVIHGGREDSRDLCQDPTIKELESIISKRNIQFSCKNIYRPDKFLQCVKNPEDSSCTSEIDKTHTCPPCPSEVSSVFIFPPKPKDVLTITLTPKVTCVVVDISQDDPEVHFSWFVDDVEVHTAQTRPPEEQFNSTFRSVSELPILHQDWLNGRTFRCKVTSAAFPSPIEKTISKPERTQVPHVYTMSPTKEEMTQNEVSITCMVKGFYPPDIYVEWQMNGQPQENYKNTPPTMDTDGSYFLYSKLNVKKEKWQQGNTFTCSVLHEGLHNHHTEKSLSHSPGK

SEQ ID NO: 230 - protein, 482 aa, synthetic construct
MAVPRWRQQWSGPGTTKRFPETVLARCVKYTEIHPEMRHVDCQSVWDAFKGAFISKHPCNITEEDYQPLMKLGTQTVPCNKKLLWSRIKDLAHQFTQVQRDMFTLEDTLLGYLADDLTWCGEFNTSKINYQSCPDWRKDCSNNPVSVFWKTVSRRFAEAACDVVHVMLNGSRSKIFDKNSTFGSVEVHNLQPEKVQTLEAWVIHGGREDSRDLCQDPTIKELESIISKRNIQFSCKNIYRPDKFLQCVKNPEDSSCTSEIDKTHTCPPCPSEVSSVFIFPPKPKDVLTITLTPKVTCVVVDISQDDPEVHFSWFVDDVEVHTAQTRPPEEQFNSTFRSVSELPILHQDWLNGRTFRCKVTSAAFPSPIEKTISKPERTQVPHVYTMSPTKEEMTQNEVSITCMVKGFYPPDIYVEWQMNGQPQENYKNTPPTMDTDGSYFLYSKLNVKKEKWQQGNTFTCSVLHEGLHNHHTEKSLSHSPGK

SEQ ID NO: 231 - protein, 351 aa, synthetic construct; identical to SEQ ID NO: 228

SEQ ID NO: 232 - protein, 482 aa, synthetic construct; identical to SEQ ID NO: 229

SEQ ID NO: 233 - protein, 482 aa, synthetic construct; identical to SEQ ID NO: 230

SEQ ID NO: 234 - protein, 347 aa, synthetic construct
MAQLLFNKTKSVEFTFCNDTVVIPCFVTNMEAQNTTEVYVKWKFKGRDIYTFDGALNKSTVPTDFSSAKIEVSQLLKGDASLKMDKSDAVSHTGNYTCEVTELTREGETIIELKYRVVSWFSPNEDKTHTCPPCPSEVSSVFIFPPKPKDVLTITLTPKVTCVVVDISQDDPEVHFSWFVDDVEVHTAQTRPPEEQFNSTFRSVSELPILHQDWLNGRTFRCKVTSAAFPSPIEKTISKPERTQVPHVYTMSPTKEEMTQNEVSITCMVKGFYPPDIYVEWQMNGQPQENYKNTPPTMDTDGSYFLYSKLNVKKEKWQQGNTFTCSVLHEGLHNHHTEKSLSHSPGK

SEQ ID NO: 235 - protein, 483 aa, synthetic construct
MAVPRWRQQWSGPGTTKRFPETVLARCVKYTEIHPEMRHVDCQSVWDAFKGAFISKHPCNITEEDYQPLMKLGTQTVPCNKILLWSRIKDLAHQFTQVQRDMFTLEDTLLGYLADDLTWCGEFNTSKINYQSCPDWRKDCSNNPVSVFWKTVSRRFAEAACDVVHVMLNGSRSKIFDKNSTFGSVEVHNLQPEKVQTLEAWVIHGGREDSRDLCQDPTIKELESIISKRNIQFSCKNIYRPDKFLQCVKNPEDSSCTSEIAAASPPCKCPASEVSSVFIFPPKTKDVLTITLTPKVTCVVVDISQNDPEVRFSWFIDDVEVHTAQTHAPEKQSNSTLRSVSELPIVHRDWLNGKTFKCKVNSGAFPAPIEKSISKPETPRGPQVYTMAPPKEEMTQSQVSITCMVKGFYPPDIYTEWKMNGQPQENYKNTPPTMDTDGSYFLYSKLNVKKETWQQGNTFTCSVLHEGLHNHHTEKSLSHSPGK

SEQ ID NO: 236 - protein, 483 aa, synthetic construct
MAVPRWRQQWSGPGTTKRFPETVLARCVKYTEIHPEMRHVDCQSVWDAFKGAFISKHPCNITEEDYQPLMKLGTQTVPCNKKLLWSRIKDLAHQFTQVQRDMFTLEDTLLGYLADDLTWCGEFNTSKINYQSCPDWRKDCSNNPVSVFWKTVSRRFAEAACDVVHVMLNGSRSKIFDKNSTFGSVEVHNLQPEKVQTLEAWVIHGGREDSRDLCQDPTIKELESIISKRNIQFSCKNIYRPDKFLQCVKNPEDSSCTSEIAAASPPCKCPASEVSSVFIFPPKTKDVLTITLTPKVTCVVVDISQNDPEVRFSWFIDDVEVHTAQTHAPEKQSNSTLRSVSELPIVHRDWLNGKTFKCKVNSGAFPAPIEKSISKPETPRGPQVYTMAPPKEEMTQSQVSITCMVKGFYPPDIYTEWKMNGQPQENYKNTPPTMDTDGSYFLYSKLNVKKETWQQGNTFTCSVLHEGLHNHHTEKSLSHSPGK

SEQ ID NO: 237 - protein, 348 aa, synthetic construct
MAQLLFNKTKSVEFTFCNDTVVIPCFVTNMEAQNTTEVYVKWKFKGRDIYTFDGALNKSTVPTDFSSAKIEVSQLLKGDASLKMDKSDAVSHTGNYTCEVTELTREGETIIELKYRVVSWFSPNEAAASPPCKCPASEVSSVFIFPPKTKDVLTITLTPKVTCVVVDISQNDPEVRFSWFIDDVEVHTAQTHAPEKQSNSTLRSVSELPIVHRDWLNGKTFKCKVNSGAFPAPIEKSISKPETPRGPQVYTMAPPKEEMTQSQVSITCMVKGFYPPDIYTEWKMNGQPQENYKNTPPTMDTDGSYFLYSKLNVKKETWQQGNTFTCSVLHEGLHNHHTEKSLSHSPGK

SEQ ID NO: 238 - protein, 483 aa, synthetic construct
MAVPRWRQQWSGPGTTKRFPETVLARCVKYTEIHPEMRHVDCQSVWDAFKGAFISKHPCNITEEDYQPLMKLGTQTVPCNKILLWSRIKDLAHQFTQVQRDMFTLEDTLLGYLADDLTWCGEFNTSKINYQSCPDWRKDCSNNPVSVFWKTVSRRFAEAACDVVHVMLNGSRSKIFDKNSTFGSVEVHNLQPEKVQTLEAWVIHGGREDSRDLCQDPTIKELESIISKRNIQFSCKNIYRPDKFLQCVKNPEDSSCTSEIGGGSPPCKCPASEVSSVFIFPPKTKDVLTITLTPKVTCVVVDISQNDPEVRFSWFIDDVEVHTAQTHAPEKQSNSTLRSVSELPIVHRDWLNGKTFKCKVNSGAFPAPIEKSISKPETPRGPQVYTMAPPKEEMTQSQVSITCMVKGFYPPDIYTEWKMNGQPQENYKNTPPTMDTDGSYFLYSKLNVKKETWQQGNTFTCSVLHEGLHNHHTEKSLSHSPGK

SEQ ID NO: 239 - protein, 483 aa, synthetic construct
MAVPRWRQQWSGPGTTKRFPETVLARCVKYTEIHPEMRHVDCQSVWDAFKGAFISKHPCNITEEDYQPLMKLGTQTVPCNKKLLWSRIKDLAHQFTQVQRDMFTLEDTLLGYLADDLTWCGEFNTSKINYQSCPDWRKDCSNNPVSVFWKTVSRRFAEAACDVVHVMLNGSRSKIFDKNSTFGSVEVHNLQPEKVQTLEAWVIHGGREDSRDLCQDPTIKELESIISKRNIQFSCKNIYRPDKFLQCVKNPEDSSCTSEIGGGSPPCKCPASEVSSVFIFPPKTKDVLTITLTPKVTCVVVDISQNDPEVRFSWFIDDVEVHTAQTHAPEKQSNSTLRSVSELPIVHRDWLNGKTFKCKVNSGAFPAPIEKSISKPETPRGPQVYTMAPPKEEMTQSQVSITCMVKGFYPPDIYTEWKMNGQPQENYKNTPPTMDTDGSYFLYSKLNVKKETWQQGNTFTCSVLHEGLHNHHTEKSLSHSPGK

SEQ ID NO: 240 - protein, 348 aa, synthetic construct
MAQLLFNKTKSVEFTFCNDTVVIPCFVTNMEAQNTTEVYVKWKFKGRDIYTFDGALNKSTVPTDFSSAKIEVSQLLKGDASLKMDKSDAVSHTGNYTCEVTELTREGETIIELKYRVVSWFSPNEGGGSPPCKCPASEVSSVFIFPPKTKDVLTITLTPKVTCVVVDISQNDPEVRFSWFIDDVEVHTAQTHAPEKQSNSTLRSVSELPIVHRDWLNGKTFKCKVNSGAFPAPIEKSISKPETPRGPQVYTMAPPKEEMTQSQVSITCMVKGFYPPDIYTEWKMNGQPQENYKNTPPTMDTDGSYFLYSKLNVKKETWQQGNTFTCSVLHEGLHNHHTEKSLSHSPGK

SEQ ID NO: 241 - protein, 479 aa, synthetic construct
MAVPRWRQQWSGPGTTKRFPETVLARCVKYTEIHPEMRHVDCQSVWDAFKGAFISKHPCNITEEDYQPLMKLGTQTVPCNKILLWSRIKDLAHQFTQVQRDMFTLEDTLLGYLADDLTWCGEFNTSKINYQSCPDWRKDCSNNPVSVFWKTVSRRFAEAACDVVHVMLNGSRSKIFDKNSTFGSVEVHNLQPEKVQTLEAWVIHGGREDSRDLCQDPTIKELESIISKRNIQFSCKNIYRPDKFLQCVKNPEDSSCTSEIPPCKCPASEVSSVFIFPPKTKDVLTITLTPKVTCVVVDISQNDPEVRFSWFIDDVEVHTAQTHAPEKQSNSTLRSVSELPIVHRDWLNGKTFKCKVNSGAFPAPIEKSISKPETPRGPQVYTMAPPKEEMTQSQVSITCMVKGFYPPDIYTEWKMNGQPQENYKNTPPTMDTDGSYFLYSKLNVKKETWQQGNTFTCSVLHEGLHNHHTEKSLSHSPGK

SEQ ID NO: 242 - protein, 479 aa, synthetic construct
MAVPRWRQQWSGPGTTKRFPETVLARCVKYTEIHPEMRHVDCQSVWDAFKGAFISKHPCNITEEDYQPLMKLGTQTVPCNKKLLWSRIKDLAHQFTQVQRDMFTLEDTLLGYLADDLTWCGEFNTSKINYQSCPDWRKDCSNNPVSVFWKTVSRRFAEAACDVVHVMLNGSRSKIFDKNSTFGSVEVHNLQPEKVQTLEAWVIHGGREDSRDLCQDPTIKELESIISKRNIQFSCKNIYRPDKFLQCVKNPEDSSCTSEIPPCKCPASEVSSVFIFPPKTKDVLTITLTPKVTCVVVDISQNDPEVRFSWFIDDVEVHTAQTHAPEKQSNSTLRSVSELPIVHRDWLNGKTFKCKVNSGAFPAPIEKSISKPETPRGPQVYTMAPPKEEMTQSQVSITCMVKGFYPPDIYTEWKMNGQPQENYKNTPPTMDTDGSYFLYSKLNVKKETWQQGNTFTCSVLHEGLHNHHTEKSLSHSPGK

SEQ ID NO: 243 - protein, 344 aa, synthetic construct
MAQLLFNKTKSVEFTFCNDTVVIPCFVTNMEAQNTTEVYVKWKFKGRDIYTFDGALNKSTVPTDFSSAKIEVSQLLKGDASLKMDKSDAVSHTGNYTCEVTELTREGETIIELKYRVVSWFSPNEPPCKCPASEVSSVFIFPPKTKDVLTITLTPKVTCVVVDISQNDPEVRFSWFIDDVEVHTAQTHAPEKQSNSTLRSVSELPIVHRDWLNGKTFKCKVNSGAFPAPIEKSISKPETPRGPQVYTMAPPKEEMTQSQVSITCMVKGFYPPDIYTEWKMNGQPQENYKNTPPTMDTDGSYFLYSKLNVKKETWQQGNTFTCSVLHEGLHNHHTEKSLSHSPGK

SEQ ID NO: 244 - protein, 486 aa, synthetic construct
MAVPRWRQQWSGPGTTKRFPETVLARCVKYTEIHPEMRHVDCQSVWDAFKGAFISKHPCNITEEDYQPLMKLGTQTVPCNKILLWSRIKDLAHQFTQVQRDMFTLEDTLLGYLADDLTWCGEFNTSKINYQSCPDWRKDCSNNPVSVFWKTVSRRFAEAACDVVHVMLNGSRSKIFDKNSTFGSVEVHNLQPEKVQTLEAWVIHGGREDSRDLCQDPTIKELESIISKRNIQFSCKNIYRPDKFLQCVKNPEDSSCTSEIAAASPSTCSKPTCPSEVSSVFIFPPKTKDVLTITLTPKVTCVVVDISQNDPEVRFSWFIDDVEVHTAQTHAPEKQSNSTLRSVSELPIVHRDWLNGKTFKCKVNSGAFPAPIEKSISKPETPRGPQVYTMAPPKEEMTQSQVSITCMVKGFYPPDIYTEWKMNGQPQENYKNTPPTMDTDGSYFLYSKLNVKKETWQQGNTFTCSVLHEGLHNHHTEKSLSHSPGK

SEQ ID NO: 245 - protein, 486 aa, synthetic construct
MAVPRWRQQWSGPGTTKRFPETVLARCVKYTEIHPEMRHVDCQSVWDAFKGAFISKHPCNITEEDYQPLMKLGTQTVPCNKKLLWSRIKDLAHQFTQVQRDMFTLEDTLLGYLADDLTWCGEFNTSKINYQSCPDWRKDCSNNPVSVFWKTVSRRFAEAACDVVHVMLNGSRSKIFDKNSTFGSVEVHNLQPEKVQTLEAWVIHGGREDSRDLCQDPTIKELESIISKRNIQFSCKNIYRPDKFLQCVKNPEDSSCTSEIAAASPSTCSKPTCPSEVSSVFIFPPKTKDVLTITLTPKVTCVVVDISQNDPEVRFSWFIDDVEVHTAQTHAPEKQSNSTLRSVSELPIVHRDWLNGKTFKCKVNSGAFPAPIEKSISKPETPRGPQVYTMAPPKEEMTQSQVSITCMVKGFYPPDIYTEWKMNGQPQENYKNTPPTMDTDGSYFLYSKLNVKKETWQQGNTFTCSVLHEGLHNHHTEKSLSHSPGK

SEQ ID NO: 246 - protein, 351 aa, synthetic construct
MAQLLFNKTKSVEFTFCNDTVVIPCFVTNMEAQNTTEVYVKWKFKGRDIYTFDGALNKSTVPTDFSSAKIEVSQLLKGDASLKMDKSDAVSHTGNYTCEVTELTREGETIIELKYRVVSWFSPNEAAASPSTCSKPTCPSEVSSVFIFPPKTKDVLTITLTPKVTCVVVDISQNDPEVRFSWFIDDVEVHTAQTHAPEKQSNSTLRSVSELPIVHRDWLNGKTFKCKVNSGAFPAPIEKSISKPETPRGPQVYTMAPPKEEMTQSQVSITCMVKGFYPPDIYTEWKMNGQPQENYKNTPPTMDTDGSYFLYSKLNVKKETWQQGNTFTCSVLHEGLHNHHTEKSLSHSPGK

SEQ ID NO: 247 - protein, 486 aa, synthetic construct
MAVPRWRQQWSGPGTTKRFPETVLARCVKYTEIHPEMRHVDCQSVWDAFKGAFISKHPCNITEEDYQPLMKLGTQTVPCNKILLWSRIKDLAHQFTQVQRDMFTLEDTLLGYLADDLTWCGEFNTSKINYQSCPDWRKDCSNNPVSVFWKTVSRRFAEAACDVVHVMLNGSRSKIFDKNSTFGSVEVHNLQPEKVQTLEAWVIHGGREDSRDLCQDPTIKELESIISKRNIQFSCKNIYRPDKFLQCVKNPEDSSCTSEIGGGSPSTCSKPTCPSEVSSVFIFPPKTKDVLTITLTPKVTCVVVDISQNDPEVRFSWFIDDVEVHTAQTHAPEKQSNSTLRSVSELPIVHRDWLNGKTFKCKVNSGAFPAPIEKSISKPETPRGPQVYTMAPPKEEMTQSQVSITCMVKGFYPPDIYTEWKMNGQPQENYKNTPPTMDTDGSYFLYSKLNVKKETWQQGNTFTCSVLHEGLHNHHTEKSLSHSPGK

SEQ ID NO: 248 - protein, 486 aa, synthetic construct
MAVPRWRQQWSGPGTTKRFPETVLARCVKYTEIHPEMRHVDCQSVWDAFKGAFISKHPCNITEEDYQPLMKLGTQTVPCNKKLLWSRIKDLAHQFTQVQRDMFTLEDTLLGYLADDLTWCGEFNTSKINYQSCPDWRKDCSNNPVSVFWKTVSRRFAEAACDVVHVMLNGSRSKIFDKNSTFGSVEVHNLQPEKVQTLEAWVIHGGREDSRDLCQDPTIKELESIISKRNIQFSCKNIYRPDKFLQCVKNPEDSSCTSEIGGGSPSTCSKPTCPSEVSSVFIFPPKTKDVLTITLTPKVTCVVVDISQNDPEVRFSWFIDDVEVHTAQTHAPEKQSNSTLRSVSELPIVHRDWLNGKTFKCKVNSGAFPAPIEKSISKPETPRGPQVYTMAPPKEEMTQSQVSITCMVKGFYPPDIYTEWKMNGQPQENYKNTPPTMDTDGSYFLYSKLNVKKETWQQGNTFTCSVLHEGLHNHHTEKSLSHSPGK

SEQ ID NO: 249 - protein, 351 aa, synthetic construct
MAQLLFNKTKSVEFTFCNDTVVIPCFVTNMEAQNTTEVYVKWKFKGRDIYTFDGALNKSTVPTDFSSAKIEVSQLLKGDASLKMDKSDAVSHTGNYTCEVTELTREGETIIELKYRVVSWFSPNEGGGSPSTCSKPTCPSEVSSVFIFPPKTKDVLTITLTPKVTCVVVDISQNDPEVRFSWFIDDVEVHTAQTHAPEKQSNSTLRSVSELPIVHRDWLNGKTFKCKVNSGAFPAPIEKSISKPETPRGPQVYTMAPPKEEMTQSQVSITCMVKGFYPPDIYTEWKMNGQPQENYKNTPPTMDTDGSYFLYSKLNVKKETWQQGNTFTCSVLHEGLHNHHTEKSLSHSPGK

SEQ ID NO: 250 - protein, 482 aa, unidentified
MAVPRWRQQWSGPGTTKRFPETVLARCVKYTEIHPEMRHVDCQSVWDAFKGAFISKHPCNITEEDYQPLMKLGTQTVPCNKILLWSRIKDLAHQFTQVQRDMFTLEDTLLGYLADDLTWCGEFNTSKINYQSCPDWRKDCSNNPVSVFWKTVSRRFAEAACDVVHVMLNGSRSKIFDKNSTFGSVEVHNLQPEKVQTLEAWVIHGGREDSRDLCQDPTIKELESIISKRNIQFSCKNIYRPDKFLQCVKNPEDSSCTSEIPSTCSKPTCPSEVSSVFIFPPKTKDVLTITLTPKVTCVVVDISQNDPEVRFSWFIDDVEVHTAQTHAPEKQSNSTLRSVSELPIVHRDWLNGKTFKCKVNSGAFPAPIEKSISKPETPRGPQVYTMAPPKEEMTQSQVSITCMVKGFYPPDIYTEWKMNGQPQENYKNTPPTMDTDGSYFLYSKLNVKKETWQQGNTFTCSVLHEGLHNHHTEKSLSHSPGK

SEQ ID NO: 251 - protein, 482 aa, synthetic construct
MAVPRWRQQWSGPGTTKRFPETVLARCVKYTEIHPEMRHVDCQSVWDAFKGAFISKHPCNITEEDYQPLMKLGTQTVPCNKKLLWSRIKDLAHQFTQVQRDMFTLEDTLLGYLADDLTWCGEFNTSKINYQSCPDWRKDCSNNPVSVFWKTVSRRFAEAACDVVHVMLNGSRSKIFDKNSTFGSVEVHNLQPEKVQTLEAWVIHGGREDSRDLCQDPTIKELESIISKRNIQFSCKNIYRPDKFLQCVKNPEDSSCTSEIPSTCSKPTCPSEVSSVFIFPPKTKDVLTITLTPKVTCVVVDISQNDPEVRFSWFIDDVEVHTAQTHAPEKQSNSTLRSVSELPIVHRDWLNGKTFKCKVNSGAFPAPIEKSISKPETPRGPQVYTMAPPKEEMTQSQVSITCMVKGFYPPDIYTEWKMNGQPQENYKNTPPTMDTDGSYFLYSKLNVKKETWQQGNTFTCSVLHEGLHNHHTEKSLSHSPGK

SEQ ID NO: 252 - protein, 347 aa, synthetic construct
MAQLLFNKTKSVEFTFCNDTVVIPCFVTNMEAQNTTEVYVKWKFKGRDIYTFDGALNKSTVPTDFSSAKIEVSQLLKGDASLKMDKSDAVSHTGNYTCEVTELTREGETIIELKYRVVSWFSPNEPSTCSKPTCPSEVSSVFIFPPKTKDVLTITLTPKVTCVVVDISQNDPEVRFSWFIDDVEVHTAQTHAPEKQSNSTLRSVSELPIVHRDWLNGKTFKCKVNSGAFPAPIEKSISKPETPRGPQVYTMAPPKEEMTQSQVSITCMVKGFYPPDIYTEWKMNGQPQENYKNTPPTMDTDGSYFLYSKLNVKKETWQQGNTFTCSVLHEGLHNHHTEKSLSHSPGK

SEQ ID NO: 253 - protein, 482 aa, synthetic construct
MAVPRWRQQWSGPGTTKRFPETVLARCVKYTEIHPEMRHVDCQSVWDAFKGAFISKHPCNITEEDYQPLMKLGTQTVPCNKILLWSRIKDLAHQFTQVQRDMFTLEDTLLGYLADDLTWCGEFNTSKINYQSCPDWRKDCSNNPVSVFWKTVSRRFAEAACDVVHVMLNGSRSKIFDKNSTFGSVEVHNLQPEKVQTLEAWVIHGGREDSRDLCQDPTIKELESIISKRNIQFSCKNIYRPDKFLQCVKNPEDSSCTSEIAAASNPCGCTSEVSSVFIFPPKTKDVLTITLTPKVTCVVVDISQNDPEVRFSWFIDDVEVHTAQTHAPEKQSNSTLRSVSELPIVHRDWLNGKTFKCKVNSGAFPAPIEKSISKPETPRGPQVYTMAPPKEEMTQSQVSITCMVKGFYPPDIYTEWKMNGQPQENYKNTPPTMDTDGSYFLYSKLNVKKETWQQGNTFTCSVLHEGLHNHHTEKSLSHSPGK

SEQ ID NO: 254 - protein, 482 aa, synthetic construct
MAVPRWRQQWSGPGTTKRFPETVLARCVKYTEIHPEMRHVDCQSVWDAFKGAFISKHPCNITEEDYQPLMKLGTQTVPCNKKLLWSRIKDLAHQFTQVQRDMFTLEDTLLGYLADDLTWCGEFNTSKINYQSCPDWRKDCSNNPVSVFWKTVSRRFAEAACDVVHVMLNGSRSKIFDKNSTFGSVEVHNLQPEKVQTLEAWVIHGGREDSRDLCQDPTIKELESIISKRNIQFSCKNIYRPDKFLQCVKNPEDSSCTSEIAAASNPCGCTSEVSSVFIFPPKTKDVLTITLTPKVTCVVVDISQNDPEVRFSWFIDDVEVHTAQTHAPEKQSNSTLRSVSELPIVHRDWLNGKTFKCKVNSGAFPAPIEKSISKPETPRGPQVYTMAPPKEEMTQSQVSITCMVKGFYPPDIYTEWKMNGQPQENYKNTPPTMDTDGSYFLYSKLNVKKETWQQGNTFTCSVLHEGLHNHHTEKSLSHSPGK

SEQ ID NO: 255 - protein, 347 aa, synthetic construct
MAQLLFNKTKSVEFTFCNDTVVIPCFVTNMEAQNTTEVYVKWKFKGRDIYTFDGALNKSTVPTDFSSAKIEVSQLLKGDASLKMDKSDAVSHTGNYTCEVTELTREGETIIELKYRVVSWFSPNEAAASNPCGCTSEVSSVFIFPPKTKDVLTITLTPKVTCVVVDISQNDPEVRFSWFIDDVEVHTAQTHAPEKQSNSTLRSVSELPIVHRDWLNGKTFKCKVNSGAFPAPIEKSISKPETPRGPQVYTMAPPKEEMTQSQVSITCMVKGFYPPDIYTEWKMNGQPQENYKNTPPTMDTDGSYFLYSKLNVKKETWQQGNTFTCSVLHEGLHNHHTEKSLSHSPGK

SEQ ID NO: 256 - protein, 482 aa, synthetic construct
MAVPRWRQQWSGPGTTKRFPETVLARCVKYTEIHPEMRHVDCQSVWDAFKGAFISKHPCNITEEDYQPLMKLGTQTVPCNKILLWSRIKDLAHQFTQVQRDMFTLEDTLLGYLADDLTWCGEFNTSKINYQSCPDWRKDCSNNPVSVFWKTVSRRFAEAACDVVHVMLNGSRSKIFDKNSTFGSVEVHNLQPEKVQTLEAWVIHGGREDSRDLCQDPTIKELESIISKRNIQFSCKNIYRPDKFLQCVKNPEDSSCTSEIGGGSNPCGCTSEVSSVFIFPPKTKDVLTITLTPKVTCVVVDISQNDPEVRFSWFIDDVEVHTAQTHAPEKQSNSTLRSVSELPIVHRDWLNGKTFKCKVNSGAFPAPIEKSISKPETPRGPQVYTMAPPKEEMTQSQVSITCMVKGFYPPDIYTEWKMNGQPQENYKNTPPTMDTDGSYFLYSKLNVKKETWQQGNTFTCSVLHEGLHNHHTEKSLSHSPGK

SEQ ID NO: 257 - protein, 482 aa, synthetic construct
MAVPRWRQQWSGPGTTKRFPETVLARCVKYTEIHPEMRHVDCQSVWDAFKGAFISKHPCNITEEDYQPLMKLGTQTVPCNKKLLWSRIKDLAHQFTQVQRDMFTLEDTLLGYLADDLTWCGEFNTSKINYQSCPDWRKDCSNNPVSVFWKTVSRRFAEAACDVVHVMLNGSRSKIFDKNSTFGSVEVHNLQPEKVQTLEAWVIHGGREDSRDLCQDPTIKELESIISKRNIQFSCKNIYRPDKFLQCVKNPEDSSCTSEIGGGSNPCGCTSEVSSVFIFPPKTKDVLTITLTPKVTCVVVDISQNDPEVRFSWFIDDVEVHTAQTHAPEKQSNSTLRSVSELPIVHRDWLNGKTFKCKVNSGAFPAPIEKSISKPETPRGPQVYTMAPPKEEMTQSQVSITCMVKGFYPPDIYTEWKMNGQPQENYKNTPPTMDTDGSYFLYSKLNVKKETWQQGNTFTCSVLHEGLHNHHTEKSLSHSPGK

SEQ ID NO: 258 - protein, 347 aa, synthetic construct
MAQLLFNKTKSVEFTFCNDTVVIPCFVTNMEAQNTTEVYVKWKFKGRDIYTFDGALNKSTVPTDFSSAKIEVSQLLKGDASLKMDKSDAVSHTGNYTCEVTELTREGETIIELKYRVVSWFSPNEGGGSNPCGCTSEVSSVFIFPPKTKDVLTITLTPKVTCVVVDISQNDPEVRFSWFIDDVEVHTAQTHAPEKQSNSTLRSVSELPIVHRDWLNGKTFKCKVNSGAFPAPIEKSISKPETPRGPQVYTMAPPKEEMTQSQVSITCMVKGFYPPDIYTEWKMNGQPQENYKNTPPTMDTDGSYFLYSKLNVKKETWQQGNTFTCSVLHEGLHNHHTEKSLSHSPGK

SEQ ID NO: 259 - protein, 478 aa, synthetic construct
MAVPRWRQQWSGPGTTKRFPETVLARCVKYTEIHPEMRHVDCQSVWDAFKGAFISKHPCNITEEDYQPLMKLGTQTVPCNKILLWSRIKDLAHQFTQVQRDMFTLEDTLLGYLADDLTWCGEFNTSKINYQSCPDWRKDCSNNPVSVFWKTVSRRFAEAACDVVHVMLNGSRSKIFDKNSTFGSVEVHNLQPEKVQTLEAWVIHGGREDSRDLCQDPTIKELESIISKRNIQFSCKNIYRPDKFLQCVKNPEDSSCTSEINPCGCTSEVSSVFIFPPKTKDVLTITLTPKVTCVVVDISQNDPEVRFSWFIDDVEVHTAQTHAPEKQSNSTLRSVSELPIVHRDWLNGKTFKCKVNSGAFPAPIEKSISKPETPRGPQVYTMAPPKEEMTQSQVSITCMVKGFYPPDIYTEWKMNGQPQENYKNTPPTMDTDGSYFLYSKLNVKKETWQQGNTFTCSVLHEGLHNHHTEKSLSHSPGK

SEQ ID NO: 260 - protein, 478 aa, synthetic construct
MAVPRWRQQWSGPGTTKRFPETVLARCVKYTEIHPEMRHVDCQSVWDAFKGAFISKHPCNITEEDYQPLMKLGTQTVPCNKKLLWSRIKDLAHQFTQVQRDMFTLEDTLLGYLADDLTWCGEFNTSKINYQSCPDWRKDCSNNPVSVFWKTVSRRFAEAACDVVHVMLNGSRSKIFDKNSTFGSVEVHNLQPEKVQTLEAWVIHGGREDSRDLCQDPTIKELESIISKRNIQFSCKNIYRPDKFLQCVKNPEDSSCTSEINPCGCTSEVSSVFIFPPKTKDVLTITLTPKVTCVVVDISQNDPEVRFSWFIDDVEVHTAQTHAPEKQSNSTLRSVSELPIVHRDWLNGKTFKCKVNSGAFPAPIEKSISKPETPRGPQVYTMAPPKEEMTQSQVSITCMVKGFYPPDIYTEWKMNGQPQENYKNTPPTMDTDGSYFLYSKLNVKKETWQQGNTFTCSVLHEGLHNHHTEKSLSHSPGK

SEQ ID NO: 261 - protein, 343 aa, synthetic construct
MAQLLFNKTKSVEFTFCNDTVVIPCFVTNMEAQNTTEVYVKWKFKGRDIYTFDGALNKSTVPTDFSSAKIEVSQLLKGDASLKMDKSDAVSHTGNYTCEVTELTREGETIIELKYRVVSWFSPNENPCGCTSEVSSVFIFPPKTKDVLTITLTPKVTCVVVDISQNDPEVRFSWFIDDVEVHTAQTHAPEKQSNSTLRSVSELPIVHRDWLNGKTFKCKVNSGAFPAPIEKSISKPETPRGPQVYTMAPPKEEMTQSQVSITCMVKGFYPPDIYTEWKMNGQPQENYKNTPPTMDTDGSYFLYSKLNVKKETWQQGNTFTCSVLHEGLHNHHTEKSLSHSPGK

SEQ ID NO: 262 - protein, 486 aa, synthetic construct
MAVPRWRQQWSGPGTTKRFPETVLARCVKYTEIHPEMRHVDCQSVWDAFKGAFISKHPCNITEEDYQPLMKLGTQTVPCNKILLWSRIKDLAHQFTQVQRDMFTLEDTLLGYLADDLTWCGEFNTSKINYQSCPDWRKDCSNNPVSVFWKTVSRRFAEAACDVVHVMLNGSRSKIFDKNSTFGSVEVHNLQPEKVQTLEAWVIHGGREDSRDLCQDPTIKELESIISKRNIQFSCKNIYRPDKFLQCVKNPEDSSCTSEIAAASDKTHTCPPCPSEVSSVFIFPPKTKDVLTITLTPKVTCVVVDISQNDPEVRFSWFIDDVEVHTAQTHAPEKQSNSTLRSVSELPIVHRDWLNGKTFKCKVNSGAFPAPIEKSISKPETPRGPQVYTMAPPKEEMTQSQVSITCMVKGFYPPDIYTEWKMNGQPQENYKNTPPTMDTDGSYFLYSKLNVKKETWQQGNTFTCSVLHEGLHNHHTEKSLSHSPGK

SEQ ID NO: 263 - protein, 486 aa, synthetic construct
MAVPRWRQQWSGPGTTKRFPETVLARCVKYTEIHPEMRHVDCQSVWDAFKGAFISKHPCNITEEDYQPLMKLGTQTVPCNKKLLWSRIKDLAHQFTQVQRDMFTLEDTLLGYLADDLTWCGEFNTSKINYQSCPDWRKDCSNNPVSVFWKTVSRRFAEAACDVVHVMLNGSRSKIFDKNSTFGSVEVHNLQPEKVQTLEAWVIHGGREDSRDLCQDPTIKELESIISKRNIQFSCKNIYRPDKFLQCVKNPEDSSCTSEIAAASDKTHTCPPCPSEVSSVFIFPPKTKDVLTITLTPKVTCVVVDISQNDPEVRFSWFIDDVEVHTAQTHAPEKQSNSTLRSVSELPIVHRDWLNGKTFKCKVNSGAFPAPIEKSISKPETPRGPQVYTMAPPKEEMTQSQVSITCMVKGFYPPDIYTEWKMNGQPQENYKNTPPTMDTDGSYFLYSKLNVKKETWQQGNTFTCSVLHEGLHNHHTEKSLSHSPGK

SEQ ID NO: 264 - protein, 351 aa, synthetic construct
MAQLLFNKTKSVEFTFCNDTVVIPCFVTNMEAQNTTEVYVKWKFKGRDIYTFDGALNKSTVPTDFSSAKIEVSQLLKGDASLKMDKSDAVSHTGNYTCEVTELTREGETIIELKYRVVSWFSPNEAAASDKTHTCPPCPSEVSSVFIFPPKTKDVLTITLTPKVTCVVVDISQNDPEVRFSWFIDDVEVHTAQTHAPEKQSNSTLRSVSELPIVHRDWLNGKTFKCKVNSGAFPAPIEKSISKPETPRGPQVYTMAPPKEEMTQSQVSITCMVKGFYPPDIYTEWKMNGQPQENYKNTPPTMDTDGSYFLYSKLNVKKETWQQGNTFTCSVLHEGLHNHHTEKSLSHSPGK

SEQ ID NO: 265 - protein, 486 aa, synthetic construct
MAVPRWRQQWSGPGTTKRFPETVLARCVKYTEIHPEMRHVDCQSVWDAFKGAFISKHPCNITEEDYQPLMKLGTQTVPCNKILLWSRIKDLAHQFTQVQRDMFTLEDTLLGYLADDLTWCGEFNTSKINYQSCPDWRKDCSNNPVSVFWKTVSRRFAEAACDVVHVMLNGSRSKIFDKNSTFGSVEVHNLQPEKVQTLEAWVIHGGREDSRDLCQDPTIKELESIISKRNIQFSCKNIYRPDKFLQCVKNPEDSSCTSEIGGGSDKTHTCPPCPSEVSSVFIFPPKTKDVLTITLTPKVTCVVVDISQNDPEVRFSWFIDDVEVHTAQTHAPEKQSNSTLRSVSELPIVHRDWLNGKTFKCKVNSGAFPAPIEKSISKPETPRGPQVYTMAPPKEEMTQSQVSITCMVKGFYPPDIYTEWKMNGQPQENYKNTPPTMDTDGSYFLYSKLNVKKETWQQGNTFTCSVLHEGLHNHHTEKSLSHSPGK

SEQ ID NO: 266 - protein, 486 aa, synthetic construct
MAVPRWRQQWSGPGTTKRFPETVLARCVKYTEIHPEMRHVDCQSVWDAFKGAFISKHPCNITEEDYQPLMKLGTQTVPCNKKLLWSRIKDLAHQFTQVQRDMFTLEDTLLGYLADDLTWCGEFNTSKINYQSCPDWRKDCSNNPVSVFWKTVSRRFAEAACDVVHVMLNGSRSKIFDKNSTFGSVEVHNLQPEKVQTLEAWVIHGGREDSRDLCQDPTIKELESIISKRNIQFSCKNIYRPDKFLQCVKNPEDSSCTSEIGGGSDKTHTCPPCPSEVSSVFIFPPKTKDVLTITLTPKVTCVVVDISQNDPEVRFSWFIDDVEVHTAQTHAPEKQSNSTLRSVSELPIVHRDWLNGKTFKCKVNSGAFPAPIEKSISKPETPRGPQVYTMAPPKEEMTQSQVSITCMVKGFYPPDIYTEWKMNGQPQENYKNTPPTMDTDGSYFLYSKLNVKKETWQQGNTFTCSVLHEGLHNHHTEKSLSHSPGK

SEQ ID NO: 267 - protein, 351 aa, synthetic construct
MAQLLFNKTKSVEFTFCNDTVVIPCFVTNMEAQNTTEVYVKWKFKGRDIYTFDGALNKSTVPTDFSSAKIEVSQLLKGDASLKMDKSDAVSHTGNYTCEVTELTREGETIIELKYRVVSWFSPNEGGGSDKTHTCPPCPSEVSSVFIFPPKTKDVLTITLTPKVTCVVVDISQNDPEVRFSWFIDDVEVHTAQTHAPEKQSNSTLRSVSELPIVHRDWLNGKTFKCKVNSGAFPAPIEKSISKPETPRGPQVYTMAPPKEEMTQSQVSITCMVKGFYPPDIYTEWKMNGQPQENYKNTPPTMDTDGSYFLYSKLNVKKETWQQGNTFTCSVLHEGLHNHHTEKSLSHSPGK

SEQ ID NO: 268 - protein, 482 aa, synthetic construct
MAVPRWRQQWSGPGTTKRFPETVLARCVKYTEIHPEMRHVDCQSVWDAFKGAFISKHPCNITEEDYQPLMKLGTQTVPCNKILLWSRIKDLAHQFTQVQRDMFTLEDTLLGYLADDLTWCGEFNTSKINYQSCPDWRKDCSNNPVSVFWKTVSRRFAEAACDVVHVMLNGSRSKIFDKNSTFGSVEVHNLQPEKVQTLEAWVIHGGREDSRDLCQDPTIKELESIISKRNIQFSCKNIYRPDKFLQCVKNPEDSSCTSEIDKTHTCPPCPSEVSSVFIFPPKTKDVLTITLTPKVTCVVVDISQNDPEVRFSWFIDDVEVHTAQTHAPEKQSNSTLRSVSELPIVHRDWLNGKTFKCKVNSGAFPAPIEKSISKPETPRGPQVYTMAPPKEEMTQSQVSITCMVKGFYPPDIYTEWKMNGQPQENYKNTPPTMDTDGSYFLYSKLNVKKETWQQGNTFTCSVLHEGLHNHHTEKSLSHSPGK

SEQ ID NO: 269 - protein, 482 aa, synthetic construct
MAVPRWRQQWSGPGTTKRFPETVLARCVKYTEIHPEMRHVDCQSVWDAFKGAFISKHPCNITEEDYQPLMKLGTQTVPCNKKLLWSRIKDLAHQFTQVQRDMFTLEDTLLGYLADDLTWCGEFNTSKINYQSCPDWRKDCSNNPVSVFWKTVSRRFAEAACDVVHVMLNGSRSKIFDKNSTFGSVEVHNLQPEKVQTLEAWVIHGGREDSRDLCQDPTIKELESIISKRNIQFSCKNIYRPDKFLQCVKNPEDSSCTSEIDKTHTCPPCPSEVSSVFIFPPKTKDVLTITLTPKVTCVVVDISQNDPEVRFSWFIDDVEVHTAQTHAPEKQSNSTLRSVSELPIVHRDWLNGKTFKCKVNSGAFPAPIEKSISKPETPRGPQVYTMAPPKEEMTQSQVSITCMVKGFYPPDIYTEWKMNGQPQENYKNTPPTMDTDGSYFLYSKLNVKKETWQQGNTFTCSVLHEGLHNHHTEKSLSHSPGK

SEQ ID NO: 270 - protein, 347 aa, synthetic construct
MAQLLFNKTKSVEFTFCNDTVVIPCFVTNMEAQNTTEVYVKWKFKGRDIYTFDGALNKSTVPTDFSSAKIEVSQLLKGDASLKMDKSDAVSHTGNYTCEVTELTREGETIIELKYRVVSWFSPNEDKTHTCPPCPSEVSSVFIFPPKTKDVLTITLTPKVTCVVVDISQNDPEVRFSWFIDDVEVHTAQTHAPEKQSNSTLRSVSELPIVHRDWLNGKTFKCKVNSGAFPAPIEKSISKPETPRGPQVYTMAPPKEEMTQSQVSITCMVKGFYPPDIYTEWKMNGQPQENYKNTPPTMDTDGSYFLYSKLNVKKETWQQGNTFTCSVLHEGLHNHHTEKSLSHSPGK

SEQ ID NO: 271 - protein, 483 aa, synthetic construct; identical to SEQ ID NO: 199

SEQ ID NO: 272 - protein, 483 aa, synthetic construct; identical to SEQ ID NO: 200

SEQ ID NO: 273 - protein, 348 aa, synthetic construct; identical to SEQ ID NO: 201

SEQ ID NO: 274 - protein, 483 aa, synthetic construct; identical to SEQ ID NO: 202

SEQ ID NO: 275 - protein, 483 aa, synthetic construct; identical to SEQ ID NO: 203

SEQ ID NO: 276 - protein, 348 aa, synthetic construct; identical to SEQ ID NO: 204

SEQ ID NO: 277 - protein, 479 aa, synthetic construct; identical to SEQ ID NO: 205

SEQ ID NO: 278 - protein, 479 aa, synthetic construct; identical to SEQ ID NO: 206

SEQ ID NO: 279 - protein, 344 aa, synthetic construct; identical to SEQ ID NO: 207

SEQ ID NO: 280 - protein, 486 aa, synthetic construct; identical to SEQ ID NO: 208

SEQ ID NO: 281 - protein, 486 aa, synthetic construct; identical to SEQ ID NO: 209

SEQ ID NO: 282 - protein, 351 aa, synthetic construct; identical to SEQ ID NO: 210

SEQ ID NO: 283 - protein, 486 aa, synthetic construct; identical to SEQ ID NO: 211

SEQ ID NO: 284 - protein, 486 aa, synthetic construct; identical to SEQ ID NO: 212

SEQ ID NO: 285 - protein, 351 aa, synthetic construct; identical to SEQ ID NO: 213

SEQ ID NO: 286 - protein, 482 aa, synthetic construct; identical to SEQ ID NO: 214

SEQ ID NO: 287 - protein, 482 aa, synthetic construct; identical to SEQ ID NO: 215

SEQ ID NO: 288 - protein, 347 aa, synthetic construct; identical to SEQ ID NO: 216

SEQ ID NO: 289 - protein, 482 aa, synthetic construct; identical to SEQ ID NO: 217

SEQ ID NO: 290 - protein, 482 aa, synthetic construct; identical to SEQ ID NO: 218

SEQ ID NO: 291 - protein, 347 aa, synthetic construct; identical to SEQ ID NO: 219

SEQ ID NO: 292 - protein, 482 aa, synthetic construct; identical to SEQ ID NO: 220

SEQ ID NO: 293 - protein, 482 aa, synthetic construct; identical to SEQ ID NO: 221

SEQ ID NO: 294 - protein, 347 aa, synthetic construct; identical to SEQ ID NO: 222

SEQ ID NO: 295 - protein, 478 aa, synthetic construct
MAVPRWRQQWSGPGTTKRFPETVLARCVKYTEIHPEMRHVDCQSVWDAFKGAFISKHPCNITEEDYQPLMKLGTQTVPCNKILLWSRIKDLAHQFTQVQRDMFTLEDTLLGYLADDLTWCGEFNTSKINYQSCPDWRKDCSNNPVSVFWKTVSRRFAEAACDVVHVMLNGSRSKIFDKNSTFGSVEVHNLQPEKVQTLEAWVIHGGREDSRDLCQDPTIKELESIISKRNIQFSCKNIYRPDKFLQCVKNPEDSSCTSEINPCGCTSEVSSVFIFPPKPKDVLTITLTPKVTCVVVDISQDDPEVHFSWFVDDVEVHTAQTRPPEEQFNSTFRSVSELPILHQDWLNGRTFRCKVTSAAFPSPIEKTISKPERTQVPHVYTMSPTKEEMTQNEVSITCMVKGFYPPDIYVEWQMNGQPQENYKNTPPTMDTDGSYFLYSKLNVKKEKWQQGNTFTCSVLHEGLHNHHTEKSLSHSPGK

SEQ ID NO: 296 - protein, 478 aa, synthetic construct
MAVPRWRQQWSGPGTTKRFPETVLARCVKYTEIHPEMRHVDCQSVWDAFKGAFISKHPCNITEEDYQPLMKLGTQTVPCNKKLLWSRIKDLAHQFTQVQRDMFTLEDTLLGYLADDLTWCGEFNTSKINYQSCPDWRKDCSNNPVSVFWKTVSRRFAEAACDVVHVMLNGSRSKIFDKNSTFGSVEVHNLQPEKVQTLEAWVIHGGREDSRDLCQDPTIKELESIISKRNIQFSCKNIYRPDKFLQCVKNPEDSSCTSEINPCGCTSEVSSVFIFPPKPKDVLTITLTPKVTCVVVDISQDDPEVHFSWFVDDVEVHTAQTRPPEEQFNSTFRSVSELPILHQDWLNGRTFRCKVTSAAFPSPIEKTISKPERTQVPHVYTMSPTKEEMTQNEVSITCMVKGFYPPDIYVEWQMNGQPQENYKNTPPTMDTDGSYFLYSKLNVKKEKWQQGNTFTCSVLHEGLHNHHTEKSLSHSPGK

SEQ ID NO: 297 - protein, 343 aa, synthetic construct
MAQLLFNKTKSVEFTFCNDTVVIPCFVTNMEAQNTTEVYVKWKFKGRDIYTFDGALNKSTVPTDFSSAKIEVSQLLKGDASLKMDKSDAVSHTGNYTCEVTELTREGETIIELKYRVVSWFSPNENPCGCTSEVSSVFIFPPKPKDVLTITLTPKVTCVVVDISQDDPEVHFSWFVDDVEVHTAQTRPPEEQFNSTFRSVSELPILHQDWLNGRTFRCKVTSAAFPSPIEKTISKPERTQVPHVYTMSPTKEEMTQNEVSITCMVKGFYPPDIYVEWQMNGQPQENYKNTPPTMDTDGSYFLYSKLNVKKEKWQQGNTFTCSVLHEGLHNHHTEKSLSHSPGK

SEQ ID NO: 298 - protein, 486 aa, synthetic construct; identical to SEQ ID NO: 223

SEQ ID NO: 299 - protein, 486 aa, synthetic construct; identical to SEQ ID NO: 224

SEQ ID NO: 300 - protein, 351 aa, synthetic construct; identical to SEQ ID NO: 225

SEQ ID NO: 301 - protein, 536 aa, synthetic construct
SEQIDNOCDISOFORMGSLINKERHUMANIGGHINGERATIGGBFCCHCHMAVPRWRQQWSGPGTTKRFPETVLARCVKYTEIHPEMRHVDCQSVWDAFKGAFISKHPCNITEEDYQPLMKLGTQTVPCNKILLWSRIKDLAHQFTQVQRDMFTLEDTLLGYLADDLTWCGEFNTSKINYQSCPDWRKDCSNNPVSVFWKTVSRRFAEAACDVVHVMLNGSRSKIFDKNSTFGSVEVHNLQPEKVQTLEAWVIHGGREDSRDLCQDPTIKELESIISKRNIQFSCKNIYRPDKFLQCVKNPEDSSCTSEIGGGSDKTHTCPPCPSEVSSVFIFPPKPKDVLTITLTPKVTCVVVDISQDDPEVHFSWFVDDVEVHTAQTRPPEEQFNSTFRSVSELPILHQDWLNGRTFRCKVTSAAFPSPIEKTISKPERTQVPHVYTMSPTKEEMTQNEVSITCMVKGFYPPDIYVEWQMNGQPQENYKNTPPTMDTDGSYFLYSKLNVKKEKWQQGNTFTCSVLHEGLHNHHTEKSLSHSPGK

SEQ ID NO: 302 - protein, 486 aa, synthetic construct; identical to SEQ ID NO: 227

SEQ ID NO: 303 - protein, 351 aa, synthetic construct; identical to SEQ ID NO: 228

SEQ ID NO: 304 - protein, 482 aa, synthetic construct; identical to SEQ ID NO: 229

SEQ ID NO: 305 - protein, 482 aa, synthetic construct; identical to SEQ ID NO: 230

SEQ ID NO: 306 - protein, 347 aa, synthetic construct; identical to SEQ ID NO: 234

SEQ ID NO: 307 - protein, 486 aa, synthetic construct
MAVPRWRQQWSGPGTTKRFPETVLARCVKYTEIHPEMRHVDCQSVWDAFKGAFISKHPCNITEEDYQPLMKLGTQTVPCNKILLWSRIKDLAHQFTQVQRDMFTLEDTLLGYLADDLTWCGEFNTSKINYQSCPDWRKDCSNNPVSVFWKTVSRRFAEAACDVVHVMLNGSRSKIFDKNSTFGSVEVHNLQPEKVQTLEAWVIHGGREDSRDLCQDPTIKELESIISKRNIQFSCKNIYRPDKFLQCVKNPEDSSCTSEIAAASPPCKCPADDNLGRPSVFIFPPKPKDILMITLTPKVTCVVVDVSEEEPDVQFSWFVDNVRVFTAQTQPHEEQLNGTFRVVSTLHIQHQDWMSGKEFKCKVNNKDLPSPIEKTISKPRKARTPQVYTIPPPREQMSKNKVSLTCMVTSFYPASISVEWERNGELEQDYKNTLPVLDSDESYFLYSKLSVDTDSWMRGDIYTCSVVHEALHNHHTQKNLSRSPGK

SEQ ID NO: 308 - protein, 486 aa, synthetic construct
MAVPRWRQQWSGPGTTKRFPETVLARCVKYTEIHPEMRHVDCQSVWDAFKGAFISKHPCNITEEDYQPLMKLGTQTVPCNKKLLWSRIKDLAHQFTQVQRDMFTLEDTLLGYLADDLTWCGEFNTSKINYQSCPDWRKDCSNNPVSVFWKTVSRRFAEAACDVVHVMLNGSRSKIFDKNSTFGSVEVHNLQPEKVQTLEAWVIHGGREDSRDLCQDPTIKELESIISKRNIQFSCKNIYRPDKFLQCVKNPEDSSCTSEIAAASPPCKCPADDNLGRPSVFIFPPKPKDILMITLTPKVTCVVVDVSEEEPDVQFSWFVDNVRVFTAQTQPHEEQLNGTFRVVSTLHIQHQDWMSGKEFKCKVNNKDLPSPIEKTISKPRKARTPQVYTIPPPREQMSKNKVSLTCMVTSFYPASISVEWERNGELEQDYKNTLPVLDSDESYFLYSKLSVDTDSWMRGDIYTCSVVHEALHNHHTQKNLSRSPGK

SEQ ID NO: 309 - protein, 351 aa, synthetic construct
MAQLLFNKTKSVEFTFCNDTVVIPCFVTNMEAQNTTEVYVKWKFKGRDIYTFDGALNKSTVPTDFSSAKIEVSQLLKGDASLKMDKSDAVSHTGNYTCEVTELTREGETIIELKYRVVSWFSPNEAAASPPCKCPADDNLGRPSVFIFPPKPKDILMITLTPKVTCVVVDVSEEEPDVQFSWFVDNVRVFTAQTQPHEEQLNGTFRVVSTLHIQHQDWMSGKEFKCKVNNKDLPSPIEKTISKPRKARTPQVYTIPPPREQMSKNKVSLTCMVTSFYPASISVEWERNGELEQDYKNTLPVLDSDESYFLYSKLSVDTDSWMRGDIYTCSVVHEALHNHHTQKNLSRSPGK

SEQ ID NO: 310 - protein, 486 aa, synthetic construct
MAVPRWRQQWSGPGTTKRFPETVLARCVKYTEIHPEMRHVDCQSVWDAFKGAFISKHPCNITEEDYQPLMKLGTQTVPCNKILLWSRIKDLAHQFTQVQRDMFTLEDTLLGYLADDLTWCGEFNTSKINYQSCPDWRKDCSNNPVSVFWKTVSRRFAEAACDVVHVMLNGSRSKIFDKNSTFGSVEVHNLQPEKVQTLEAWVIHGGREDSRDLCQDPTIKELESIISKRNIQFSCKNIYRPDKFLQCVKNPEDSSCTSEIGGGSPPCKCPADDNLGRPSVFIFPPKPKDILMITLTPKVTCVVVDVSEEEPDVQFSWFVDNVRVFTAQTQPHEEQLNGTFRVVSTLHIQHQDWMSGKEFKCKVNNKDLPSPIEKTISKPRKARTPQVYTIPPPREQMSKNKVSLTCMVTSFYPASISVEWERNGELEQDYKNTLPVLDSDESYFLYSKLSVDTDSWMRGDIYTCSVVHEALHNHHTQKNLSRSPGK

SEQ ID NO: 311 - protein, 486 aa, synthetic construct
MAVPRWRQQWSGPGTTKRFPETVLARCVKYTEIHPEMRHVDCQSVWDAFKGAFISKHPCNITEEDYQPLMKLGTQTVPCNKKLLWSRIKDLAHQFTQVQRDMFTLEDTLLGYLADDLTWCGEFNTSKINYQSCPDWRKDCSNNPVSVFWKTVSRRFAEAACDVVHVMLNGSRSKIFDKNSTFGSVEVHNLQPEKVQTLEAWVIHGGREDSRDLCQDPTIKELESIISKRNIQFSCKNIYRPDKFLQCVKNPEDSSCTSEIGGGSPPCKCPADDNLGRPSVFIFPPKPKDILMITLTPKVTCVVVDVSEEEPDVQFSWFVDNVRVFTAQTQPHEEQLNGTFRVVSTLHIQHQDWMSGKEFKCKVNNKDLPSPIEKTISKPRKARTPQVYTIPPPREQMSKNKVSLTCMVTSFYPASISVEWERNGELEQDYKNTLPVLDSDESYFLYSKLSVDTDSWMRGDIYTCSVVHEALHNHHTQKNLSRSPGK

SEQ ID NO: 312 - protein, 351 aa, synthetic construct
MAQLLFNKTKSVEFTFCNDTVVIPCFVTNMEAQNTTEVYVKWKFKGRDIYTFDGALNKSTVPTDFSSAKIEVSQLLKGDASLKMDKSDAVSHTGNYTCEVTELTREGETIIELKYRVVSWFSPNEGGGSPPCKCPADDNLGRPSVFIFPPKPKDILMITLTPKVTCVVVDVSEEEPDVQFSWFVDNVRVFTAQTQPHEEQLNGTFRVVSTLHIQHQDWMSGKEFKCKVNNKDLPSPIEKTISKPRKARTPQVYTIPPPREQMSKNKVSLTCMVTSFYPASISVEWERNGELEQDYKNTLPVLDSDESYFLYSKLSVDTDSWMRGDIYTCSVVHEALHNHHTQKNLSRSPGK

SEQ ID NO: 313 - protein, 482 aa, synthetic construct
MAVPRWRQQWSGPGTTKRFPETVLARCVKYTEIHPEMRHVDCQSVWDAFKGAFISKHPCNITEEDYQPLMKLGTQTVPCNKILLWSRIKDLAHQFTQVQRDMFTLEDTLLGYLADDLTWCGEFNTSKINYQSCPDWRKDCSNNPVSVFWKTVSRRFAEAACDVVHVMLNGSRSKIFDKNSTFGSVEVHNLQPEKVQTLEAWVIHGGREDSRDLCQDPTIKELESIISKRNIQFSCKNIYRPDKFLQCVKNPEDSSCTSEIPPCKCPADDNLGRPSVFIFPPKPKDILMITLTPKVTCVVVDVSEEEPDVQFSWFVDNVRVFTAQTQPHEEQLNGTFRVVSTLHIQHQDWMSGKEFKCKVNNKDLPSPIEKTISKPRKARTPQVYTIPPPREQMSKNKVSLTCMVTSFYPASISVEWERNGELEQDYKNTLPVLDSDESYFLYSKLSVDTDSWMRGDIYTCSVVHEALHNHHTQKNLSRSPGK

SEQ ID NO: 314 - protein, 482 aa, synthetic construct
MAVPRWRQQWSGPGTTKRFPETVLARCVKYTEIHPEMRHVDCQSVWDAFKGAFISKHPCNITEEDYQPLMKLGTQTVPCNKKLLWSRIKDLAHQFTQVQRDMFTLEDTLLGYLADDLTWCGEFNTSKINYQSCPDWRKDCSNNPVSVFWKTVSRRFAEAACDVVHVMLNGSRSKIFDKNSTFGSVEVHNLQPEKVQTLEAWVIHGGREDSRDLCQDPTIKELESIISKRNIQFSCKNIYRPDKFLQCVKNPEDSSCTSEIPPCKCPADDNLGRPSVFIFPPKPKDILMITLTPKVTCVVVDVSEEEPDVQFSWFVDNVRVFTAQTQPHEEQLNGTFRVVSTLHIQHQDWMSGKEFKCKVNNKDLPSPIEKTISKPRKARTPQVYTIPPPREQMSKNKVSLTCMVTSFYPASISVEWERNGELEQDYKNTLPVLDSDESYFLYSKLSVDTDSWMRGDIYTCSVVHEALHNHHTQKNLSRSPGK

SEQ ID NO: 315 - protein, 347 aa, synthetic construct
MAQLLFNKTKSVEFTFCNDTVVIPCFVTNMEAQNTTEVYVKWKFKGRDIYTFDGALNKSTVPTDFSSAKIEVSQLLKGDASLKMDKSDAVSHTGNYTCEVTELTREGETIIELKYRVVSWFSPNEPPCKCPADDNLGRPSVFIFPPKPKDILMITLTPKVTCVVVDVSEEEPDVQFSWFVDNVRVFTAQTQPHEEQLNGTFRVVSTLHIQHQDWMSGKEFKCKVNNKDLPSPIEKTISKPRKARTPQVYTIPPPREQMSKNKVSLTCMVTSFYPASISVEWERNGELEQDYKNTLPVLDSDESYFLYSKLSVDTDSWMRGDIYTCSVVHEALHNHHTQKNLSRSPGK

SEQ ID NO: 316 - protein, 489 aa, synthetic construct
MAVPRWRQQWSGPGTTKRFPETVLARCVKYTEIHPEMRHVDCQSVWDAFKGAFISKHPCNITEEDYQPLMKLGTQTVPCNKILLWSRIKDLAHQFTQVQRDMFTLEDTLLGYLADDLTWCGEFNTSKINYQSCPDWRKDCSNNPVSVFWKTVSRRFAEAACDVVHVMLNGSRSKIFDKNSTFGSVEVHNLQPEKVQTLEAWVIHGGREDSRDLCQDPTIKELESIISKRNIQFSCKNIYRPDKFLQCVKNPEDSSCTSEIAAASPSTCSKPTCPDDNLGRPSVFIFPPKPKDILMITLTPKVTCVVVDVSEEEPDVQFSWFVDNVRVFTAQTQPHEEQLNGTFRVVSTLHIQHQDWMSGKEFKCKVNNKDLPSPIEKTISKPRKARTPQVYTIPPPREQMSKNKVSLTCMVTSFYPASISVEWERNGELEQDYKNTLPVLDSDESYFLYSKLSVDTDSWMRGDIYTCSVVHEALHNHHTQKNLSRSPGK

SEQ ID NO: 317 - protein, 489 aa, synthetic construct
MAVPRWRQQWSGPGTTKRFPETVLARCVKYTEIHPEMRHVDCQSVWDAFKGAFISKHPCNITEEDYQPLMKLGTQTVPCNKKLLWSRIKDLAHQFTQVQRDMFTLEDTLLGYLADDLTWCGEFNTSKINYQSCPDWRKDCSNNPVSVFWKTVSRRFAEAACDVVHVMLNGSRSKIFDKNSTFGSVEVHNLQPEKVQTLEAWVIHGGREDSRDLCQDPTIKELESIISKRNIQFSCKNIYRPDKFLQCVKNPEDSSCTSEIAAASPSTCSKPTCPDDNLGRPSVFIFPPKPKDILMITLTPKVTCVVVDVSEEEPDVQFSWFVDNVRVFTAQTQPHEEQLNGTFRVVSTLHIQHQDWMSGKEFKCKVNNKDLPSPIEKTISKPRKARTPQVYTIPPPREQMSKNKVSLTCMVTSFYPASISVEWERNGELEQDYKNTLPVLDSDESYFLYSKLSVDTDSWMRGDIYTCSVVHEALHNHHTQKNLSRSPGK

SEQ ID NO: 318 - protein, 354 aa, synthetic construct
MAQLLFNKTKSVEFTFCNDTVVIPCFVTNMEAQNTTEVYVKWKFKGRDIYTFDGALNKSTVPTDFSSAKIEVSQLLKGDASLKMDKSDAVSHTGNYTCEVTELTREGETIIELKYRVVSWFSPNEAAASPSTCSKPTCPDDNLGRPSVFIFPPKPKDILMITLTPKVTCVVVDVSEEEPDVQFSWFVDNVRVFTAQTQPHEEQLNGTFRVVSTLHIQHQDWMSGKEFKCKVNNKDLPSPIEKTISKPRKARTPQVYTIPPPREQMSKNKVSLTCMVTSFYPASISVEWERNGELEQDYKNTLPVLDSDESYFLYSKLSVDTDSWMRGDIYTCSVVHEALHNHHTQKNLSRSPGK

SEQ ID NO: 319 - protein, 489 aa, synthetic construct
MAVPRWRQQWSGPGTTKRFPETVLARCVKYTEIHPEMRHVDCQSVWDAFKGAFISKHPCNITEEDYQPLMKLGTQTVPCNKILLWSRIKDLAHQFTQVQRDMFTLEDTLLGYLADDLTWCGEFNTSKINYQSCPDWRKDCSNNPVSVFWKTVSRRFAEAACDVVHVMLNGSRSKIFDKNSTFGSVEVHNLQPEKVQTLEAWVIHGGREDSRDLCQDPTIKELESIISKRNIQFSCKNIYRPDKFLQCVKNPEDSSCTSEIGGGSPSTCSKPTCPDDNLGRPSVFIFPPKPKDILMITLTPKVTCVVVDVSEEEPDVQFSWFVDNVRVFTAQTQPHEEQLNGTFRVVSTLHIQHQDWMSGKEFKCKVNNKDLPSPIEKTISKPRKARTPQVYTIPPPREQMSKNKVSLTCMVTSFYPASISVEWERNGELEQDYKNTLPVLDSDESYFLYSKLSVDTDSWMRGDIYTCSVVHEALHNHHTQKNLSRSPGK

SEQ ID NO: 320 - protein, 489 aa, synthetic construct
MAVPRWRQQWSGPGTTKRFPETVLARCVKYTEIHPEMRHVDCQSVWDAFKGAFISKHPCNITEEDYQPLMKLGTQTVPCNKKLLWSRIKDLAHQFTQVQRDMFTLEDTLLGYLADDLTWCGEFNTSKINYQSCPDWRKDCSNNPVSVFWKTVSRRFAEAACDVVHVMLNGSRSKIFDKNSTFGSVEVHNLQPEKVQTLEAWVIHGGREDSRDLCQDPTIKELESIISKRNIQFSCKNIYRPDKFLQCVKNPEDSSCTSEIGGGSPSTCSKPTCPDDNLGRPSVFIFPPKPKDILMITLTPKVTCVVVDVSEEEPDVQFSWFVDNVRVFTAQTQPHEEQLNGTFRVVSTLHIQHQDWMSGKEFKCKVNNKDLPSPIEKTISKPRKARTPQVYTIPPPREQMSKNKVSLTCMVTSFYPASISVEWERNGELEQDYKNTLPVLDSDESYFLYSKLSVDTDSWMRGDIYTCSVVHEALHNHHTQKNLSRSPGK

SEQ ID NO: 321 - protein, 354 aa, synthetic construct
MAQLLFNKTKSVEFTFCNDTVVIPCFVTNMEAQNTTEVYVKWKFKGRDIYTFDGALNKSTVPTDFSSAKIEVSQLLKGDASLKMDKSDAVSHTGNYTCEVTELTREGETIIELKYRVVSWFSPNEGGGSPSTCSKPTCPDDNLGRPSVFIFPPKPKDILMITLTPKVTCVVVDVSEEEPDVQFSWFVDNVRVFTAQTQPHEEQLNGTFRVVSTLHIQHQDWMSGKEFKCKVNNKDLPSPIEKTISKPRKARTPQVYTIPPPREQMSKNKVSLTCMVTSFYPASISVEWERNGELEQDYKNTLPVLDSDESYFLYSKLSVDTDSWMRGDIYTCSVVHEALHNHHTQKNLSRSPGK

SEQ ID NO: 322 - protein, 485 aa, synthetic construct
MAVPRWRQQWSGPGTTKRFPETVLARCVKYTEIHPEMRHVDCQSVWDAFKGAFISKHPCNITEEDYQPLMKLGTQTVPCNKILLWSRIKDLAHQFTQVQRDMFTLEDTLLGYLADDLTWCGEFNTSKINYQSCPDWRKDCSNNPVSVFWKTVSRRFAEAACDVVHVMLNGSRSKIFDKNSTFGSVEVHNLQPEKVQTLEAWVIHGGREDSRDLCQDPTIKELESIISKRNIQFSCKNIYRPDKFLQCVKNPEDSSCTSEIPSTCSKPTCPDDNLGRPSVFIFPPKPKDILMITLTPKVTCVVVDVSEEEPDVQFSWFVDNVRVFTAQTQPHEEQLNGTFRVVSTLHIQHQDWMSGKEFKCKVNNKDLPSPIEKTISKPRKARTPQVYTIPPPREQMSKNKVSLTCMVTSFYPASISVEWERNGELEQDYKNTLPVLDSDESYFLYSKLSVDTDSWMRGDIYTCSVVHEALHNHHTQKNLSRSPGK

SEQ ID NO: 323 - protein, 485 aa, synthetic construct
MAVPRWRQQWSGPGTTKRFPETVLARCVKYTEIHPEMRHVDCQSVWDAFKGAFISKHPCNITEEDYQPLMKLGTQTVPCNKKLLWSRIKDLAHQFTQVQRDMFTLEDTLLGYLADDLTWCGEFNTSKINYQSCPDWRKDCSNNPVSVFWKTVSRRFAEAACDVVHVMLNGSRSKIFDKNSTFGSVEVHNLQPEKVQTLEAWVIHGGREDSRDLCQDPTIKELESIISKRNIQFSCKNIYRPDKFLQCVKNPEDSSCTSEIPSTCSKPTCPDDNLGRPSVFIFPPKPKDILMITLTPKVTCVVVDVSEEEPDVQFSWFVDNVRVFTAQTQPHEEQLNGTFRVVSTLHIQHQDWMSGKEFKCKVNNKDLPSPIEKTISKPRKARTPQVYTIPPPREQMSKNKVSLTCMVTSFYPASISVEWERNGELEQDYKNTLPVLDSDESYFLYSKLSVDTDSWMRGDIYTCSVVHEALHNHHTQKNLSRSPGK

SEQ ID NO: 324 - protein, 350 aa, synthetic construct
MAQLLFNKTKSVEFTFCNDTVVIPCFVTNMEAQNTTEVYVKWKFKGRDIYTFDGALNKSTVPTDFSSAKIEVSQLLKGDASLKMDKSDAVSHTGNYTCEVTELTREGETIIELKYRVVSWFSPNEPSTCSKPTCPDDNLGRPSVFIFPPKPKDILMITLTPKVTCVVVDVSEEEPDVQFSWFVDNVRVFTAQTQPHEEQLNGTFRVVSTLHIQHQDWMSGKEFKCKVNNKDLPSPIEKTISKPRKARTPQVYTIPPPREQMSKNKVSLTCMVTSFYPASISVEWERNGELEQDYKNTLPVLDSDESYFLYSKLSVDTDSWMRGDIYTCSVVHEALHNHHTQKNLSRSPGK

SEQ ID NO: 325 - protein, 485 aa, synthetic construct
MAVPRWRQQWSGPGTTKRFPETVLARCVKYTEIHPEMRHVDCQSVWDAFKGAFISKHPCNITEEDYQPLMKLGTQTVPCNKILLWSRIKDLAHQFTQVQRDMFTLEDTLLGYLADDLTWCGEFNTSKINYQSCPDWRKDCSNNPVSVFWKTVSRRFAEAACDVVHVMLNGSRSKIFDKNSTFGSVEVHNLQPEKVQTLEAWVIHGGREDSRDLCQDPTIKELESIISKRNIQFSCKNIYRPDKFLQCVKNPEDSSCTSEIAAASNPCGCTDDNLGRPSVFIFPPKPKDILMITLTPKVTCVVVDVSEEEPDVQFSWFVDNVRVFTAQTQPHEEQLNGTFRVVSTLHIQHQDWMSGKEFKCKVNNKDLPSPIEKTISKPRKARTPQVYTIPPPREQMSKNKVSLTCMVTSFYPASISVEWERNGELEQDYKNTLPVLDSDESYFLYSKLSVDTDSWMRGDIYTCSVVHEALHNHHTQKNLSRSPGK

SEQ ID NO: 326 - protein, 485 aa, synthetic construct
MAVPRWRQQWSGPGTTKRFPETVLARCVKYTEIHPEMRHVDCQSVWDAFKGAFISKHPCNITEEDYQPLMKLGTQTVPCNKKLLWSRIKDLAHQFTQVQRDMFTLEDTLLGYLADDLTWCGEFNTSKINYQSCPDWRKDCSNNPVSVFWKTVSRRFAEAACDVVHVMLNGSRSKIFDKNSTFGSVEVHNLQPEKVQTLEAWVIHGGREDSRDLCQDPTIKELESIISKRNIQFSCKNIYRPDKFLQCVKNPEDSSCTSEIAAASNPCGCTDDNLGRPSVFIFPPKPKDILMITLTPKVTCVVVDVSEEEPDVQFSWFVDNVRVFTAQTQPHEEQLNGTFRVVSTLHIQHQDWMSGKEFKCKVNNKDLPSPIEKTISKPRKARTPQVYTIPPPREQMSKNKVSLTCMVTSFYPASISVEWERNGELEQDYKNTLPVLDSDESYFLYSKLSVDTDSWMRGDIYTCSVVHEALHNHHTQKNLSRSPGK

SEQ ID NO: 327 - protein, 350 aa, synthetic construct
MAQLLFNKTKSVEFTFCNDTVVIPCFVTNMEAQNTTEVYVKWKFKGRDIYTFDGALNKSTVPTDFSSAKIEVSQLLKGDASLKMDKSDAVSHTGNYTCEVTELTREGETIIELKYRVVSWFSPNEAAASNPCGCTDDNLGRPSVFIFPPKPKDILMITLTPKVTCVVVDVSEEEPDVQFSWFVDNVRVFTAQTQPHEEQLNGTFRVVSTLHIQHQDWMSGKEFKCKVNNKDLPSPIEKTISKPRKARTPQVYTIPPPREQMSKNKVSLTCMVTSFYPASISVEWERNGELEQDYKNTLPVLDSDESYFLYSKLSVDTDSWMRGDIYTCSVVHEALHNHHTQKNLSRSPGK

SEQ ID NO: 328 - protein, 485 aa, synthetic construct
MAVPRWRQQWSGPGTTKRFPETVLARCVKYTEIHPEMRHVDCQSVWDAFKGAFISKHPCNITEEDYQPLMKLGTQTVPCNKILLWSRIKDLAHQFTQVQRDMFTLEDTLLGYLADDLTWCGEFNTSKINYQSCPDWRKDCSNNPVSVFWKTVSRRFAEAACDVVHVMLNGSRSKIFDKNSTFGSVEVHNLQPEKVQTLEAWVIHGGREDSRDLCQDPTIKELESIISKRNIQFSCKNIYRPDKFLQCVKNPEDSSCTSEIGGGSNPCGCTDDNLGRPSVFIFPPKPKDILMITLTPKVTCVVVDVSEEEPDVQFSWFVDNVRVFTAQTQPHEEQLNGTFRVVSTLHIQHQDWMSGKEFKCKVNNKDLPSPIEKTISKPRKARTPQVYTIPPPREQMSKNKVSLTCMVTSFYPASISVEWERNGELEQDYKNTLPVLDSDESYFLYSKLSVDTDSWMRGDIYTCSVVHEALHNHHTQKNLSRSPGK

SEQ ID NO: 329 - protein, 485 aa, synthetic construct
MAVPRWRQQWSGPGTTKRFPETVLARCVKYTEIHPEMRHVDCQSVWDAFKGAFISKHPCNITEEDYQPLMKLGTQTVPCNKKLLWSRIKDLAHQFTQVQRDMFTLEDTLLGYLADDLTWCGEFNTSKINYQSCPDWRKDCSNNPVSVFWKTVSRRFAEAACDVVHVMLNGSRSKIFDKNSTFGSVEVHNLQPEKVQTLEAWVIHGGREDSRDLCQDPTIKELESIISKRNIQFSCKNIYRPDKFLQCVKNPEDSSCTSEIGGGSNPCGCTDDNLGRPSVFIFPPKPKDILMITLTPKVTCVVVDVSEEEPDVQFSWFVDNVRVFTAQTQPHEEQLNGTFRVVSTLHIQHQDWMSGKEFKCKVNNKDLPSPIEKTISKPRKARTPQVYTIPPPREQMSKNKVSLTCMVTSFYPASISVEWERNGELEQDYKNTLPVLDSDESYFLYSKLSVDTDSWMRGDIYTCSVVHEALHNHHTQKNLSRSPGK

SEQ ID NO: 330 - protein, 350 aa, synthetic construct
MAQLLFNKTKSVEFTFCNDTVVIPCFVTNMEAQNTTEVYVKWKFKGRDIYTFDGALNKSTVPTDFSSAKIEVSQLLKGDASLKMDKSDAVSHTGNYTCEVTELTREGETIIELKYRVVSWFSPNEGGGSNPCGCTDDNLGRPSVFIFPPKPKDILMITLTPKVTCVVVDVSEEEPDVQFSWFVDNVRVFTAQTQPHEEQLNGTFRVVSTLHIQHQDWMSGKEFKCKVNNKDLPSPIEKTISKPRKARTPQVYTIPPPREQMSKNKVSLTCMVTSFYPASISVEWERNGELEQDYKNTLPVLDSDESYFLYSKLSVDTDSWMRGDIYTCSVVHEALHNHHTQKNLSRSPGK

SEQ ID NO: 331 - protein, 481 aa, synthetic construct
MAVPRWRQQWSGPGTTKRFPETVLARCVKYTEIHPEMRHVDCQSVWDAFKGAFISKHPCNITEEDYQPLMKLGTQTVPCNKILLWSRIKDLAHQFTQVQRDMFTLEDTLLGYLADDLTWCGEFNTSKINYQSCPDWRKDCSNNPVSVFWKTVSRRFAEAACDVVHVMLNGSRSKIFDKNSTFGSVEVHNLQPEKVQTLEAWVIHGGREDSRDLCQDPTIKELESIISKRNIQFSCKNIYRPDKFLQCVKNPEDSSCTSEINPCGCTDDNLGRPSVFIFPPKPKDILMITLTPKVTCVVVDVSEEEPDVQFSWFVDNVRVFTAQTQPHEEQLNGTFRVVSTLHIQHQDWMSGKEFKCKVNNKDLPSPIEKTISKPRKARTPQVYTIPPPREQMSKNKVSLTCMVTSFYPASISVEWERNGELEQDYKNTLPVLDSDESYFLYSKLSVDTDSWMRGDIYTCSVVHEALHNHHTQKNLSRSPGK

SEQ ID NO: 332 - protein, 481 aa, synthetic construct
MAVPRWRQQWSGPGTTKRFPETVLARCVKYTEIHPEMRHVDCQSVWDAFKGAFISKHPCNITEEDYQPLMKLGTQTVPCNKKLLWSRIKDLAHQFTQVQRDMFTLEDTLLGYLADDLTWCGEFNTSKINYQSCPDWRKDCSNNPVSVFWKTVSRRFAEAACDVVHVMLNGSRSKIFDKNSTFGSVEVHNLQPEKVQTLEAWVIHGGREDSRDLCQDPTIKELESIISKRNIQFSCKNIYRPDKFLQCVKNPEDSSCTSEINPCGCTDDNLGRPSVFIFPPKPKDILMITLTPKVTCVVVDVSEEEPDVQFSWFVDNVRVFTAQTQPHEEQLNGTFRVVSTLHIQHQDWMSGKEFKCKVNNKDLPSPIEKTISKPRKARTPQVYTIPPPREQMSKNKVSLTCMVTSFYPASISVEWERNGELEQDYKNTLPVLDSDESYFLYSKLSVDTDSWMRGDIYTCSVVHEALHNHHTQKNLSRSPGK

SEQ ID NO: 333 - protein, 346 aa, synthetic construct
MAQLLFNKTKSVEFTFCNDTVVIPCFVTNMEAQNTTEVYVKWKFKGRDIYTFDGALNKSTVPTDFSSAKIEVSQLLKGDASLKMDKSDAVSHTGNYTCEVTELTREGETIIELKYRVVSWFSPNENPCGCTDDNLGRPSVFIFPPKPKDILMITLTPKVTCVVVDVSEEEPDVQFSWFVDNVRVFTAQTQPHEEQLNGTFRVVSTLHIQHQDWMSGKEFKCKVNNKDLPSPIEKTISKPRKARTPQVYTIPPPREQMSKNKVSLTCMVTSFYPASISVEWERNGELEQDYKNTLPVLDSDESYFLYSKLSVDTDSWMRGDIYTCSVVHEALHNHHTQKNLSRSPGK

SEQ ID NO: 334 - protein, 489 aa, synthetic construct
MAVPRWRQQWSGPGTTKRFPETVLARCVKYTEIHPEMRHVDCQSVWDAFKGAFISKHPCNITEEDYQPLMKLGTQTVPCNKILLWSRIKDLAHQFTQVQRDMFTLEDTLLGYLADDLTWCGEFNTSKINYQSCPDWRKDCSNNPVSVFWKTVSRRFAEAACDVVHVMLNGSRSKIFDKNSTFGSVEVHNLQPEKVQTLEAWVIHGGREDSRDLCQDPTIKELESIISKRNIQFSCKNIYRPDKFLQCVKNPEDSSCTSEIAAASDKTHTCPPCPDDNLGRPSVFIFPPKPKDILMITLTPKVTCVVVDVSEEEPDVQFSWFVDNVRVFTAQTQPHEEQLNGTFRVVSTLHIQHQDWMSGKEFKCKVNNKDLPSPIEKTISKPRKARTPQVYTIPPPREQMSKNKVSLTCMVTSFYPASISVEWERNGELEQDYKNTLPVLDSDESYFLYSKLSVDTDSWMRGDIYTCSVVHEALHNHHTQKNLSRSPGK

SEQ ID NO: 335 - protein, 489 aa, synthetic construct
MAVPRWRQQWSGPGTTKRFPETVLARCVKYTEIHPEMRHVDCQSVWDAFKGAFISKHPCNITEEDYQPLMKLGTQTVPCNKKLLWSRIKDLAHQFTQVQRDMFTLEDTLLGYLADDLTWCGEFNTSKINYQSCPDWRKDCSNNPVSVFWKTVSRRFAEAACDVVHVMLNGSRSKIFDKNSTFGSVEVHNLQPEKVQTLEAWVIHGGREDSRDLCQDPTIKELESIISKRNIQFSCKNIYRPDKFLQCVKNPEDSSCTSEIAAASDKTHTCPPCPDDNLGRPSVFIFPPKPKDILMITLTPKVTCVVVDVSEEEPDVQFSWFVDNVRVFTAQTQPHEEQLNGTFRVVSTLHIQHQDWMSGKEFKCKVNNKDLPSPIEKTISKPRKARTPQVYTIPPPREQMSKNKVSLTCMVTSFYPASISVEWERNGELEQDYKNTLPVLDSDESYFLYSKLSVDTDSWMRGDIYTCSVVHEALHNHHTQKNLSRSPGK

SEQ ID NO: 336 - protein, 354 aa, synthetic construct
MAQLLFNKTKSVEFTFCNDTVVIPCFVTNMEAQNTTEVYVKWKFKGRDIYTFDGALNKSTVPTDFSSAKIEVSQLLKGDASLKMDKSDAVSHTGNYTCEVTELTREGETIIELKYRVVSWFSPNEAAASDKTHTCPPCPDDNLGRPSVFIFPPKPKDILMITLTPKVTCVVVDVSEEEPDVQFSWFVDNVRVFTAQTQPHEEQLNGTFRVVSTLHIQHQDWMSGKEFKCKVNNKDLPSPIEKTISKPRKARTPQVYTIPPPREQMSKNKVSLTCMVTSFYPASISVEWERNGELEQDYKNTLPVLDSDESYFLYSKLSVDTDSWMRGDIYTCSVVHEALHNHHTQKNLSRSPGK

SEQ ID NO: 337 - protein, 489 aa, synthetic construct
MAVPRWRQQWSGPGTTKRFPETVLARCVKYTEIHPEMRHVDCQSVWDAFKGAFISKHPCNITEEDYQPLMKLGTQTVPCNKILLWSRIKDLAHQFTQVQRDMFTLEDTLLGYLADDLTWCGEFNTSKINYQSCPDWRKDCSNNPVSVFWKTVSRRFAEAACDVVHVMLNGSRSKIFDKNSTFGSVEVHNLQPEKVQTLEAWVIHGGREDSRDLCQDPTIKELESIISKRNIQFSCKNIYRPDKFLQCVKNPEDSSCTSEIGGGSDKTHTCPPCPDDNLGRPSVFIFPPKPKDILMITLTPKVTCVVVDVSEEEPDVQFSWFVDNVRVFTAQTQPHEEQLNGTFRVVSTLHIQHQDWMSGKEFKCKVNNKDLPSPIEKTISKPRKARTPQVYTIPPPREQMSKNKVSLTCMVTSFYPASISVEWERNGELEQDYKNTLPVLDSDESYFLYSKLSVDTDSWMRGDIYTCSVVHEALHNHHTQKNLSRSPGK

SEQ ID NO: 338 - protein, 489 aa, synthetic construct
MAVPRWRQQWSGPGTTKRFPETVLARCVKYTEIHPEMRHVDCQSVWDAFKGAFISKHPCNITEEDYQPLMKLGTQTVPCNKKLLWSRIKDLAHQFTQVQRDMFTLEDTLLGYLADDLTWCGEFNTSKINYQSCPDWRKDCSNNPVSVFWKTVSRRFAEAACDVVHVMLNGSRSKIFDKNSTFGSVEVHNLQPEKVQTLEAWVIHGGREDSRDLCQDPTIKELESIISKRNIQFSCKNIYRPDKFLQCVKNPEDSSCTSEIGGGSDKTHTCPPCPDDNLGRPSVFIFPPKPKDILMITLTPKVTCVVVDVSEEEPDVQFSWFVDNVRVFTAQTQPHEEQLNGTFRVVSTLHIQHQDWMSGKEFKCKVNNKDLPSPIEKTISKPRKARTPQVYTIPPPREQMSKNKVSLTCMVTSFYPASISVEWERNGELEQDYKNTLPVLDSDESYFLYSKLSVDTDSWMRGDIYTCSVVHEALHNHHTQKNLSRSPGK

SEQ ID NO: 339 - protein, 354 aa, synthetic construct
MAQLLFNKTKSVEFTFCNDTVVIPCFVTNMEAQNTTEVYVKWKFKGRDIYTFDGALNKSTVPTDFSSAKIEVSQLLKGDASLKMDKSDAVSHTGNYTCEVTELTREGETIIELKYRVVSWFSPNEGGGSDKTHTCPPCPDDNLGRPSVFIFPPKPKDILMITLTPKVTCVVVDVSEEEPDVQFSWFVDNVRVFTAQTQPHEEQLNGTFRVVSTLHIQHQDWMSGKEFKCKVNNKDLPSPIEKTISKPRKARTPQVYTIPPPREQMSKNKVSLTCMVTSFYPASISVEWERNGELEQDYKNTLPVLDSDESYFLYSKLSVDTDSWMRGDIYTCSVVHEALHNHHTQKNLSRSPGK

SEQ ID NO: 340 - protein, 485 aa, synthetic construct
MAVPRWRQQWSGPGTTKRFPETVLARCVKYTEIHPEMRHVDCQSVWDAFKGAFISKHPCNITEEDYQPLMKLGTQTVPCNKILLWSRIKDLAHQFTQVQRDMFTLEDTLLGYLADDLTWCGEFNTSKINYQSCPDWRKDCSNNPVSVFWKTVSRRFAEAACDVVHVMLNGSRSKIFDKNSTFGSVEVHNLQPEKVQTLEAWVIHGGREDSRDLCQDPTIKELESIISKRNIQFSCKNIYRPDKFLQCVKNPEDSSCTSEIDKTHTCPPCPDDNLGRPSVFIFPPKPKDILMITLTPKVTCVVVDVSEEEPDVQFSWFVDNVRVFTAQTQPHEEQLNGTFRVVSTLHIQHQDWMSGKEFKCKVNNKDLPSPIEKTISKPRKARTPQVYTIPPPREQMSKNKVSLTCMVTSFYPASISVEWERNGELEQDYKNTLPVLDSDESYFLYSKLSVDTDSWMRGDIYTCSVVHEALHNHHTQKNLSRSPGK

SEQ ID NO: 341 - protein, 485 aa, synthetic construct
MAVPRWRQQWSGPGTTKRFPETVLARCVKYTEIHPEMRHVDCQSVWDAFKGAFISKHPCNITEEDYQPLMKLGTQTVPCNKKLLWSRIKDLAHQFTQVQRDMFTLEDTLLGYLADDLTWCGEFNTSKINYQSCPDWRKDCSNNPVSVFWKTVSRRFAEAACDVVHVMLNGSRSKIFDKNSTFGSVEVHNLQPEKVQTLEAWVIHGGREDSRDLCQDPTIKELESIISKRNIQFSCKNIYRPDKFLQCVKNPEDSSCTSEIDKTHTCPPCPDDNLGRPSVFIFPPKPKDILMITLTPKVTCVVVDVSEEEPDVQFSWFVDNVRVFTAQTQPHEEQLNGTFRVVSTLHIQHQDWMSGKEFKCKVNNKDLPSPIEKTISKPRKARTPQVYTIPPPREQMSKNKVSLTCMVTSFYPASISVEWERNGELEQDYKNTLPVLDSDESYFLYSKLSVDTDSWMRGDIYTCSVVHEALHNHHTQKNLSRSPGK

SEQ ID NO: 342 - protein, 350 aa, synthetic construct
MAQLLFNKTKSVEFTFCNDTVVIPCFVTNMEAQNTTEVYVKWKFKGRDIYTFDGALNKSTVPTDFSSAKIEVSQLLKGDASLKMDKSDAVSHTGNYTCEVTELTREGETIIELKYRVVSWFSPNEDKTHTCPPCPDDNLGRPSVFIFPPKPKDILMITLTPKVTCVVVDVSEEEPDVQFSWFVDNVRVFTAQTQPHEEQLNGTFRVVSTLHIQHQDWMSGKEFKCKVNNKDLPSPIEKTISKPRKARTPQVYTIPPPREQMSKNKVSLTCMVTSFYPASISVEWERNGELEQDYKNTLPVLDSDESYFLYSKLSVDTDSWMRGDIYTCSVVHEALHNHHTQKNLSRSPGK